European Patent Application EP 4 209 502 A1, published July 12, 2023. Title: Fucose sensing and signalling in plants. Applicant: KWS SAAT SE & Co. KGaA. The sequence listing filed with the application follows.

SEQUENCE LISTING (154 sequences)

SEQ ID NO: 1 - DNA, 1467 bp, Arabidopsis thaliana
  AtERDL4 (At1g19450)
atgagttttagggatgataatacggaagagggaagaaatgatcttcggcgaccgttcttacacacaggaagttggtatcggatgggttcgagacaatctagtatgttggaatcgtctcaagttattcgagacagctcaatttctgtcttagcttgtgttttgattgttgctcttggtcctattcaattcggattcacttgtggttattcctcaccaactcaagctgccattactaaggatcttggtttaactgtatcagagtactctgtgtttgggtctctatccaatgtgggtgctatggttggagcaattgcgagtggtcagattgctgaatacgttggacggaaagggtctctgatgattgctgcaattcccaatattattggatggctttcgatatcatttgcaaaagatacttcttttctttacatgggaagattgttagaaggcttcggagttgggattatctcctatacggttcccgtatatatagctgagatcgctccacagaccatgagaggagccttaggttcagttaaccagctttctgtaacaattgggataatgctggcgtatttactcggtctctttgttccatggagaattcttgcagttttgggagtattgccatgtacattgttgataccgggtctttttttcattcctgaatctcctcggtggttggcaaagatgggtttgacagatgatttcgaaacttcattgcaagttcttcgtggatttgagactgatattaccgttgaggttaatgaaatcaagagatctgtggcatcatctagcaaacgttctgcagttcggtttgtagacctcaagcgcaggagatactatttcccactgatggttggtatagggctgcttgcacttcaacaacttggaggaatcaatggtgtcttgttctattcgagtacaatttttgaatctgcaggggtgacatcaagtaatgtggcgacatttggagttggcgttgttcaggtagtggcgactgggatagcgacatggttggtggataaagcaggtcgtcggcttctactcatgatctcttctatcggaatgacgataagcctcgtgattgtagcagttgcattttaccttaaggaatttgtatcacctgattccaacatgtacaacattctaagcatggtttccgtagttggagttgtggctatggttatttcttgctctctaggaatgggaccaattccatggctgattatgtctgagattctgccagtgaatataaagggtttagccggaagtatagcaactttgttaaactggttcgtgtcatggttagtgacaatgactgcaaatatgctgttagcatggagcagtgggggaactttcactctctacgctttggtttgtggattcactgtggtttttgtgagtctttgggttcctgagactaaaggaaaaacgcttgaagagatccaagctttgttcagatga

SEQ ID NO: 2 - DNA, 2220 bp, Arabidopsis thaliana
  AtTST2 (At4g35300)
atgagtggagctgtgcttgttgctattgctgctgctgttggcaacttgttacaaggatgggataacgcaactattgcaggagctgtgttgtacataaaaaaggagtttaatttggagagtaatccatcagtggaaggtctaattgtggcgatgtcacttattggtgctactctgattacaacatgctctggaggggtagctgattggcttggtcgccgtcccatgctaatattgtcctcaattctctactttgttggttctctagtaatgctatggtctccgaatgtttatgtgttgctcttaggaaggttgttagatggatttggggttggtcttgtggtcacacttgttcctatttatatatctgagactgcaccacctgagattaggggactgttgaatacgctaccgcagttcactggctctggagggatgttcttatcttactgtatggttttcggaatgtcgttgatgccatcacctagctggagattgatgcttggtgtccttttcatcccttcccttgtctttttcttcctcacggtcttcttcttgcccgagtccccaaggtggctcgtgagcaaaggtcgaatgcttgaagcaaagcgggttcttcagagactgcgtggtcgcgaagatgtgtctggtgagatggctttgttggttgagggtcttggaattggaggtgaaacaaccatagaggaatatataattggtcccgcggatgaagttactgatgatcatgatatagctgtggataaggatcaaattaagttatatggtgcagaagaagggctgagttgggttgctaggccagtcaaaggaggaagcactatgagtgttttgtctcgccatggaagtacaatgagcaggaggcaaggctcattgattgatcctcttgtcacactgtttgggagcgttcacgagaagatgccggacactggaagcatgaggagtgccttgttcccacattttgggagtatgttcagtgttggagggaatcaaccaagacatgaagattgggatgaagagaatcttgttggagaaggtgaggattatccatccgaccatggagatgattctgaagatgatcttcattctccgttgatctcacgtcaaacgacaagcatggagaaagacatgcctcacactgctcatggaactctttctaccttcagacatggaagtcaagtgcagggagctcaaggggaaggagcgggtagtatggggattggaggtggatggcaagtggcatggaaatggacggaaagagaagatgaatcgggacagaaagaaggtgggtttaaacggatatacttgcatcaagaaggtttcccaggatctcgacgtggctcaattgtttcattgcctggtggtgatggaaccggtgaggcagattttgtacaagcgtctgctttggttagccaaccagctctttattccaaagaccttctcaaagaacatacaattggtcctgctatggtacatccatccgaaacaactaaagggtcaatttggcatgatcttcatgatcctggagtcaagcgtgcattagtcgtaggagttggacttcaaatacttcagcagttctcaggcatcaacggagttctttactacacaccgcaaatccttgagcaggcgggtgtcgggatcctactatcgaacatggggattagttcttcctcagcatccttacttataagtgcattgacaacctttgtgatgttacctgcaatagctgttgcaatgaggctcatggatctttctggtcgaaggaccttgcttctcaccacgataccaatcctgatagcatctctattggttttagtaatctcaaatcttgttcacatgaacagcattgtgcacgcggtcttatcaaccgtaagcgttgtgctctacttctgcttcttcgtgatgggtttcggtcctgctccaaacatcctctgttcagagatttttccaactcgagtccgcggaatctgcatcgccatctgcgcactcaccttctggatctgtgacataatcgtcacttacagtctccccgtgctgctcaaatccattggactagctggtgtgtttggaatgtacgcaatcgtatgttgcatttcatgggtctttgtgttcattaaagtcccggaaactaaaggcatgccacttgaagtcatcacagagttcttttctgttggagctagacaagctgaagctgctaaaaacgagtga

SEQ ID NO: 3 - DNA, 1512 bp, Arabidopsis thaliana
  AtVGT1 (At3g03090)
atggggtttgatcccgagaaccaatcgatctcttccgttggacaggttgttggtgattcttcttcaggtgggattactgctgaaaaggaacctttgttaaaggaaaaccacagcccagagaactactctgttcttgcagccattcctccgtttctctttccagctcttggagcattgctttttggttatgaaattggtgcaacatcttgtgctatcatgtctcttaagtcgcctactctaagtggaatttcatggtacgacttgtcttcagtggatgttggtataattaccagtggctcactgtatggtgccttaattggctccattgttgcatttagtgttgccgacattataggaaggagaaaggagctgattttggctgcattcttgtatcttgttggagccattgtgactgtagtagcacctgtcttttccatactgataattggacgagttacgtatggcatggggattggactgaccatgcacgcggctccaatgtacattgcagagactgctccaagtcaaatacgtggacggatgatatcactaaaggaattctccactgtccttgggatggttgggggttatggaatcggtagcctttggattacggttatttctggttggcgttacatgtacgcaacaattctcccttttccagttattatgggaactggaatgtgttggctaccagcatctccgaggtggcttttactgcgcgctctccagggacaaggaaatggggagaatcttcaacaggctgcgattagatctctttgtcgccttagagggtctgtcatagctgactcagcagctgaacaagtaaacgaaatattggctgaactttcccttgtgggtgaagacaaagaagctacatttggtgaattatttcgaggcaaatgcttgaaagctctcactatagcaggagggttagtcttgttccaacagataactgggcaaccaagtgtactatattatgcaccatcaatactacagactgccggcttttctgctgcagctgatgcaactcggatctcaattctgctcggcctattgaagttggttatgacaggagtttctgtgatagttatcgacagagttggaaggagacctttacttctttgtggtgttagcggaatggtgatctcattgttcctcctgggatcctactacatgttttataaaaatgtaccagctgttgctgtagctgcattgctactgtatgtaggctgttaccagctgtcctttggccctattggttggctgatgatttcagagatatttcccttaaaattaagaggtagaggaatcagtctagcagtgcttgtgaattttggcgcaaacgcacttgtgacattcgctttctcaccgctaaaggagctgttaggagctggaatactgttctgtgcatttggagtgatatgtgtcgtgtctctcttcttcatatactacattgtgccagagacaaagggtctcactcttgaagaaattgaagccaaatgtctctaa

SEQ ID NO: 4 - DNA, 1512 bp, Arabidopsis thaliana
  AtVGT2 (At5g17010)
atggcgcttgatcctgagcagcagcaaccaatctcctctgtttccagagagtttggtaagtcatctggtgagatcagcccagaaagggagcctcttattaaagagaatcatgtcccagaaaactactctgtcgttgccgccattctcccgtttttatttccagctctcggaggactgctttatggttatgaaattggtgcaacttcttgtgcaaccatttcacttcagtcgccttcattaagtggaatttcatggtacaacttgtcctcagtggatgttggtctagttaccagtggctcactttacggtgcattatttggctcaattgtggcttttactatcgctgacgttataggaagaagaaaggagctgattttggctgcattattgtatctcgttggagcccttgtgactgcactagccccaacctattccgttctgataattggacgggttatttatggggtctcagttggactggcaatgcatgcggctccgatgtacattgcagagactgctccaagtccgatacgtggacagctggtatcattaaaggaattcttcatagtccttgggatggttggaggttatggaatcggtagtcttacagtcaatgttcattctggttggcgatacatgtatgcaacaagtgtccctttggcagttattatgggaattgggatgtggtggctcccagcatcccctaggtggcttttgttgcgcgtcatacaggggaaagggaatgtggagaaccaacgagaggctgcaatcaaatctctctgctgccttagaggccctgcttttgttgattcagctgctgaacaagtaaatgagattttggctgaactaacttttgtgggcgaggataaagaagtcacatttggtgaattatttcaagggaagtgcttgaaagctctcatcataggaggaggtctagtcttgtttcagcagataactggacaaccaagtgtgctttattatgcaccatcaatactgcagaccgctggcttttcagccgcaggtgatgcaacaagggtctcaattctacttggtctattgaagttgattatgacaggagtagctgttgtagttatcgacagacttggaaggagacctttacttcttggtggagttggtggcatggttgtttcattattcctgctggggtcatactacctctttttcagcgcctcaccagttgttgctgtagttgcactgctgctttatgtgggctgttaccagctatcttttggtccaattggttggctgatgatttcagagatatttccccttaaactaagaggtcgaggtctcagtctagcagtgcttgtgaattttggtgcaaacgcacttgtgacatttgcgttttcacccctaaaggaactgctgggagctgggatactgttttgtgggtttggtgtgatatgtgtattgtctctggtattcatattcttcattgtgccagagacaaagggtctcactcttgaggaaattgaagccaaatgtctctaa

SEQ ID NO: 5 - DNA, 726 bp, Arabidopsis thaliana
  AtSWEET17 (At4g15920)
atggcagaggcaagtttctatatcggagtcataggaaatgtaatctccgtactagttttcctctcaccagtggagacgttttggaaaatagtgaagcggagatcaacggaggagtacaaaagcttgccgtacatttgcacgttgttaggatcatcgctatggacatattacggcatcgtcactcccggagaatatcttgtctccaccgttaatggctttggtgctcttgttgaaaccatctacgtttcactttttctcttttatgcccctcgacatctcaagctgaaaacagtggatgtggaagcgatgttgaacgtgttttttccaatcgcggcgattgtggcaacgagaagtgcgtttgaagatgagaagatgcgttctcaatcaataggtttcatatctgctggtctaaacattataatgtatggttctccactttcagcaatgaaaacagtagtgacaacaaagagcgtgaaatacatgccgttttggttgtcgtttttcctcttcttaaacggcgcgatttgggctgtctatgctttactccaacacgacgttttcttactcgtgccaaatggagtggggtttgtgtttgggacaatgcaactcatactttatggaatttacagaaatgccaaaccggttggtttaagcaacggtttaagtgagattgctcaagatgaagaggaaggcctcacatcacgtgttgaacctctcctctcttaa

SEQ ID NO: 6 - DNA, 1326 bp, Arabidopsis thaliana
  AtCIPK6 (At4g30960)
atggtcggagcaaaaccggtggagaatggatctgacggtggtagtagtacggggctgcttcacggccgttacgagctagggcgtcttctaggtcacggaacattcgcgaaggtgtaccacgctcgtaacatacaaaccggaaaaagcgtggcgatgaaagtcgtcggaaaagagaaagtggtgaaagttggtatggttgatcagatcaaacgagagatctctgtgatgaggatggtgaaacatccaaacatcgtcgagcttcacgaagtcatggcgagtaaatccaagatctatttcgccatggagcttgtacgaggcggtgagttattcgctaaggtggctaaaggaagactacgtgaagacgtagctcgtgtttatttccagcaattgatctcagccgttgatttctgtcatagccgtggtgtttatcaccgagatctgaaaccggagaatctcttgttagatgaagaaggtaatctcaaggtgactgattttggtctctctgctttcactgagcatttgaaacaagacggacttcttcatacaacttgtggaactccggcttatgttgcgccggaggttatattgaagaaaggatacgacggagctaaggcggatctgtggtcttgtggtgttatactttttgtgcttcttgctggttatttgccgtttcaagatgataatcttgtgaatatgtataggaagatttacagaggagatttcaaatgtcctggttggctttcttctgatgctagacggcttgtgactaagcttcttgatccgaatccgaatacgaggattactattgagaaggttatggattcgccttggttcaagaaacaagcaacgagatcaagaaacgaaccagtggctgccacaatcacaaccacggaagaggatgttgatttcttggtgcacaagtcgaaggaagagacggagacgttaaacgcgtttcatataatcgcgttatcggaagggtttgatttgtcgccgttgtttgaggagaagaagaaagaggagaaaagagagatgagattcgcgacgtctcggccagcgagtagcgtgatttcgagtttggaagaagcggcgagagttgggaataagtttgatgtgaggaagagtgagagtagagtaaggattgaaggtaaacagaatggtcggaaagggaaattggcggtggaagcggagatattcgcggtggctccgtcgtttgttgtcgtggaagtgaagaaagatcatggagatacgcttgagtacaacaacttctgcagtactgctcttagaccagctctcaaggacattttctggacctctacacctgcttga

SEQ ID NO: 7 - DNA, 1032 bp, Arabidopsis thaliana
  AtFrcK1 (At5g51830)
atgggtgaggatgcaatctcaggtaatctcaagaatctaacgatcgacacaagagattcagaaactcttgtggtatgtttcggtgaaatgttgattgattttgttcctacggtgggaggtgtttcattggctgaagcaccagctttcaagaaagctcctggaggagctcctgctaatgtagctgttggtgtctctagacttggtggctcctctgctttcattggaaaggttggtgatgatgagtttggaagaatgttagctgatattctaaggctgaacaatgttgacaactctgggatgagattcgaccataatgcacggactgctttggcctttgttacgctaagaggtgatggagagagggagtttttgttcttcaggcatccgagtgctgatatgcttcttttggaatctgagcttgacaagaacctcatccaaaaggccaagatctttcactacggatctatcagtttgattgaggaaccttgccgttctactcagcttgtagctatgaaaatcgctaaggctgcagggagtcttttatcttatgacccgaatttgagattgccgttgtggccatcagaagaagctgctaggaaagagataatgagtatctggaatttagctgatgttataaagattagcgaagacgagataacattcctgaccggtggtgatgatccttatgatgatgatgtggtgttgcaaaagctctttcatcccaatcttaagcttcttgttgtttcagaaggacctaatggctgtagatactacactcaggagtttaaaggtagagttggtggagtaaaagtgaagccagttgatacaaccggtgcaggagatgcattcgtgagcgggttattgaacagcttagcttctgatcttactcttctcaaggatgagaagaaactaagagaggcgcttctatttgcaaacgcatgtggagccattacagtaacagagagaggagcgataccggcgatgccaagcatggatgctgttcaagatcttctttcttctactcgctcctaa

SEQ ID NO: 8 - DNA, 978 bp, Arabidopsis thaliana
  AtFrcK2 (At2g31390)
atggcatccaacggtgataaaggactgatcgttagcttcggcgagatgctaatcgatttcgtccctaccgaatcaggcgtctctctcgccgaagctcctggattcctcaaagctccaggcggtgctcccgctaacgtcgcaatcgctgtttctcgtctcggtggacgatctgctttcgtcggaaaacttggagacgacgagttcggtcatatgttggctgggattttgaggaagaacggtgttgatgatcaggggattaacttcgatactggagctagaactgctttagctttcgttacgttacgtgctgatggagatcgtgagtttatgttttaccgcaatcctagcgccgatatgcttcttcgtcctgatgaactcaatctcgacctcatcagatccgcgaaagtgtttcactatggatcaataagtttgatagtggagccgtgtaggtcagctcatttgaaggccatggaagtggcgaaagaagcaggagctcttctttcctatgacccaaacctcagggagcctctgtggccatcaaaagaagaagccaaaacacagatcatgagcatttgggacaaagctgagatcatcaaggtgagcgatgttgagcttgagtttctaactggaagcaacaagattgatgatgagaccgcgttgaccttgtggcatcccaacttgaagctgttgttagtcactcttggtgaaaagggctgtcggtattacaccaagactttcaaaggagccgttgaccctttccatgtgaacgctgtggacacaaccggagctggagattcctttgtcggtgctcttctaaaccagattgtcgatgatcgatccgttctcgaggacgaagagagattgaggaaagtgctgagattcgcaaatgcttgtggagcaatcacaacgaccaaaaaaggagccattccagctcttccctcagatgctgaagttcggagctttctcgaaaagaaatag

SEQ ID NO: 9 - DNA, 1155 bp, Arabidopsis thaliana
  AtFrcK3 (At1g66430)
atggctctccaagccactactactacgttctgcttctccggtccaactttccgatcaactcctcactcactcacttcaaaacgtcctatctccatcaaagctactacttcttctccttcaagactctccaattcacgatctaatctcaaaggaagagcattgtctagtgatggttcaacacaagaatctccttatgtagtctgttttggagaaatgctaatcgattttgtaccgacgacaagcggactttcattagccgatgcaccggcttttaaaaaagctccaggtggtgcacctgctaatgtagctgttggtattgctcgtcttggtggttcttcagctttcattggaaaggttggtgaagatgagtttggttatatgcttgcgaatattttgaaagataataatgtgaacaatgatggtatgaggtttgatccaggagcaagaactgctttagcttttgtgactttgactaatgaaggtgaaagagagtttatgttttaccgaaacccgagtgctgatatgttgttagaggagtctgagcttgattttgatttgatcaaaaaggcaaagatatttcattacggttcgataagtcttatcaccgaaccgtgcaagtctgcgcatatttctgcagctaaggcggctaaggaggctggtgttatactctcttatgaccctaaccttaggcttccgttgtggccttctgcagacaatgctagggaagagattctgagcatttgggagactgctgatattataaagataagtgaagaggagattgtctttctaacgaaaggagaagatccgtatgatgataatgttgtacgcaagttgtttcatcctaagctgaaacttctccttgtcactgaaggtcctgaaggctgtcggtactacaccaaggattttagtgggagagtgcatggattgaaggtggatgtagtggacacaacaggtgctggtgatgcatttgttgcggggatactatcgcaactagccaatgatctctccttgcttcaggacgaagagcgactgagagaggctcttatgtttgcgaatgcatgcggggcattaaccgttaaagtgagaggcgcaatcccggcccttccaaccaaagaagctgtacatgaggctctactcaaagccgtcgtttaa

SEQ ID NO: 10 - DNA, 975 bp, Arabidopsis thaliana
  AtFrcK4 (At4g10260)
atggctaatactccattgatagtttcctttggtgaaatgcttatcgactttgtccctgacacttctggtgtttctttagctgagtccaccggttttctcaaagcccctggtggtgctcctgctaatgttgcttgtgccatcaccaaactcggtggcaaatcagctttcatcggcaagtttggtgatgatgagtttggacacatgttggttaacatattgaagaagaacggtgtgaacagtgaaggtgtttgctttgataccaatgcaagaaccgcgttggcctttgtgactttgaagaaagatggtgagagagagtttatgttttacaggaaccctagtgcggacatgctcttgaaagaatctgaactcaacaaggatcttatcaagaaagctaagattttccactatggttccattagcttgatctctgagccatgtagaacagctcacatggctgcgatgaaaaccgctaaagatgcgggagtcttactctcttatgacccgaacgttcggttgcctctttggccttctactgaagctgctatagaaggcatcaaaagtatttggaatgaggctgatattatcaaggtaagcgatgatgaggtaacgtttctaacgcgtggagatgcggagaaggatgatgttgttttgtctcttatgcatgataagcttaagctgcttattgttactgatggagagaaaggttgcagatactacacaaagaaattcaaagggagagtgcctggatacgctgtgaaagcagttgacacaactggagctggtgattcatttgttggtgcatttcttgtctcattgggaaaagatggctccatactcgatgatgaagggaagctgaaggaagcacttgcctttgcaaatgcatgtggagcagtgtgtactactcagaaaggagctattcctgcacttcccactccagctgatgctcaaaagctcatgaaatctaagtctaaatag

SEQ ID NO: 11 - DNA, 990 bp, Arabidopsis thaliana
  AtFrcK5 (At1g06030)
atgacgtcatccaacggcgataataaaggtctcgtcgttagcttcggcgagatgctcattgacttcgtgcccacggaatccggcgtctccctctctgaatcctctggatttctcaaagctcctggtggtgctccagcaaacgtcgctatcgctgtttcccgtctcggaggtcgcgccgccttcgtcggaaaactcggggacgatgagtttggccatatgcttgccggaatcttgagaaagaacgatgtcgacgatcaggggatcaatttcgataaaggagcaagaaccgcactcgcttttgtgactctgcgttctgacggagaacgagagtttatgttttaccggaatcccagcgccgatatgcttctccggccagatgaactcaacctcgaactaatcagatccgcgaaagtgtttcactatggatcaataagtttgattacagagccatgtagatcagctcacatgaaggcgatggaggtggcgaaagaagctggagctcttctttcctacgatccaaacctcagggaacctctgtggccatcccctgaagaagctaggaaacagatcatgagtatctgggacaaggctgacattattaaggtcagtgacgtcgagcttgagttcttgacaggaaacaaaacgattgatgatgagacagctatgtctctgtggcatcctaatttgaagctcttgcttgttacacttggcgaaaatggatgtcgttactacactaaggatttccatggatctgttgaaactttccatgttgacgctgtggatactactggagctggtgattcttttgttggcgcgcttctaaaccagattgttgatgatcaatctgtactcgaggaggaagagagattgagaaaagtgctgagatttgcaaacgcttgtggagcaatcacgacgactaaaaagggagccattccagctcttcctacagattgtgaagctctcagttttcttaagatacaagtagaatag

SEQ ID NO: 12 - DNA, 981 bp, Arabidopsis thaliana
  AtFrcK6 (At3g59480)
atggctgcatctaacggcgagaaaagcttgatcgtgagcttcggtgaaatgctcatcgatttcgtcccaaccgtctccggtgtatccctcgccgatgctcctggcttcatcaaagcccccggtggtgcacctgccaacgttgccatcgccatttcccgtctaggcggtcgtgccgctttcgttggaaaactcggtgacgacgagttcggtcacatgctcgccggaatcttgaaacagaacggtgtctctgctgaaggtatcaatttcgacactggagccaggactgcacttgcgttcgtgacactaagatctgatggagaacgtgagttcatgttctaccggaaccctagtgccgatatgctcctccgtcccgacgagctcaatcttgatgtcatcagatctgctaaggtgttccactacggatccataagcttgatcgttgagccatgtcgatctgctcacttgaaagccatggaggtggctaaggaagctggtgcgttgctttcatatgatccgaacttgaggcttcctttgtggccctcgaaggaggaggctcagaagcagattcttagcatctgggacaaagctgaagtgatcaaagtcagcgatgaagagcttatgttcttgactggatctgataaggttgatgatgagactgctttgtctctgtggcactctaatctgaaacttctcttggtcactctaggtgaaaagggttgtagatactacaccaagagcttccgtggatctgttgatcccttccatgtggatgcagtagatacaactggtgctggtgattcatttgttggtgcattgctttgcaagattgttgatgaccgtgctgtgcttgaggacgaagctcggctgagagaagtgcttaggcttgcgaatgcttgtggagccatcacaacaacaaagaaaggagctattccagctctccctacagagtctgaagttcagagcctcctgaaaggaaactga

SEQ ID NO: 13 - DNA, 1038 bp, Arabidopsis thaliana
  AtFrcK7 (At1g06020)
atggcatcatccaccggcgagaaaggtctcatcgtgagcttcggcgagatgctcattgacttcgtccctaccgtatccggcgtctccctctccgaatcccccggatttctcaaagctcccggcggtgctccggccaacgtcgccatcgctgtttcacgtcttggaggtcgtgccgccttcgttgggaagctgggagacgatgatttcggtcatatgctcgccggaatcttgagaaagaacggtgtcgacgatcaggggatcaatttcgacgaaggggcgagaactgcactcgcttttgtcactttgcgttctgacggagaacgagagtttatgttttaccggaatcccagcgccgatatgcttctccggccagatgaactgaatcttgaacttatcagatccgcgaaagtgttccactatggatcaataagtttgataacagagccatgtagatcagctcacatgaaggcaatggaagtggcgaaagaagctggagctcttctttcctacgatccaaacctcagggaacctctttggccatcacctgaagaagctaggacacagatcatgagtatctgggacaaggctgacatcattaaggtcagtgacgtggagcttgaattcttgaccgaaaacaaaaccatggatgataagacagcaatgtctctatggcatcccaaccttaagctcttgcttgttactctcggcgaaaagggatgtacttatttcacaaagaaattccatggatcggtagaaacattccatgtggacgccgtggatactaccggagctggagattcgtttgttggtgcacttctacaacagattgttgatgaccagtccgtactcgaggatgaagcgaggttgagaaaagtgctgagatttgcaaacgcttgtggagccatcacaacaactaaaaaaggagccattccagctcttcctacagacattgaagctctcagttttcttaaagaccaaaagaaacgtcaaaccaatcttaaattctcaaaatggtgttgtacggcttctccttgttaa

SEQ ID NO: 14 - DNA, 1416 bp, Arabidopsis thaliana
  AtFrcK8 (At3g54090)
atggcttcacttcttattttcccccaccttcaccattttgattcttcactggaccgtagagaggtactagtagttcgccattcacaagcatcaaggcgatttctcactccgaaagcttcaattaatggcagcggaatcacaaacggagctgcagcggaaaccacctctaaacctagtcgcaaagggaggaagaagaagcaaacatcgacggtaattgagaaagataacaccgagactgatcctgaattgaatccggagttagctgattacgacgacgggatcgagtttccgtacgacgatccgcctcttgtgtgttgcttcggagctgtacagaaggagtttgttccggtggtgcgagtccatgataatccgatgcatcctgatatgtactcgcagtggaagatgctacagtgggatccaccggagtttgggagagctccgggaggtccgccgtcgaatgtggcgatctctcatgtacggttaggtgggagagctgcgtttatggggaaagtaggtgaagatgattttggagatgagcttgttctgatgatgaatcaggagagagttcagacgagagctgtgaaattcgatgagaattcgaaaactgcttgtactcgtgtcaagatcaagtttaaggacgggaaaatgatggcggagactgtgaaagaaccacctgaggactcgctatttgcttcagaactcaatttagctgtgcttaaagaggcgaggatttttcatttcaattcagaagtgttgacgtctcctacaatgcaatcaactctttttacggcaatacaatggtctaagaagtttggtgggcttattttctttgacttgaatctcccattaccgctgtggagatcgcgcaatgagactaggaagttgatcaagaaagcatggaatgaagcaaacatcattgaagtttcacagcaagagcttgagtttctacttgatgaagattactacgagaggagaagaaactacacaccacagtacttcgctgaggattttgatcagacgaaaaacagaagagactattaccattacacaccagaggaaatcaagtcattgtggcatgacaagctgaagctactggttgtgactgatggaacacttcggcttcattactatactcctacttttgatggtgttgtgattggaacagaagatgtgcttataactcctttcacctgtgataggacaggttctggtgatgctgttgttgcagggataatgagaaagctaacaacttgtcctgagatgtttgaggatcaggatgtgatggagcgacagctcaggtttgcagttgctgctgggatcatagcgcagtggacaattggtgcagttagaggtttccctactgaaagcgcgacacagaatttgaaagaacaagtttatgttccatcaatgtggtag

SEQ ID NO: 15 - DNA, 1845 bp, Arabidopsis thaliana
  AtFrcK9 (At1g69200)
atggcgtctctctccttcacccaattcttatcattccccagatgcaatgcagatgttccttgtctgctccagtcgcatggttttgtgaagtttagaggtgaaagatggaatgggaaacaaagcttttctatggctgctggtaggagaaagttatcagagtcagcacctcttgaagaagaaggtaatgatggaaacggtgcggttgtgggaaagaaaccatctaaaagtgttaagagaacaacgaagaagaaggttgtggttaaggatgaaccattagaagaaatttctgaatttttggttgataatgatgatgttttagacaaggaaagcattgtctcagctttgaaaccaaaaaagacaagaactagaaagaaagctgcagcagcttcttctgatgtggaggaagtaaaaaccgagaagaaagtgagacgaaagaggactgttaagaaagataaagatgtggaggatgatttagctactattatggatgctgaggttagtgatgtcgaggaagcattggctgttgaaagcactgatacagagagtgaagaagaagagattgatctgagtaaacatgaaggtgaagatattagtcacacttatggatggcctcctctcgtgtgttgctttggatctgcacaacatgcttttgtgccttcgggaaggccagcaaacaggctattagattatgaactacacgaacggatgagagatgcaaagtgggctccagagaagtatatccgggctcctggaggatgtgcaggaggtgttgctattgctcttgcaagcttgggtggtaaggttgcttttatgggcaaacttggggctgatgactatggtcaagccatgttgtattatctgaatgtgtgcaaagtccaaactagatcagttaagattgatggtaaaagggttacggcgtgttctactatgaagatcagcaagagaggtcgcttgaaatcgacttgtattaagccatgtgcagaggattcactttcaaaatctgaaatcaacgttgatgtgctcaaagaggcgaaaatgttctacttcagcacgcattctctactcgataagaagatgatgtcaactacgatacaagccatcaagatatcaaagcaactaggcaatgtcattttttatgacttgaatctccctttaccactatggcactccagcgaagaaaccaagtctttcatacaggaagtgtggaatcttgcagacgtcattgaaatcacaaaacaggaacttgaattcttatgcggaatcgagcctactgaagagttcgatacagaaaacaatgacatcagtaagtttgtccattacccgccagaaactgtggaacagctttggcatgaaaatctcaaggtcttgtttgtgaccaatggcacttctaagatccattactataccaaagagcacaatggtgctgtttccggaatggaggatgttcccattactccttttacaagggatatgtcagcatctggagatggcatcgttgcaggtctaataagaatgcttacggttcagccagatcttatgaacaataaagggtacctggaacgcacagcgagatatgcaattgagtgtggtattattgatcaatggttgctggcacaaacccgaggatatcctccaaaggatgacatggaagaagaagaagatgatgaagaagaagatgaagtggaatcagatccaaacggtataagatcgataacagagaaggaatacagaacctcaaagccttatgatgaaccagatggtccatacgttatgaaaccagtagaggaaagggagtacaagaagttagagcttgttggctcaatgtttgaagatggtagtttatga

SEQ ID NO: 16 - DNA, 1491 bp, Arabidopsis thaliana
  AtHxK1 (At4g29130)
atgggtaaagtagctgttggagcgactgttgtttgcacggcggcggtttgtgcggtggctgttttggttgttcgacgacggatgcagagctcagggaagtggggacgtgttttggctatcctcaaggcctttgaagaggattgtgcgactccgatctcgaaactgagacaagtggctgatgctatgaccgttgagatgcatgctggtcttgcatccgacggtggtagcaaactcaagatgcttatcagctacgttgataatcttccttccggggatgaaaagggtctcttttatgcattggacctaggggggacaaacttccgtgtcatgcgtgtgcttcttggcgggaagcaagagcgtgttgttaaacaagaattcgaagaagtttcgattcctcctcatttgatgactggtggttcagatgagttgttcaattttatagctgaagctcttgcgaagtttgtcgctacagaatgcgaagactttcatcttccagaaggtagacagagggaattaggtttcactttctcgtttcctgttaagcagacttctctgtcctctggtagtctcatcaaatggacaaaaggcttttccatcgaagaagcagttggacaagatgttgttggagcacttaataaggctctggaaagagttggtcttgacatgcgaatcgcagcacttgttaatgataccgttggaacactagccggtggtagatactataacccggatgttgttgctgctgttattttaggcactgggacaaacgcagcctatgttgagcgtgcaaccgcgatccctaaatggcatggtctgcttccaaaatcaggagaaatggttataaacatggaatggggaaacttcaggtcatcacatcttccattaaccgagtttgatcacacgctggatttcgagagtctgaatccaggcgaacagattcttgagaaaatcatttccggtatgtacttgggagagattttgcgaagagttcttctaaagatggctgaagatgctgctttctttggcgatacagtcccatctaagctgagaataccattcatcattaggactcctcacatgtcggctatgcacaacgacacttctccagacttgaagattgttgggagcaagattaaggatatattggaggtccctacaacttctctgaaaatgagaaaagttgtgatcagtctctgcaacatcatagcaacccgaggagctcgtctctctgctgctggaatctatggtattctgaagaaactgggaagagatactactaaagacgaggaggtgcagaaatcggttatagccatggatggtggattgtttgagcattacactcagtttagtgagtgtatggagagctcactaaaagagttgcttggagatgaagcttcaggaagcgttgaagtcactcactccaatgatggatcaggcattggagctgcgcttcttgctgcttctcactctctctaccttgaagactcttaa

SEQ ID NO: 17 - DNA, 1509 bp, Arabidopsis thaliana
  AtHxK2 (At2g19860)
atgggtaaagtggcagttgcaacgacggtagtgtgttcggtggcggtatgtgcggcggcggcgttgatagtacggaggagaatgaaaagcgcagggaaatgggcaagagtgatagagatattgaaagcctttgaagaagattgtgcaacgccaattgccaaattgagacaagtggctgatgctatgactgttgagatgcatgctggtcttgcttctgaaggtggcagcaagcttaagatgcttattagctacgttgataatcttccttctggggatgagactggttttttctatgcgttggatctaggcggaacaaacttccgtgttatgcgtgtgcttcttggtgggaagcacgaccgtgttgttaaacgagaattcaaagaagaatctattcctcctcatttgatgaccgggaagtcacatgaattattcgattttatcgttgatgttcttgccaagtttgtcgctacagaaggcgaggactttcatctcccacctggtagacaacgggaactaggttttactttctcatttccggttaagcagctatctttatcctctggcactctcatcaactggacgaagggcttttccattgacgatacagttgataaagatgttgttggagaacttgttaaagctatggaaagagttgggctggacatgcttgtcgcagcgcttgttaatgataccattggaacacttgcgggtggtagatacactaacccggatgtcgttgtcgcagttattttgggcaccggcacaaatgcagcctatgtcgaacgtgcacatgcaattcccaaatggcatggtttgctacccaaatcaggagaaatggtgatcaacatggaatggggaaacttcaggtcatcacatcttccattgacagagtacgaccactctctagatgtcgatagtttgaatcctggtgaacagattcttgagaaaatcatttccggaatgtatctgggagaaatcttgcgtagagttcttctgaagatggctgaagaagctgccttctttggcgatatcgtcccacctaagctgaaaataccattcatcataaggaccccgaacatgtctgctatgcacagtgatacttccccggatttgaaggttgtaggaagcaagttaaaagacatattggaggtccagactagttctctgaagatgaggaaagttgtgatcagcctatgtaacatcattgcaagccgaggagctcgtttatctgctgcggggatctatggaatcctcaagaaaataggaagagacgcaacaaaagatggagaagctcagaaatctgtgatagcgatggacggtgggctattcgagcattacactcagttcagtgagtcgatgaagagttcattgaaagagttgcttggagatgaagtttcagagagtgttgaagtgatactgtcgaatgatggttcaggtgttggagctgcattacttgctgcttctcactctcagtatctcgaacttgaagatgactctgaaacaagttaa

SEQ ID NO: 18 - DNA, 1497 bp, Arabidopsis thaliana
  AtHxK3 (At1g50460)
atggggaaagtggcggttgcgtttgcggcggttgctgttgttgcggcttgttctgttgccgcggtgatggttgggaggaggatgaagagtcggaggaaatggaggactgttgttgagattttgaaagagttggaggatgattgtgatactccggttgggaggttgaggcaagtggttgatgctatggccgtggagatgcacgctggtttggcttctgaaggtggctctaagcttaaaatgctcctcactttcgtcgatgatttgcccactgggagggagaaaggtacttattatgcacttcaccttggaggcacttattttaggattttaagggttcttctgggtgatcaaaggtcttatctagatgttcaagatgttgaacgacacccaataccttcacatttgatgaatagcaccagcgaggttcttttcaactttctcgccttttccttggaaaggtttattgaaaaggaggaaaacgggtccgattcacaaggtgttagaagggaacttgcatttacgttctcattccctgtcaagcatacttctatttcttcaggagttctaattaaatggaccaaaggttttgagattagtgaaatggttgggcaagatatagctgaatgtctacaaggagctctgaacagaagaggcctagatatgcatgttgcggctcttgtgaatgatactgttggagccttgtcgcttggatattatcacgatccagatacggttgttgcggttgtatttggaacaggtagtaatgcatgttacttggaaagaaccgatgccataatcaagtgtcagggtctgcttacaacttctggaagcatggtggtaaatatggagtggggaaatttttggtcctctcatttgcctagaacttcgtatgacattgacttggatgcagagagttcaaatgcaaatgatatgggatttgagaagatgatatcaggaatgtatctgggtgacattgttcgtagagtaattctccgcatgtcagaagattctgatatctttggacccatctcgcccgtgttatctgagccttacgttctaagaacaaattcagtctcagccatacatgaagatgacacacctgagttacaagaagtagcaagaatcttgaaagacataggggtatcagatgtaccactgaaggtgagaaaactagtggtgaaaatatgcgatgtggttacacgaagagcagggaggcttgcagcagcaggaatagcaggaatcttgaagaagataggccgagatggaagcgggggaatcacgagcgggagaagcagaagtgaaatccaaatgcagaaaagaacagttgttgcggtagaaggaggtttgtacatgaattacaccatgtttagggaatacatggaagaagctctcgtagagatactaggagaagaagtgagtcaatacgtggtggttaaagccatggaagatggttctagcattggctctgctctcctcgttgcctctttacagtcatga

SEQ ID NO: 19 - DNA, 1509 bp, Arabidopsis thaliana
  AtHxK4 (At3g20040)
atggggaaggttttggtgatgttgacggcagctgcggctgtggtggcttgttcagtggcgactgtgatggtgagaaggaggatgaaagggaggaggaaatggaggagggtggtgggtttacttaaggatttggaggaagcttgtgagacgcctttaggaaggttgaggcagatggttgatgccatagctgtggagatgcaagctggtttggtttctgaaggagggtcaaagcttaaaatgttgctcacttttgttgatgatcttcccaatgggagcgagacaggaacctattatgcacttcatcttggaggctcctactttaggataataaaggttcatctaggtggtcaaagatcatctcttgaagttcaagatgttgaacgacattccataccaacatctttgatgaatagcactagcgaggttctcttcgactttctcgcatcatccttgcagaggtttattgaaaaagaagggaacgatttcagtttgtcacaacctttaaaaagggaacttgcgtttactttttctttcccagtcaagcagacatccatctcatcaggagttctaattaaatggaccaaaggttttgcaattagtgaaatggctggggaagacattgctgaatgtctacaaggagcgttgaacaagagagggctagatattcgcgttgcagctcttgtgaatgatactgttggggctttatcctttggacattttcatgacccagacacaattgctgctgttgtctttggaacaggtagtaatgcatgttaccttgaacgaactgatgccataatcaagtgtcaaaatccacgcacgacttctggaagcatggtggtcaatatggagtggggaaacttttggtcatctcgtctgccaagaacttcatatgaccttgagttggatgcagagagtatgaattcaaatgacatgggctttgagaagatgataggagggatgtatctgggcgacattgtccgcagagtaattcttcgaatgtcacaagagtccgacatctttggacctatctcatccattttatccacgcctttcgttctgagaacaaattctgtctcagcaatgcatgaagatgacacatccgagttacaagaagtagcacgaatcttgaaagatttaggggtgtcagaggtaccaatgaaggtgaggaaacttgtagtgaagatctgcgatgtagtgacacgcagagcagctaggctagcagcagcaggaattgcaggaatcttgaagaaggtagggagagatgggagcggaggaggaaggagaagcgataagcagataatgagaagaacagtggtggcagttgaaggaggtctgtatttgaactacaggatgttcagagaatatatggacgaagctctgagagatatactgggagaagatgtggctcaacacgtagtggtgaaggccatggaagatggttccagcattggctctgcattgttgctggcttcgtcacaaagtgttcaaacaataccatccgtatga

SEQ ID NO: 20 - DNA, 1482 bp, Arabidopsis thaliana
  AtHxK5 (At1g47840)
atgtcactcatgttttcttcccctgtcgtcaccccagcactcggatctttcaccttctcatctcgaccacgctccaattacatcgtgatgtccgccgtccgatctaactctgcttcgacgtgtcctatactgaccaagtttcagaaagactgcgccactcctacaccgtacctacgcaacgtagccaacgccattgctgatgacatgcgagatggtctagctgttgaaggaggaggagatctcgagatgatcttgacttttgttgacgctttgccttctgggaatgaggaagggttgttctatgcattggatttaggaggtacaaattttcgggtgcgtagcgtgcaattaggaggaaagaaagagcgagtcttagctaccgaatctgaacaaatatctatttctcaaaagcttatgattggtacaagtgaggagcttttcgggttcattgcttcaaagcttgcaaattttgttgcaaaggagaagccaggtcggtttcttttagaagaagggaggaaaagggagttagggtttaccttttcattccctgtgaagcaaacctctattgattcaggcacattaagcaagtggactaaaggctttaaagtgtctggaatggaaggaaaaaatgtggttgcttgtttaaatgaagctatggaagcacatggactcgatatgcgagtttctgctcttgtaaatgatggagtgggaacattagctggagcaaggtattgggatgaggatgtgatggtcggtgtgattcttggcactgggaccaatgcttgttatgtagaacagaaacatgcaattcctaaactccgaagcaaatcttcttctggaacaacgatcataaacactgagtggggagggttctctaagattcttccgcaaaccatttttgacctagagatggatgagacaagcctgaatcctggtgaacatttatatgagaagatgatctcagggatgtaccttggtgaaattgtaaggagggttttgctccatatgtgtgaaactagtgacttgtttggacacttcgctcctgccaaactctccactcctttggcactcaggaccgagcatctatgcaaaatgcaagaggacaatacagatgatcttcgggatgttggatcaatcctatacgactttttagatgtagaggcgaatatgaatgcaaggaggagagtggtggaagtgtgtgacacagtagtgaaacgcggagggcgtctagcaggagctggtatagtggcaattctggagaagattgaaaaagataccaaaagaatgggttcaggtaaaagaaccgttgtggctatggacggtgcactgtatgagaagtacccacaatatcgacagtatatgcaagacgcactagtcgagcttcttggccataagcttgcaagtcacgttgcgatcaaacataccaaagacgtgtctgggctcggtgctgctcttttggcggccactaactccatttactag

SEQ ID NO: 21 - DNA, 1482 bp, Arabidopsis thaliana
  AtHxK6 (At4g37840)
atgaccaggaaagaggtggttctggccgtgacggctgcaaccattacggcggttgcagcaggtgtactaatgggtcggtggatccggaggaaagagcggcggttgaaacatacgcagagaattttgaggaaattcgctagagaatgcgccacgccggtttcgaagctttgggcggtggcggacgccttggtcgccgacatgaccgcctctttaaccgccgagtgttgcggttccctcaacatgctcgtttcattcaccggttctctcccttccggtgatgagaaaggggtacactatggagtcaacttgagaggcaaggaactattactgttacgtgggacgctaggtggtaacgaagagcctatttccgatgtacagaagcatgagattccgatccctgacgatgttttaaatggttctttcaaggagttgtgcgatttcatatcattggagcttgttaaatttcttgcgatgaatcccggtggagaagcagaagaagtgaagaatctcgggtttacgttgacgcgctctgttgagcagattgggtcacattcaatctcgtcgatacataggaagagtttagcaaatgacgatgatgagaaggttttgaaagatttggtgaatgatatgaatgaatcactggaaacacacggtctgaaaattcggatgaacacagcgctggtggataatactataggagaattggctggaggaaggtattatcacaaggacactgtggctgcagtatcattaggtatgggaaccaacgctgcttacattgaacaagctcaagagatatcgaggtggaaatctgcgatacgtgagccacaagagatcgttgttagcacagagtggggagatttcagatcttgccatcttcctataaccgagttcgatgcttctcttgacgcggaaagcttgaatcccggacatcgaatatttgagaagatggtgtcaggaagatacttaggggagatagtaagaagagtgttactaaaaatgtctgaagaatctgctctctttggagatacactacctccaaaactcacaattccttacattttatggtctccagatatggctgcaatgcatcaagatatatccgaagaacgggagactgtaaacaaaaagctcaaggaagttttcggtataatggattcaactcttgcggcgagagaagttgtagttgaagtatgcgatgtagtcgcggaacgagcggctcgtttagcgggagcaggaatagttgggatgataaagaagcttggaagattagagaagaaaatgagcattgtgatagttgaaggaggattgtatgatcattatagggtatttagaaactatcttcatagcagcgtttgggaaatgcttggtgatgagttatcagatcacgtcgtcattgagcattctcacggtggatctgctgccggagctctcttccttgccgcatgtggcgacggtcatcaagattctgaaagcaagtga

SEQ ID NO: 22 - protein, 488 aa, Arabidopsis thaliana
  AtERDL4 (At1g19450)
MSFRDDNTEEGRNDLRRPFLHTGSWYRMGSRQSSMLESSQVIRDSSISVLACVLIVALGPIQFGFTCGYSSPTQAAITKDLGLTVSEYSVFGSLSNVGAMVGAIASGQIAEYVGRKGSLMIAAIPNIIGWLSISFAKDTSFLYMGRLLEGFGVGIISYTVPVYIAEIAPQTMRGALGSVNQLSVTIGIMLAYLLGLFVPWRILAVLGVLPCTLLIPGLFFIPESPRWLAKMGLTDDFETSLQVLRGFETDITVEVNEIKRSVASSSKRSAVRFVDLKRRRYYFPLMVGIGLLALQQLGGINGVLFYSSTIFESAGVTSSNVATFGVGVVQVVATGIATWLVDKAGRRLLLMISSIGMTISLVIVAVAFYLKEFVSPDSNMYNILSMVSVVGVVAMVISCSLGMGPIPWLIMSEILPVNIKGLAGSIATLLNWFVSWLVTMTANMLLAWSSGGTFTLYALVCGFTVVFVSLWVPETKGKTLEEIQALFR

SEQ ID NO: 23 - protein, 487 aa, Arabidopsis thaliana
  AtERDL6 (At1g75220)
MSFRDDNEEARNDLRRPFIHTGSWYRMGSRQSSMMGSSQVIRDSSISVLACVLIVALGPIQFGFTCGYSSPTQAAITKDLGLTVSEYSVFGSLSNVGAMVGAIASGQIAEYIGRKGSLMIAAIPNIIGWLCISFAKDTSFLYMGRLLEGFGVGIISYTVPVYIAEIAPQNMRGGLGSVNQLSVTIGIMLAYLLGLFVPWRILAVLGILPCTLLIPGLFFIPESPRWLAKMGMTDEFETSLQVLRGFETDITVEVNEIKRSVASSTKRNTVRFVDLKRRRYYFPLMVGIGLLVLQQLGGINGVLFYSSTIFESAGVTSSNAATFGVGAIQVVATAISTWLVDKAGRRLLLTISSVGMTISLVIVAAAFYLKEFVSPDSDMYSWLSILSVVGVVAMVVFFSLGMGPIPWLIMSEILPVNIKGLAGSIATLANWFFSWLITMTANLLLAWSSGGTFTLYGLVCAFTVVFVTLWVPETKGKTLEELQSLFR

SEQ ID NO: 24 - protein, 463 aa, Arabidopsis thaliana
  AtERDL7 (At2g48020)
MSKASDAVREPLVDKNMAGSKPDQPWMVYLSTFVAVCGSFAFGSCAGYSSPAQAAIRNDLSLTIAEFSLFGSLLTFGAMIGAITSGPIADLVGRKGAMRVSSAFCVVGWLAIIFAKGVVALDLGRLATGYGMGAFSYVVPIFIAEIAPKTFRGALTTLNQILICTGVSVSFIIGTLVTWRVLALIGIIPCAASFLGLFFIPESPRWLAKVGRDTEFEAALRKLRGKKADISEEAAEIQDYIETLERLPKAKMLDLFQRRYIRSVLIAFGLMVFQQFGGINGICFYTSSIFEQAGFPTRLGMIIYAVLQVVITALNAPIVDRAGRKPLLLVSATGLVIGCLIAAVSFYLKVHDMAHEAVPVLAVVGIMVYIGSFSAGMGAMPWVVMSEIFPINIKGVAGGMATLVNWFGAWAVSYTFNFLMSWSSYGTFLIYAAINALAIVFVIAIVPETKGKTLEQIQAIVNP

SEQ ID NO: 25 - protein, 739 aa, Arabidopsis thaliana
  AtTST2 (At4g35300)
MSGAVLVAIAAAVGNLLQGWDNATIAGAVLYIKKEFNLESNPSVEGLIVAMSLIGATLITTCSGGVADWLGRRPMLILSSILYFVGSLVMLWSPNVYVLLLGRLLDGFGVGLVVTLVPIYISETAPPEIRGLLNTLPQFTGSGGMFLSYCMVFGMSLMPSPSWRLMLGVLFIPSLVFFFLTVFFLPESPRWLVSKGRMLEAKRVLQRLRGREDVSGEMALLVEGLGIGGETTIEEYIIGPADEVTDDHDIAVDKDQIKLYGAEEGLSWVARPVKGGSTMSVLSRHGSTMSRRQGSLIDPLVTLFGSVHEKMPDTGSMRSALFPHFGSMFSVGGNQPRHEDWDEENLVGEGEDYPSDHGDDSEDDLHSPLISRQTTSMEKDMPHTAHGTLSTFRHGSQVQGAQGEGAGSMGIGGGWQVAWKWTEREDESGQKEGGFKRIYLHQEGFPGSRRGSIVSLPGGDGTGEADFVQASALVSQPALYSKDLLKEHTIGPAMVHPSETTKGSIWHDLHDPGVKRALVVGVGLQILQQFSGINGVLYYTPQILEQAGVGILLSNMGISSSSASLLISALTTFVMLPAIAVAMRLMDLSGRRTLLLTTIPILIASLLVLVISNLVHMNSIVHAVLSTVSVVLYFCFFVMGFGPAPNILCSEIFPTRVRGICIAICALTFWICDIIVTYSLPVLLKSIGLAGVFGMYAIVCCISWVFVFIKVPETKGMPLEVITEFFSVGARQAEAAKNE

SEQ ID NO: 26 - protein, 503 aa, Arabidopsis thaliana
  AtVGT1 (At3g03090)
MGFDPENQSISSVGQVVGDSSSGGITAEKEPLLKENHSPENYSVLAAIPPFLFPALGALLFGYEIGATSCAIMSLKSPTLSGISWYDLSSVDVGIITSGSLYGALIGSIVAFSVADIIGRRKELILAAFLYLVGAIVTVVAPVFSILIIGRVTYGMGIGLTMHAAPMYIAETAPSQIRGRMISLKEFSTVLGMVGGYGIGSLWITVISGWRYMYATILPFPVIMGTGMCWLPASPRWLLLRALQGQGNGENLQQAAIRSLCRLRGSVIADSAAEQVNEILAELSLVGEDKEATFGELFRGKCLKALTIAGGLVLFQQITGQPSVLYYAPSILQTAGFSAAADATRISILLGLLKLVMTGVSVIVIDRVGRRPLLLCGVSGMVISLFLLGSYYMFYKNVPAVAVAALLLYVGCYQLSFGPIGWLMISEIFPLKLRGRGISLAVLVNFGANALVTFAFSPLKELLGAGILFCAFGVICVVSLFFIYYIVPETKGLTLEEIEAKCL

SEQ ID NO: 27 - protein, 503 aa, Arabidopsis thaliana
  AtVGT2 (At5g17010)
MALDPEQQQPISSVSREFGKSSGEISPEREPLIKENHVPENYSVVAAILPFLFPALGGLLYGYEIGATSCATISLQSPSLSGISWYNLSSVDVGLVTSGSLYGALFGSIVAFTIADVIGRRKELILAALLYLVGALVTALAPTYSVLIIGRVIYGVSVGLAMHAAPMYIAETAPSPIRGQLVSLKEFFIVLGMVGGYGIGSLTVNVHSGWRYMYATSVPLAVIMGIGMWWLPASPRWLLLRVIQGKGNVENQREAAIKSLCCLRGPAFVDSAAEQVNEILAELTFVGEDKEVTFGELFQGKCLKALIIGGGLVLFQQITGQPSVLYYAPSILQTAGFSAAGDATRVSILLGLLKLIMTGVAVVVIDRLGRRPLLLGGVGGMVVSLFLLGSYYLFFSASPVVAVVALLLYVGCYQLSFGPIGWLMISEIFPLKLRGRGLSLAVLVNFGANALVTFAFSPLKELLGAGILFCGFGVICVLSLVFIFFIVPETKGLTLEEIEAKCL

SEQ ID NO: 28 - protein, 241 aa, Arabidopsis thaliana
  AtSWEET17 (At4g15920)
MAEASFYIGVIGNVISVLVFLSPVETFWKIVKRRSTEEYKSLPYICTLLGSSLWTYYGIVTPGEYLVSTVNGFGALVETIYVSLFLFYAPRHLKLKTVDVEAMLNVFFPIAAIVATRSAFEDEKMRSQSIGFISAGLNIIMYGSPLSAMKTVVTTKSVKYMPFWLSFFLFLNGAIWAVYALLQHDVFLLVPNGVGFVFGTMQLILYGIYRNAKPVGLSNGLSEIAQDEEEGLTSRVEPLLS

SEQ ID NO: 29 - protein, 441 aa, Arabidopsis thaliana [sequence omitted]

SEQ ID NO: 30 - protein, 343 aa, Arabidopsis thaliana
  AtFrcK1 (At5g51830)
MGEDAISGNLKNLTIDTRDSETLVVCFGEMLIDFVPTVGGVSLAEAPAFKKAPGGAPANVAVGVSRLGGSSAFIGKVGDDEFGRMLADILRLNNVDNSGMRFDHNARTALAFVTLRGDGEREFLFFRHPSADMLLLESELDKNLIQKAKIFHYGSISLIEEPCRSTQLVAMKIAKAAGSLLSYDPNLRLPLWPSEEAARKEIMSIWNLADVIKISEDEITFLTGGDDPYDDDVVLQKLFHPNLKLLVVSEGPNGCRYYTQEFKGRVGGVKVKPVDTTGAGDAFVSGLLNSLASDLTLLKDEKKLREALLFANACGAITVTERGAIPAMPSMDAVQDLLSSTRS

SEQ ID NO: 31 - protein, 325 aa, Arabidopsis thaliana
  AtFrcK2 (At2g31390)
MASNGDKGLIVSFGEMLIDFVPTESGVSLAEAPGFLKAPGGAPANVAIAVSRLGGRSAFVGKLGDDEFGHMLAGILRKNGVDDQGINFDTGARTALAFVTLRADGDREFMFYRNPSADMLLRPDELNLDLIRSAKVFHYGSISLIVEPCRSAHLKAMEVAKEAGALLSYDPNLREPLWPSKEEAKTQIMSIWDKAEIIKVSDVELEFLTGSNKIDDETALTLWHPNLKLLLVTLGEKGCRYYTKTFKGAVDPFHVNAVDTTGAGDSFVGALLNQIVDDRSVLEDEERLRKVLRFANACGAITTTKKGAIPALPSDAEVRSFLEKK

SEQ ID NO: 32 - protein, 384 aa, Arabidopsis thaliana
  AtFrcK3 (At1g66430)
MALQATTTTFCFSGPTFRSTPHSLTSKRPISIKATTSSPSRLSNSRSNLKGRALSSDGSTQESPYVVCFGEMLIDFVPTTSGLSLADAPAFKKAPGGAPANVAVGIARLGGSSAFIGKVGEDEFGYMLANILKDNNVNNDGMRFDPGARTALAFVTLTNEGEREFMFYRNPSADMLLEESELDFDLIKKAKIFHYGSISLITEPCKSAHISAAKAAKEAGVILSYDPNLRLPLWPSADNAREEILSIWETADIIKISEEEIVFLTKGEDPYDDNVVRKLFHPKLKLLLVTEGPEGCRYYTKDFSGRVHGLKVDVVDTTGAGDAFVAGILSQLANDLSLLQDEERLREALMFANACGALTVKVRGAIPALPTKEAVHEALLKAVV

SEQ ID NO: 33 - protein, 324 aa, Arabidopsis thaliana
  AtFrcK4 (At4g10260)
MANTPLIVSFGEMLIDFVPDTSGVSLAESTGFLKAPGGAPANVACAITKLGGKSAFIGKFGDDEFGHMLVNILKKNGVNSEGVCFDTNARTALAFVTLKKDGEREFMFYRNPSADMLLKESELNKDLIKKAKIFHYGSISLISEPCRTAHMAAMKTAKDAGVLLSYDPNVRLPLWPSTEAAIEGIKSIWNEADIIKVSDDEVTFLTRGDAEKDDVVLSLMHDKLKLLIVTDGEKGCRYYTKKFKGRVPGYAVKAVDTTGAGDSFVGAFLVSLGKDGSILDDEGKLKEALAFANACGAVCTTQKGAIPALPTPADAQKLMKSKSK

SEQ ID NO: 34 - protein, 329 aa, Arabidopsis thaliana
  AtFrcK5 (At1g06030)
MTSSNGDNKGLVVSFGEMLIDFVPTESGVSLSESSGFLKAPGGAPANVAIAVSRLGGRAAFVGKLGDDEFGHMLAGILRKNDVDDQGINFDKGARTALAFVTLRSDGEREFMFYRNPSADMLLRPDELNLELIRSAKVFHYGSISLITEPCRSAHMKAMEVAKEAGALLSYDPNLREPLWPSPEEARKQIMSIWDKADIIKVSDVELEFLTGNKTIDDETAMSLWHPNLKLLLVTLGENGCRYYTKDFHGSVETFHVDAVDTTGAGDSFVGALLNQIVDDQSVLEEEERLRKVLRFANACGAITTTKKGAIPALPTDCEALSFLKIQVE

SEQ ID NO: 35 - protein, 326 aa, Arabidopsis thaliana
  AtFrcK6 (At3g59480)
MAASNGEKSLIVSFGEMLIDFVPTVSGVSLADAPGFIKAPGGAPANVAIAISRLGGRAAFVGKLGDDEFGHMLAGILKQNGVSAEGINFDTGARTALAFVTLRSDGEREFMFYRNPSADMLLRPDELNLDVIRSAKVFHYGSISLIVEPCRSAHLKAMEVAKEAGALLSYDPNLRLPLWPSKEEAQKQILSIWDKAEVIKVSDEELMFLTGSDKVDDETALSLWHSNLKLLLVTLGEKGCRYYTKSFRGSVDPFHVDAVDTTGAGDSFVGALLCKIVDDRAVLEDEARLREVLRLANACGAITTTKKGAIPALPTESEVQSLLKGN

SEQ ID NO: 36 - protein, 345 aa, Arabidopsis thaliana
  AtFrcK7 (At1g06020)
MASSTGEKGLIVSFGEMLIDFVPTVSGVSLSESPGFLKAPGGAPANVAIAVSRLGGRAAFVGKLGDDDFGHMLAGILRKNGVDDQGINFDEGARTALAFVTLRSDGEREFMFYRNPSADMLLRPDELNLELIRSAKVFHYGSISLITEPCRSAHMKAMEVAKEAGALLSYDPNLREPLWPSPEEARTQIMSIWDKADIIKVSDVELEFLTENKTMDDKTAMSLWHPNLKLLLVTLGEKGCTYFTKKFHGSVETFHVDAVDTTGAGDSFVGALLQQIVDDQSVLEDEARLRKVLRFANACGAITTTKKGAIPALPTDIEALSFLKDQKKRQTNLKFSKWCCTASPC

SEQ ID NO: 37 - protein, 471 aa, Arabidopsis thaliana
  AtFrcK8 (At3g54090)
MASLLIFPHLHHFDSSLDRREVLVVRHSQASRRFLTPKASINGSGITNGAAAETTSKPSRKGRKKKQTSTVIEKDNTETDPELNPELADYDDGIEFPYDDPPLVCCFGAVQKEFVPVVRVHDNPMHPDMYSQWKMLQWDPPEFGRAPGGPPSNVAISHVRLGGRAAFMGKVGEDDFGDELVLMMNQERVQTRAVKFDENSKTACTRVKIKFKDGKMMAETVKEPPEDSLFASELNLAVLKEARIFHFNSEVLTSPTMQSTLFTAIQWSKKFGGLIFFDLNLPLPLWRSRNETRKLIKKAWNEANIIEVSQQELEFLLDEDYYERRRNYTPQYFAEDFDQTKNRRDYYHYTPEEIKSLWHDKLKLLVVTDGTLRLHYYTPTFDGVVIGTEDVLITPFTCDRTGSGDAVVAGIMRKLTTCPEMFEDQDVMERQLRFAVAAGIIAQWTIGAVRGFPTESATQNLKEQVYVPSMW

SEQ ID NO: 38 - protein, 614 aa, Arabidopsis thaliana
  AtFrcK9 (At1g69200)
MASLSFTQFLSFPRCNADVPCLLQSHGFVKFRGERWNGKQSFSMAAGRRKLSESAPLEEEGNDGNGAVVGKKPSKSVKRTTKKKVVVKDEPLEEISEFLVDNDDVLDKESIVSALKPKKTRTRKKAAAASSDVEEVKTEKKVRRKRTVKKDKDVEDDLATIMDAEVSDVEEALAVESTDTESEEEEIDLSKHEGEDISHTYGWPPLVCCFGSAQHAFVPSGRPANRLLDYELHERMRDAKWAPEKYIRAPGGCAGGVAIALASLGGKVAFMGKLGADDYGQAMLYYLNVCKVQTRSVKIDGKRVTACSTMKISKRGRLKSTCIKPCAEDSLSKSEINVDVLKEAKMFYFSTHSLLDKKMMSTTIQAIKISKQLGNVIFYDLNLPLPLWHSSEETKSFIQEVWNLADVIEITKQELEFLCGIEPTEEFDTENNDISKFVHYPPETVEQLWHENLKVLFVTNGTSKIHYYTKEHNGAVSGMEDVPITPFTRDMSASGDGIVAGLIRMLTVQPDLMNNKGYLERTARYAIECGIIDQWLLAQTRGYPPKDDMEEEEDDEEEDEVESDPNGIRSITEKEYRTSKPYDEPDGPYVMKPVEEREYKKLELVGSMFEDGSL

SEQ ID NO: 39 - DNA, 1473 bp, Beta vulgaris
  BvERDL4;1 (BvIMP; Bv1_015950_zugk.t1)
atgagttcagattcagaagcaggtttaggaggaggaggaggagatctgcggaaaccatttttgcatacaggaagttggtatagaatgggttccagacaatcaagtttgatgggttcttctcaagttattcgagaaagctccatctctgtccttgcttgtgttcttattgttgctcttggtcctattcagtttggttttactgctggttattcatctccaactcaatcagcaattacaaatgaacttggtctttctgttgcagagtactcatggtttggttctctatccaatgtgggtgccatggttggggcaattgcaagtggtcaaatatctgagtatattggaagaaaagggtctttgatgattgctgctatccccaacataattggatggcttgctatatcatttgccaaagattcttcatttctgtatatgggaaggatgttggaaggttttggcgtgggaataatatcttacacggttcctgtgtacatttctgaaatagcaccacagaatttgaggggagctttgggttcagtaaaccagctatccgttacaatcggtataatgctatcgtatatgctggggctttttgtcccgtggaggatacttgcagttttaggaattttaccatgcactatattgatacctggcttattcttcataccggaatctcctaggtggttggcgaaaatgggtatgatggaagaatttgaggtttccttgcaagttctccggggctttgacactgatatatctcttgaagttaatgaaatcaagagatctgttgcttcaagtagcaaaagaaccaccataagatttgcagaactacgacaaagaagatattggttacccttgatgatagggaatggtttacttattttgcaacaactcagtggaatcaatggtgtcctgttctattctagtaccatctttaaagaggctggggtcacatcaagcaacgctgcaacatttggccttggtgctgttcaggttatcgcaactgttgtgactacctggttggtggataaatcaggacgcagacttcttctaattgtctcttcttctgggatgacattgagtcttctagtggtcgcaatgtccttctttttaaaggaaatggtatcagacgaatctacatggtacagtgtattctccatcctttcagttgttggagttgtggctatggtggttactttctcactaggaattggagcaattccgtggattataatgtcagagattcttccaattaacatcaaggggctggctggaagtattgctacacttgccaactggtttgtagcatggattgtgacaatgactgcaaacataatgttgtcatggaatagtggaggtactttctctatttacatggttgtttgtgctttcactgtggcctttgtggtcatttgggtccccgagacaaaggggagaacattggaggagattcagtggtccttcagaagataa

SEQ ID NO: 40 - DNA, 1509 bp, Beta vulgaris
  BvERDL4;2 (BvIMP2; Bv6_128840_qhip.t1)
atgagtagcagtgatgcggaggatgcgagggcggagctccgaaaaccgtttcttcatacgggtagttggtatcggatgagtacgggtggtggaaaagatccgattagtagtggtagtatgatgatgggttcaagacaatctagtattttcgggtctattgctaatatgcgtgaatccgccatttccattgttttctgtgtttttgttgttgctttgggtcccatccaatttggtttcacctgtgggtattcatccccaactcaatccgacatcattaaggatcttgaccttaaagtttccgagttctcattgtttggatcattggctaatgtgggagcaatggtgggggcaattgcgagtggacagatttctgaatacattggaagaaaagggtcattaatgatcgcctcaatccctaacattataggatggcttgtcgtttcatttgcgagggatgtctcgtttctttacatgggacgcctgctggaaggttttggtgttggcattatttcctacacggtgcctgtttatatagccgaaatagcacctcaaaacatgaggggaatgcttggatcagtgaaccagcttgctgttaccattggcataatgatcgtttacctgttgggaatttttgttgagtggagagcacttgcaatcattggaatcctaccttgcgctgcgttgatacctggattgtttttcataccagaatctcctcgctggctggcaaaaatggggatgatggaagaatgtgaagcgtctttgcaagttctgagaggattcgatacagatatctcgattgaaatgaatgaaatcaaaaaatctgtgggatcatccagcaaaagaacaacaattagcatttcacatctcaagagaaaaagatattggttcccattgatgttaggaatcggattacttttgcttcagcagctctgtggtattaatggaatattgttctactcccgcaccatatttgaaatggcaggaatatctgagggtgctgtcgccacatttggtcttggaagcattcaggtggttgctactggagttgccacttggctgatggacagggctggccgaagggttcttcttatagtatcctctgttggaatgactgctagcctcctcctagtttcagtcgcattttatctggagaccatcgtaccaaaagactcggcattgcacagcacgttgggcattctctctgtcgtaggcctcgtggcaatggtggtttccttttctttgggaatgggacccattccttggcttataatgtctgagatacttccagctagtataaaaggccttgctggcagtgtagcaacaatggcgaactttctaacttcctggggtgtcactatgactgcaaacttgctgctcggctggagtagcggaggaacctttacaatttacacattttttgctgcttttactgtgatatttgtggctgcatggcttccggagacaaaaggaaagacgctcgaggagattcaagcatacttcagataa

SEQ ID NO: 41 - DNA, 2208 bp, Beta vulgaris
  BvTST2;1 (Bv5_115690_zuju.t1)
atgagtgcagcagtattagttgcaattgctgcaacagttggagatttgctgtatggatgggataatgctactattgctggggctgtattatatattaagaaagagttcaacttggagagttctccaaccttggaagggttaattgtggccacatcaataattggagccactcttattacaacatgttctggaccgattgcagatcgtcttggtcgtcgccctatgatgataatttcctcagtttgtttctttgttagtgccttaataatgttgtggtctcccaatgtttatgttttactcttcggtcggctattagatggatttggaagtggtttggcagtcactcttggtcctctttatatatcagagaccgctccaactgatataagaggctcactgaacacacttcctcagtttactggttctggtggaatgttcctcgcatactgcatggttttcgggatgtcattgatggaaacacctagctggagattaatgcttgggattctttttgttccatctactgtttattttctattaactgtattcttcttacctgagtctcctcgctggcttgttagcaaaggacggatgaatgaggctaaaaaggttcttcaatggttgcgaggcagggaagatgtctttgctgagatggctctccttgttgagggtcttagagttggaggtgatacatcaatagaggaatacttgattgagccagatgctggactcgctgaggatcaagatccgatgactgtcaaagatcaggttaggctgtatgggtccgaagcaggctgctcctgggttgccagaccagtcactggtcagagtatgctgggtattgcatctcggcagggaagcatgcagagtcctagtgttcctttaatggatccccttgtaactctttttggtagtgtacatgaaaagcttccagaacaaggaagtatgcttagtgtcatattcccaacttttggtagtatgtttagtatgggagggaaagagcccaaaaatgaagagtgggatgatgaaaatactattggggatgatgatgattatggtcatgacgatgaagattatgcaggtgatgctgatgaagatgacaatttacgtagttcacttatatctcgtcaggatacaggtccagacaaagccatggttgctcctacttcaggtagcatgttcagcatgaagcatagtagttggttacaaggaagcgaagctagtggtattggtggtggttggcagttagcttggaaatggagcgagagagaaggcttggatggtacgaaggaaggaggattcaaaagactttatctacatcaggaaggtgatgctggatctaaacgaggctctgttatttctcttgctggtggtgaggttattggcgacaatgagtatgtgaaggctgctgcactagtaagtcaacctgccctttattcgagggatttcatggatcgggatagtattggtccagctatggttcacccttccgaggcttctgcaaaaaggcctagttggagggattttttagagcctggtgtcaggcgtgcattagttgttggtgtcggacttcaacttcttcaacagttcgctgggataaatggcgttctgtattatactcctcaaatactagagcaagctggggtgggtgatcttctttcgcatatgggtataggcgcttcctctgcattgttactcatcagtgcactcacaactcttttgatgcttcctgctatagctgttgcaatgaggcttatggatctttctgggagaaggactttgctactaaccacaattccggtgttgttcttatcgctcgttgtcttaatactcgcaaatgtcataaagatgaacaccactgtgtatgcagtggtctccacagtcgcggtagttctctacttctgcttctttgtgatggggtttgggcctatcccaaatatcctatgtgcagaaattttcccaaccaagattcgtggagtctgtattgctatttgtgcacttactttctggatctgtgatatcatagtcacctacacactccctatgatgcttaaagctgttggacttgctggtctctttggcttctatgctgttgtgattttaattgcatggatatttatatttttgaaggttcctgaaaccaagggcatgccccttgaggtaatcactgagttctttgctctcggtgcaagacaagcaagccactga

SEQ ID NO: 42 - DNA, 2220 bp, Beta vulgaris
  BvTST2;2 (Bv9_215730_jzcj.t1)
atgagtggagcggtattagttgcaattgctgcggcagttgggaatttactacaaggatgggataatgctactattgctggggctgtgttgtatattaagaaagaattcaacttggagggcgcgccaaccatggaaggcttaattgtggccatgtcacttattggagccactattatcacaacatgctctggaccagtttcagatcgctttgggcgtcgccctatgatgataatctcctctatatgtttcttttttagtgccctaataatgttgtggtctcccaatgtttatgtcctactcttgggtcgattattagatggatttggaagtggtttggctgtcactcttgttcctctttatatatcagagacagctccaactgatataaggggttcattgaatacacttcctcaatttactggttcgggtggaatgtttgttgcgtactgtatggtgtttgggatgtctttaatggaaaaacctagctggagattgatgcttgggattcttgttgttccatctgctctttattttgcattaactgtattcttcttacccgagtctcctcgatggcttgttagtaaaggacgaatgaatgaggccaaaaaggttcttcaacgattgcggggcagggaagatgtctctgctgagatggctctgcttgttgagggtcttggagttggaggtgacatatcaatagaagaatacttaattgagccagatgttggcatcagcgaggaatatgatccgatggctgccaaagatcagattaaattatatgggtcagatgcaggccactcttgggttgccagaccagtcaccggccagagtatgctgggccttgcatctcgtcagggaagcattcagaaccctagtgttcccttaatggaccccctggtcacgcttttcggtagtgtacatgagaagcttccagaacaaggaagcatgcgaagtattattttcccgacttttggtagtatgtttagtatgggaggcaaagaccctagaaatgaagagtgggatgaggagaatcttcatggggatgatgatgattatgcccataatgatgatgacaatgatgattatgctgaagatgatgacaatttacatagtccacttatatctcgtcaggctacaggtacagacaaagctatggttgctccagtttcaggtagcatgttcagcatgaaacctagtggtttaatacaaggaactgaagctagtggaattggtggtggttggcagctggcttggcaatggagtgagaaagaaggtgcagatgggaggaaggagggaggattcaaaagactttacttacatcaggaaggtgatatggtatctaaacgaggatctgtaatctctcttcctggcggtgatgttactggagagacagagtatatgaaggctgctgcactagtgagtcaacctgccctctattcgagggagttgatgaatcagcatactattggaccagctatggttcatccttctgagactgctgcaaaagggtctagctggagggaccttttagaacctggtgtcaggcgtgcattgattgttggtgtcgggctccaacttcttcagcagttttctggtataaatggggttctgtattacactcctcaaatactagagcaagctggggttggtgatcttctttcaaacatgggtattggcgcttcctctgcatcattgctcatcagtgcactcacaactcttttgatgcttccttccatagctgttgcaatgaggcttatggatatttccgggaggaggactttgctgcttaccacaattccggtgttgttcctttcgctcgtcgtcctaatactcggaaatatcataaagatgagcactactgtgcacgcagtgatctcaacagtctccgtagttctctacttctgcttctttgtgatgggctttggcccaatcccaaatatcctatgcgcggaaattttcccaaccaggattcgtggtgtctgcattgctatttgtgcacttaccttttggatcggagatattatagttactgacacacttcctataatgctcaatgctgttggacttgctggtgtctttggcttctatgctgtcgttagtgtaattgcttggatttttatctttctaaaggttcccgaaaccaagggcatgcctctcgaggtcattactgagttctttgctctcggggcaagacaaccttctgaagacaaggacaactga

SEQ ID NO: 43 - DNA, 1509 bp, Beta vulgaris
  BvVGT1 (Bv3_049950_gzcg.t1)
atggcttcctctactaccgatcatcaacaccatgttctttcctcttttggaaaggcttcaggtgaatttgatcttgatgaagtagagcgaccgcttttaaatggagctcatcctactgaggattactctcttctttcctgcattgtgccatttttattccctgctcttggaggactactttttggttatgatattggtgccacatcatctgccacactttcaattcagtcaccgactcttagtggaactacatggtatgacttgagttctgttgaagttggccttattagcagtggctcattgtatggagctctaattggttctgtcttggccttcaatgttgctgatttccttgggaggaggaaagagttgatcgcagccgccatattttatcttgccggagctctaattacagcaataggtccgaacttcgtgatcatgatgataggacgctttatatttggcattggtataggactggcaatgcatgctgcgccaatgtacattgctgaaactgctccatctcatataagaggccgattaatctccctgaaagagtttttcatagtcatcggcatggttattggttatgccattgggagctttctagtgaatgttattgctggttggcgctatatgtatgggttgagttctcctctatcagtgataatggcaattgggatgtggtggctcccagattctcctagatggctacttttgtgtgctatacaaggaaaaggaaatgtgccagatttaagggagaatgccattagttgcatgtgtcgtcttagagggcgagctgtcagtgatacagcttcccagcaagtggatgagatcatggctgaactttctcttgctggtgaacttaataatgtatctacaactgagatgtttagaggaaaatacttgaaagctctggttattggctgtggtttagttttatttcagcagataacaggtcaaccaagtgtcctgtactatgctgcttctatcttgaaaagtgcaggattttctgcagcatctgatgcgacaagggtctcaattctgcttggcttttttaagctaattatgactggagttgctgttctagttgttgataaacttgggagaaggcctttactacttggtggtgtatctgggatggttatctctttgttgttccttggagcttattacactttcctcggtgatgcaccagctatagccgtcgttggtctactcctatatgttggctgttaccagttatcgtatggtccgattggctggttaatgatttcagaaattttccccttgcgcatgagaggaagaggaataagtttagcagtgctcatgaattttggagcaaatgctttggttacttttgcattttctcccttgaaggatctcattggagccggagctgtgttctttatgtttggtggcatagctgtcctgtctctcgtattcatattctttataataccggagaccaagggattgactctcgaggaaattgaggccatgttgtaa

SEQ ID NO: 44 - DNA, 1509 bp, Beta vulgaris
  BvVGT2 (Bv7_173330_nupg.t1)
atgatgggaaattcttcaatttatagtcttgaaacttctttattgcatcataaagttaatgcccagaaagaggattacccagttgaccaaactactgttgaagaagaggtctttgcttggtcttctgtaattttgccgtttttattccctgcactaggcggtttgctgtttgggtatgatattggtgctacttctggagctacgatatcactacagtctcctgagcttagtggtacaacatggttcaatctttcggcagttcaacagggtttagtggtgagcggctcactttatggagctctttttggttctatcatggtctttccgatagctgacttccttggaaggaggcgagaacttctaattgctgcaactctttatgcgattggcggcctcactactgcatttgctcctggccttgaagttcttttgtttgggaggcttatttatggccttggcattggctgggccatgcatgcggcccctctttacattgcagaaacttgcccttctcagattcgtgggactttaatttcgttgaaagaactcttcatagttcttggcattttgctgggtttctttgttggtagctttgaaatcgaggcagtaggaggatggcgttacatgtttgggttgagtgttccagttgctgcagttatgggtcttgggatgttcagtctccctccttctcctcgctggttgcttcttagggctgttcaaggtaaaggatctctgcaggagtataaggaaaaggctgttactgctctgagcaaactccgaggcagacctgctggtgataaagtttctgaaaagcaaattgatgacacactagtttcaatgaagtctgcttacgatcgggaatcagaagcaagctttttagaggtgttccaagggccaaatctgaaagcttttattattggtggaggtcttgtgctttttcagcagataactgggcagcctagtgttttgtattatgctggtcaaatcctacagagtgctgggttttctgctgcatctgatgccactcgagtttctgtgctaattggcctatttaagtttgttatgacaggagtagctgttcttaaagttgatgatcttggaaggaaaccattactaattggtggtgttagtgggatcactgtggctttattcctccttgctgcttactacaaatttcttggaggcctcccgtttgttgctgtagctgccttgcttctatacgtcggtagctatcaaatatcatttggaccgatcagttggctaatggtgtcagagatattcccccttcgcacgagaggacgaggaatcagtcttgctgttttaacaaactttggttcaaatgctcttgtgacctttgctttctcaccgttaaaggagttgcttggagctgataaccttttcctcctgtttggagtgattgctttgctatccctcgtatttgtgttgacgctcgtcccagagacaaaaggcttaagcttggaagaaatcgaggctaaattatcagaatga

SEQ ID NO: 45 - DNA, 672 bp, Beta vulgaris
  BvSWEET17 (Bv4_075980_knjf.t1)
atggataaactgagtttcattattggagttataggcaacataatctcagtgcttctcttcctttctcctttaaacactttcattcgaattgtgcggaaaaaatcgacagatggatttgaaagtatgccatatgtgtgcacattgctgagtacatgtttatggacttactatggaattataaggcctggggctcttcttgttgccactgtgaatgggtttggagctcttgtggagcttgtctatgtagctttattcatcacctttgctcctccaacaatgaaggctaaaactgccaaacttgcggcaattttggacgtgggatttcttggtgccgtaatactgatttcaaacttaatgttggaaggtgaaacgaggattaatatgataggtacaattggcgctggccttaacatcattatgtatggctctcctcttgtagccctgaaaacggtgataaaaactagaagcgtggaatatatgccttttttgttgtcattgttctcatttttgaacggaggaatatggacagtgtatgctgctcttgtcaaggatttctttcttctggtaccaaatgcgattggatttattcttggaacgattcagttagtggtctatgtttgttacatgaatccaagcaaagagcagcaatataatgagccccttatctattga

SEQ ID NO: 46 - DNA, 978 bp, Beta vulgaris
  BvFrcK1 (Bv3_066020_xjni.t1)
atgaagcatggtgaatcactggttgtttgttttggggaaatgttgattgattttgtgcccaccgttgccggggtctcgctggctgaagcacctgcattcgctaaagctgccggtggtgctcctgctaatgttgctgtgggaatctcacggttaggaggttcctccgctttcgttggaaaggtagggaaggatgagtttggcttcatgctagctgacattttgaagcaaaataaagtagataattcaggtatgagatttgaccccggggcaaggacagcactagcattcgttactttgagagccgatggagagcgtgaatttctctttttccgcaatccaagtgctgatatgctccttcatgaatccgagcttgataaagacctacttgaaaaggcgcaggtctttcactatggttcaattagtttgatagaggaaccttgcagatcagctcatcttgctgcactgacaattgtgaagaaggcaggtggtttcctttcgtatgatcccaatttgcgtaaacaattgtggccatcagaggaagctgctcgggatggcataatgagcatatgggaccaagcagatatgattaaggtaagtgaagacgaaataacattcttgactggaggtgatgacccatacgacgataatgttgttatgaagaaactctttcatcccaatcttaagctcttgatagtgactgaagggtcagaaggttgcagatactacactaagacgtttaagggcagggtttcaggcgtgaaagttaaacctgtggacacaactggtgcaggtgatgcatttgtgggaggcattctaagcaatttagcttctgacttgaatatattgaaggatgagaagaggttgagagaagctttgcattttgcaaatgcttgtggcgctgttacagttacgaagagaggggccattcctggtttaccaacaagagatgaagtccttgaaatcttgcaacaagcctga

SEQ ID NO: 47 - DNA, 996 bp, Beta vulgaris
  BvFrcK2 (Bv3_057460_dyyp.t1)
atggcggaacttaacaatggcggacattccaaaggattagtcgtaagcttcggcgagatgttaatcgacttcgtccctacatcttccggcgtttccctcgcagaagcgccgggattcctcaaagctcccggtggtgctccggcgaacgttgcgatcgctgtttctcgcctcggcggaaacgccgctttcgtcggaaaactcggtgacgatgaattcggacacatgctcgccggaatccttaagaaaaacggcgtttctgctgacggtttgagcttcgataaaggcgctagaactgcgcttgctttcgtcactttgaaatctgacggtgaaagagagttcatgttttaccggaaccctagcgccgacatgcttctcactcccgacgagcttaacctcgatctcattcgatcggctaaggtgttccattatggatcaattagcttgattgtggagccctgtagatcagcacatttgaaagcgatggaggaagccaaaaaggccggagctttgctttcatatgatccaaacctacggctgccattgtggccttctgcagaggaggctcgcgagcagatcatgagcatttgggataaggcagaggtgatcaaggtcagcgataacgagttggaattccttacaggaaactccacaatagatgatgctacagcaatgtcattgtggcaccctaacttaaagcttctcttggtcactcttggcgaccagggttgcagatactacaccaagaatttcaagggaagcttggatggatttaaggtgaatgcagttgacaccactggtgctggtgactccttcgttggtgcattgctaaacaagatcgtcgatgaccattctatcatcgaggacgaatcaagattgaaagaggtgttgaaattcgctaacgcatgtggagctattacaaccacgaagaagggagccatcccagcacttcctacagttgctgatgcgctagagcttattaagaagaacgcttcttaa

SEQ ID NO: 48 - DNA, 942 bp, Beta vulgaris
  BvFrcK3 (Bv2_027840_oqrd.t1)
atgcttattgattttgtgcccacaacaaatggggtttccttggctgaagcacctgcatttaaaaaggctgctggtggtgcccctgccaatgttgctgttggaatagctcgtcttggaggcaaatcagcattcattggcaaggttggtgaagatgaatttggctacatgcttgctaatattctgaaggagaacaatgtcaacaatgaaggaatgcgttttgatcctggtgctcgaactgctttagcattcgtgacattgaggagagatggggaacgtgaattcatgttttatcgtaatcctagtgctgacatgctccttcaggaatctgagcttgattttgagctcatcaggaaggcaaaaatatttcattatggctcaataagcttaatcacagaaccatgcaaatcagctcatattgctgctgctaaagctgcaaaagatgctggtgtgctactctcatacgatcccaacttaaggcttccattatggccatctgcagagagtgctcgtgatggaatcctcagcatctgggataccgctgacattatcaagataagtgaggaagaaatttcctttttaactcaaggagaagatccctatgatgataatgttgttcgtaagttataccatccaaacctcaaactactgcttgtgaccgagggagcagatggctgcaggtattacaccaaggattacagtgggaaagttgggggtttgaaggtagatgctgtagacaccacaggtgctggcgatgcctttgttgctggactgctatcccaactagctgctgactcaaacttgattcaggtggaggatcgattaagagatgcacttcaatttgccaacgcatgtggtgcattgactgttacagagcgaggtgcgattcctgctatgccaactcgagaagcagtgttgaatgtgatgctcaaatctgtagcttaa

SEQ ID NO: 49 - DNA, 936 bp, Beta vulgaris
  BvFrcK4 (Bv7_178860_gedd.t1)
atgctgattgatttcgtcccagatgaggctggtgtttcattggccgaatctcgcggtttcgtcaaagctcccggtggtgcacctgctaatgttgcctgtgccatcaccaagcttggtggcacatccgccttcattggaaaggttggggatgatgagttcgggaagatgctcgtagacataatcaagaagaacggtgttaacaccgaaggcgtgtgtttcgacaaagaggcaaggacagccttagcctttgtgacattgaagaagaacggtgaaagagaattcatgttctacaggaaccctagtgctgatatgctcctacaaacatcagagcttaatctagacctaatcaagcaagccaaggtattccattatggctcgatcagcttgatcactgagccatgcagatcagctcacattgcagccatgaaagccgccaaggaagccggggttaccctctcttatgaccctaatgtgagattacctctgtggtcttcccctgaggctgctagggagggtatcaagagcatttggaaccaagctgatatcattaaggtgagtgatgatgaggtagaatttttgacacaaggagatgcaaccaaggaagaagtgatcaagaccttgtggttcgacggtcttaaactactcctagtcactgacggagaaaagggctgcagatacttcaccaaggatttcaaaggatcagtgaaaggcttttctgtaaaggcaattgacacaacaggggctggagatgcatttgtgggctctttcctatattcccttgctaaagatccttcaatcttgcaggatgaaaacaagctaaaggaagcactgacattgtcgaacgcctgtggagcgatttgcacaacccagaagggtgccattcctgctctcccaagtctttctcaagcacaagatttggttaaacaaggaaactga

SEQ ID NO: 50 - DNA, 1446 bp, Beta vulgaris
  FrcK5 (Bv8_182100_hsoh.t1)
atggcaattcatctcctttcaccaattccttcttctttctctctctcctacaaaccctcctcacttttccctcccattttctcaaaaatttcaacctcttccaaaatcaaagcaacaactctcaacaaccctcaaaacgacatccaagaaccttcaaaacgacgtggtagaccaaagggaagcaaaaaatctaccactctctctcctcaaaaaacagctaaaatttcagatgggtcatcccaaaatacccaatctacaaatgggtcgaccttaaatttagatgaacttaacaatttcgatgatgggatggattttccttacttagaaccgccgctaatatgctgttttggtgcagttcaaaaggaatttttgccaacagtgagagtttcagaacagcaaatgcaccctgatatttactccgggtggaaaatgatgcagtggaatccacctgaatttgggcgggcacccggtggcccggcatcaaatgtggcgattgcgcacgttcgattgggcggaagagcagcatttatgggaaaagttggagatgatgattttggggaggatttggtttatatgatgaataaagagaaagtgcaaacaaggagtgtgaagtttgattctaatgtgaaaactggttgtacttttatgaagattaagtttagtgataatggtaagattaaaatggagttagttaaagaagctgctgaagattctttggttgcaactgaattggatttagctgtgcttaaagaggctaggatcttccacttcaattcagaagtcttgacatcgccttgtatgcacttatccctattcaaagctattaaaatatccaaattttttggaggtcttgtgttttttgatccgaatcttccattacccttgtggaaatcacgtgacgagacaagagaagttatcaaggaagcttgggaggaagccaatatcattgaggtaagcaggcaagagctggagtttcttttagacgaagaccattacgagaagaggagaaattaccggcctcaatactatgctgaagattatgaacagagtaaaaataggagggattactaccactacacacgtgaagagataactccattgtggcatgatgggctgaagtttctttttgtcacagatggaacctttaggattcattactataccccttcttttgacggtgttgtggttgggactgaagatgtgttaataaccccgttcacatgcgatagaactggatccggtgatgcaattgtggctggtattatgagaaaactgactagccaccctgagatgtatgaagatcaggatgttttggagaggcagcttcggtttgctattgctgcgggaattatatcacagtggacaattggcgcagtaaggggctttccaactgaaagcgccactcaaaatcttaaagagcaagtttatgttccatcaatgtggtag

SEQ ID NO: 51 - DNA, 1653 bp, Beta vulgaris
  BvFrcK6 (Bv6_136290_jzyk.t1)
atgctcgttgcagataatagattacggaatagatgggttttgtcagcaacatctaaaaaagcaattgtagcatctatacccgaggaggaggcatccactgaatcaaagggaaccaaaaaggctaggagtaggcaggccaacgcaagaggtagaaagaaggcaactactgaactgctggaccatgattttaatctattggctagtagttccatttcagaacaggagttctctgatctggaagcatctattagcgactctgagaaacccaagagaagaaccaggaagaaagttgtctctccaacttcgacttctggtatggaggaagtgaagacaaataaaaagtccagggggaggaagagcaaggaagagatcagtaaggttgaggatcaaacaagtgagatggaagtcaatgatttagaggaggtcgtctaccgtacaagtcaagataatgatgacagtgacattgatttacaattgggaaagagtgatggtgatgatattagtttcagttatggttggccccctcttgtttgttgctttggagcagcacagcatgcttttgtgccttcaggaaggcctgccaatagacttatagattatgaaattcatgattcacttaaagatgccttatgggaacctgaaaagtttgttagggctcctggaggttcggcaggtggtgttgcaatagcgctggcatcgctgggtggccgagtagcttttatgggtaaacttggcaatgatgactatgggcagacaatgctgtattacttaaatgtaaagaatgttcaaacacgatcagtttgtgtagatgataaacgtccaacagctgtttcacagatgaagattgccaagcggggcgctttacgaacaactactgtcaaaccttgtgcagaggattctttgtcaatatctgatatcaatattgatgtgttgaaggaggctaagatgttttatttgaatacatcctccttgcttgatgctagtatgagaagagcgactttgcgagcgcttaagatatcaaagaaattagggggtgtcatcttctatgatctgaatctcccattgtcactgtggcagtctgatgaagaaaccaaatctttcatagagcaagtgtggagccttgcagatgtcattgaagtcacaaagcaagaacttgaatttatttgtggaatcaagcctttagaggagtttgacaccaagaacaataagagatctaagtttgagcattatgaaccagatattatagctcctctatggcatgagaatctcaaagttttgtttgttacaaatgggacttctaagatacactattacaccaaagagcataatggtgctgtccttggagtggaagatgctccaatgtcccctttcacacaagatatgtcagcatctggagatggcatagtggcagctctcatgagaatgttgacagtgcaaccacatctcattacagacaaagagtacttagagcgtgcagttaaatatgcaattaattgtggagtcattgaccagtggattgtaactcggcaaaacggctttcctgctaaggaaggcctggaagaagaagatgaagacgaaggcattcctgacttaaatggcatcaggtctatcaccgagagacagttccgcactgtgatgcctgtttctagctga

SEQ ID NO: 52 - DNA, 1497 bp, Beta vulgaris
  BvHxK1 (Bv8_197580_aaut.t1)
atgaggaaggcagcggtgggtgcgacggttatatgtgcggcggcggtgtgtgcggcggcggcagtggtggtgcgtcaaaggatgaaaagttcaagtaagtgggctcgtgcaatggctatacttaaggagcttgatgaaaagtgtgagacacctttgggtaaattaagacaagtggcagatgctatgacagttgagatgcatgctggacttgcatcagagggtggttctaagcttaagatgttaatcagctatgttgataatcttcctactggggatgaacatggattgttctatgcattagaccttggtggcaccaactttcgagtactacgagtgaaattgggtggcaaagaaaaaggtgttgttcaacaagaatttgacgaagtgtcaattccacccgagttgatggttgggacgtcagaagaactgtttgattacatagctgctgcacttgctaaatttgttgcaacggaaggtgaaggtcttcatcctgaaccaaatagacagagagagctgggatttaccttctctttcccagttaaacagacatcaattgcatcagggactcttataaggtggaccaaaggcttcagcatagaagatacagttggtgaagacgtggtggccgaattgaccaaggccatgaaaagaaagggtgtagatatgcgtgtgacagctttggtcaatgatacagttggaaccttagctggaggtaggtatactaaaggaaatgtaattgctgctgtcatattgggtactggaacaaatgcagcttatgtagaacgtgctagtgcaattcctaagtggcatggtcctttgcccagatcaggggagatggttattaacatggagtggggcaatttccgttcatcgcacttgcccttgacagaatatgatattgcactagatgaagaaagtttgaatcctggtgaacagatctatgagaaaatgatatctggaatgtacttgggggagattgtgcgtagagtcttgtgtaagatggcagaagaggccagtttctttggtgatacagtcccaccaaaactgaaaactccattcatcttaaggacaccagacatgtctgccatgcatcatgacacatcacctgatcttaaagttgtcgctagcaaactgaaggatgtcttagggataccaaatacatcattgaaagtgagaaaggttatagttgacatatgtgacattatcgcttctcgtggggcctgcctttctgcagccgggatcttgggcattattaagaaactagggaaagacgcattgaagcaaggtgagaatcagaagtctgtgattgcattagatggagggttgtttgaacactacgccaagttccgagagtgcatggaggactctttgaaggaattactaggtgatgaaatcgctgacaccatcgtagtcgagcactcaaatgatggatcaggcatcggggctgctctcctagcagcatcgcattctcagtatcttgaggaagaagaatcttga

SEQ ID NO: 53 - DNA, 1542 bp, Beta vulgaris
  BvHxK2 (Bv9_224680_aote.t1)
atgggtaaggtggtaattgttgctacagtgttgggagctgcggtagtttgtgcagtaggggggttaattgtcagccgtcggatgaaaaatggggcaaattggaggcgtacgatggagatattgagggattttgaggagaaatgtgggaccccaattgagaaattgaagcaggtggctgatgccatggttatggaaatgcatgctggtcttgcttctgatgatggcagcagtattaagatgcttatcagctatgttgacaatctcccaactggagatgaggatggtttgttttatgcactggaccttggtggtacgaacttccgtgttcttcgagttcagttgggtggcaaagatggtggtatcaagcatcaggaatttgctgaagttccaatccccgtggaattgatgattggaacgtcagatgatctttttggttatattgctagtgaggttgcaaagtttatcgctcaagaaggtccagagtttcaacttccttctggtagagaaagggaacttggttttaccttttcattccctgtaatgcaaacatccattgactccggaactttgatcacttgggcaaaaggcttctcgatagatgatacggttggtaaggatgtagtggaagagttggcaaaagcattgaagaagcaaggtgttgatatgcatgtcacagctttggtaaatgatacagttggtacattagctggaggtcaattctcaaacaaagatgtcattgctgctgtgatattgggcacaggaacaaatgccgcatatgtcgaacgtgcagaggccatacctaaatggcgtggtccattaccgaaatcaggagagatggttatcaacatggaatggggcaacttccagacatcaaatcttccattgactgaatacgactatgctttggattatcacagtcctaacagtggtgagcagatttatgaaaagatgatttctggaatgtatttgggtgaaattgtacgtagagttctgtgccgaatggctgaagaagcttccttctttggtgataccattcccccaaaactgcatattccattcatcttgaggacacctgacatgtcagctatgcatcatgattcatcacccgatcttgagattgtaggctctacaatgaaggatatattagagataccaatgctttccctcaagaaaaggaaagtcatttacgacctctgcaaaattgtggcaacacgtggggctcgtcttgctgcagcgggaatttcggggattttgaagatagtgggaagagacacattgtcaagcaacgatgagaagcgaaaaagtgttatagccatggatggtggattatacgagcattatgaagaattccgaaaatgcctagagcacacattgaaagagcttctcggggataaagtctgggaaagaatctccattgagcatgctaatgatggttcgggaattggagctgctcttcttgctgcttctcactcccgctaccttgaggacaacgaaactcaagaagatattgtagttgttccagctatgctatcagatgattaa

SEQ ID NO: 54 - DNA, 1530 bp, Beta vulgaris
  BvHxK3 (Bv4_073320_tcog.t1)
atgggaaaagttggatttggtttagcggtaagtatagcggtggtaacttcggcagttgctgcggctgtggtggtaaaaagggtaaaaagtcggcgaaagtggcaaagagttgtgggtgttttgaaagaattagaagaatgttgtgggacccatgttagtagattaaaacaagttgttgatgctatggctgttgaaatgcatgctggtttagcctctgaaggtggttctaagctcaaaatgttgctcacttttgttgataaacttcctaatgggagtgagaagggaatatattatgcactagatcttggaggtactaattttagggtcttgcgggttcagctaggaggaagaagatccggcatcgttagacatgatgttgaaaggaagcccattcccgaacatttaatgactagcaccagtgaggatctgtttgatttcatcgcgacatcactaaaggacttttatggtcaagagaatgacaaaagttcagatctttctcctgtctcaagaaggaaacttggttttaccttttcttttcctgtaaagcaaatatcagtttcttccggaatcttgatgaaatggacaaaagggttttccattcgtgacatggtaggaagcgatgttagtgaatgtttgcaccaagcaatgtctagacagggactggatatgcatattgcagccttggttaatgattctgtgggaactttggcgcttggacattataatgacgaggacacggttgctgcagtgatcattgggactggaacaaatgcctgctattttgagcgggcagatgcgatcattaagtctcaaggtctccctacatcttcaggaggcatggttgtcaatatggagtggggtaacttttggtcgtcccatttgcctagaacatcttacgacatcgagttagatgcagagagccctaatccaaacgaccagggttttgagaaaatgatatctggaatgtacctgggtgagatcgtaagaagagtcatactaaggatgtccaaggagtctgacgtatttggacctatttcttctagcctatgtgaagctttcatcttgaggacgcctttaatgtcgacaatgcatgaagatgactctcctgacctagaagaagtagcaagaatattggaagaggttctcgggatttgtgatgtgcctttgaaagtccggaaacttgtagtgaacgtatgtgacgtggtaacccggcgagcagcccgtcttgcagctgccggcattgttgggatactgaaaaagatcggccgagatgggagtggtggggttgctagcagcagggccaaaggctcaagcagcagcaataggttaaagagaacagttgttgcagttgaaggcggcctatattcaaattacagaatgttcagggagtacttaaatgacgctgtggccgagatattgggggaggaaatcgccccctttgtaatcttaaaggtcactgaagatgggtcgggcatcggagctgccctgcttgcagccgcttattcatcacctgagactgtcgatacgtaa

SEQ ID NO: 55 - DNA, 1491 bp, Beta vulgaris
  BvHxK4 (Bv5_124820_xpum.t1)
atgtcaataccagcagcatcaacagccgttggatcactctgtttgccaagatcaaggatcaggtcttctgcattacagccaatgatggccgtccgatctggcactgtctcctctgtaactcaaatattaactaagttacaaaaagagtgtgcaacacctcttcctgtgttgcgccacgtggcagattccatgggtaatgatatgagagctggacttgctgttgatggtgcttctgatctcaagatgattcttagctatgttgatactctcccaactgggaatgagaaaggattgttctatgcattagatctcggtggaacgaacttccgagttttgagagtgcaattaggtggaatagatcaacgtgtaatcgctactgaagctcagcaagtttctattccacaggatttgatgttcggtacctctgaggaactctttgatttcattgcttctggtttggcaaaatttgctgaaaaggagagtggtgaattccaactcctgcaaggaagaaagagagaacttggattcacattttcttttccggtgaaacaaacatctataagttcaggaattctaatcaagtggacaaaaggttttgcggtttctggaacgtcaggaaaagatgtagtagcttgtttaaatgaagctatgcagcggcaagggctacaaatgcaagtctcagctctggttaacgatgcagtgggaactttagctggtgcgaaatattgggataacgatgtcatggtcgccgtgatcttgggaacaggaacgaatgcttgttacgttgagaggatagatgccattcctaaaatgcctggtcagaagtcacagtcaggaacaacaataatcaatactgaatggggtgcattttcaactggacttcccttgactgaatttgatagggaaatggatgctgaaagcatcaaccccggcgagcagatatttgagaaaacgatatcaggtatgtacctcggcgagatcgtgaggagggtattactaaagatggatgaagcaggttctctatttggcagtagcatgccagacaaactgcaaacaccattctcactcagaaccccgcatatatgtgccatacagcaggacacatcaaacaatttggatgaaattggctcaattctcttcaatgaggcaggagttgaagcaaaaacagaagcgaggcaaatagttctagaggtttgtgacacgatagcaaaaagaggtgggcgtttggctggtgcaggaattgtagggattctccacaagatggaagatgacatgaaaggtctaatttttggaaagcggactgttgtggcgatggatggaggcttgtatgagaattatcctcaatacagaaattatctccaggatgcagttacggagcttttaggacccgcattgtcagaaaatatagtcattgagcattccaaagacggttctggtatcggagcagctcttttagctgctgcaaattccaagtataaacatcatatctag

SEQ ID NO: 56 - DNA, 1401 bp, Beta vulgaris
  BvHxK5 (Bv9_224670_aurc.t1)
atgggtgatattgtaaatgtaaatgttggtgaaaatttgatggaaatggtgaagaagatagaagaagaattctgggtcccagctgagttgctgaaacaattggctgatgatatggaattgatgatgcgaaaaggtttagaagatgaacattcaagctccattaagatgcttgtttcttatgttgattcccttccttctggtgatgaagagggatgcttttatgcattggacttaggtgggacaaacctccgtgttatgcaagttaaactgcaagggaataggactattgacctcaaagccgaatcttatatggtgcctcctaagatgaaggtcgggacgttacatgaactttttgactatatagcagagagagtttctcatgtttttgaaacagaagaaaaccatgactttgaagatgttcctggtaagaggagggagcttggttttactttctcattcccagtgcaccagacgaggatcaactctgggactctccttaattggacaaaagactataatgcacaagatgccattggcaaagacatggtggaagagttaacaaaggctttggagaaacgagctattgatgttaatgtgactgctttgctcaatgatacagttggcactttggctggaggtagattttacgacaataatgttgttgcagctgtgattttgggtaccggaatgaatgctgcttatgtggaacagtctgaaaacattgtgaagccatatggtattccaccaaaatcaggacaaatggttattaacacagagtggggaaatttcaattcttcacttcttcctttaaccgactatgatcgtgcgttagacaatgatactccaaaccgccacaagcagattctagagaagatgctatctggtagatatttgggagaaattgtgcgaagaattttgcaacggttagctgaagatgctgcgctttttggtgacattgttcctccgagactttgtcagcattatgtattggggacggaaattgtttctgtgatgcatagtgacaaatccactgacttaaatgtggttgggaaatgcctagatgaagtcttagagataaccaacgtatccttggacaagaagcagcttattgttaagatatgtgatattgttgctacacgaggtgctcgacttgctgctgctgcaatactggcaatcctgaagaggttaggcaaagacaagacgaataaaggggagactgtagttgctattgacggttcattatttgcgaaatacaccgagttcaaatcttgcctgcagaagacgcttacagaagaattgctcgatgaagaagtgtcaaagatggtagttcttagacaattcaaagacgcgtctggcattggtgctgctgttgttgctgcatcacattcgattaacacttga

SEQ ID NO: 57 - protein, 490 aa, Beta vulgaris
  BvERDL4;1 (BvIMP; Bv1_015950_zugk.t1)
MSSDSEAGLGGGGGDLRKPFLHTGSWYRMGSRQSSLMGSSQVIRESSISVLACVLIVALGPIQFGFTAGYSSPTQSAITNELGLSVAEYSWFGSLSNVGAMVGAIASGQISEYIGRKGSLMIAAIPNIIGWLAISFAKDSSFLYMGRMLEGFGVGIISYTVPVYISEIAPQNLRGALGSVNQLSVTIGIMLSYMLGLFVPWRILAVLGILPCTILIPGLFFIPESPRWLAKMGMMEEFEVSLQVLRGFDTDISLEVNEIKRSVASSSKRTTIRFAELRQRRYWLPLMIGNGLLILQQLSGINGVLFYSSTIFKEAGVTSSNAATFGLGAVQVIATVVTTWLVDKSGRRLLLIVSSSGMTLSLLVVAMSFFLKEMVSDESTWYSVFSILSVVGVVAMVVTFSLGIGAIPWIIMSEILPINIKGLAGSIATLANWFVAWIVTMTANIMLSWNSGGTFSIYMVVCAFTVAFVVIWVPETKGRTLEEIQWSFRR

SEQ ID NO: 58 - protein, 502 aa, Beta vulgaris
  BvERDL4;2 (BvIMP2; Bv6_128840_qhip.t1)
MSSSDAEDARAELRKPFLHTGSWYRMSTGGGKDPISSGSMMMGSRQSSIFGSIANMRESAISIVFCVFVVALGPIQFGFTCGYSSPTQSDIIKDLDLKVSEFSLFGSLANVGAMVGAIASGQISEYIGRKGSLMIASIPNIIGWLVVSFARDVSFLYMGRLLEGFGVGIISYTVPVYIAEIAPQNMRGMLGSVNQLAVTIGIMIVYLLGIFVEWRALAIIGILPCAALIPGLFFIPESPRWLAKMGMMEECEASLQVLRGFDTDISIEMNEIKKSVGSSSKRTTISISHLKRKRYWFPLMLGIGLLLLQQLCGINGILFYSRTIFEMAGISEGAVATFGLGSIQVVATGVATWLMDRAGRRVLLIVSSVGMTASLLLVSVAFYLETIVPKDSALHSTLGILSVVGLVAMVVSFSLGMGPIPWLIMSEILPASIKGLAGSVATMANFLTSWGVTMTANLLLGWSSGGTFTIYTFFAAFTVIFVAAWLPETKGKTLEEIQAYFR

SEQ ID NO: 59 - protein, 486 aa, Beta vulgaris
  BvC (Bv_009790_mqfe.t1)
MAFGDDEERGEGIIQQDIQQPLIQAKRTTTDGGRNQNQNGENGSRRHPWMVYLSTFVAVCGSYEFGACAGYSSPTQSAITAELGLSTAQYALFGSILTVGAMIGAITSGPIADFIGRKGAMRVYSAFCVGGWLAIYFAKGSLALDIGRLAGGYGMGAFSYVVPVYIAEIAPVHLRGALTTLNQVMICAGVSVAFIIGIVLPWRALALTGLIPCVILLLGLFFIPESPRWLAKKGARKEFEAALQKLRGSDADINHEAAEIQNYIEELEQLPKASMFDLFQTRYLRSVTIAVGLMVFQQFGGINGICFYVSNIFEMAGFSPSVGTVIYALLQVVITTMGATLIDKAGRKPLLLVSAVGLVIGCILTAIAFYFKAHELSEKAAPILAITGILVYISAFSVGMGAVPWVVMSEIFPINVKGVAGSLATLVNWFGAWAISYTFNFLMEWSSSGTFIIYAVINAAAIIFVVMVVPETKGRSLEQIQADINA

SEQ ID NO: 60 - protein, 735 aa, Beta vulgaris
  BvTST2;1 (Bv5_115690_zuju.t1)
MSAAVLVAIAATVGDLLYGWDNATIAGAVLYIKKEFNLESSPTLEGLIVATSIIGATLITTCSGPIADRLGRRPMMIISSVCFFVSALIMLWSPNVYVLLFGRLLDGFGSGLAVTLGPLYISETAPTDIRGSLNTLPQFTGSGGMFLAYCMVFGMSLMETPSWRLMLGILFVPSTVYFLLTVFFLPESPRWLVSKGRMNEAKKVLQWLRGREDVFAEMALLVEGLRVGGDTSIEEYLIEPDAGLAEDQDPMTVKDQVRLYGSEAGCSWVARPVTGQSMLGIASRQGSMQSPSVPLMDPLVTLFGSVHEKLPEQGSMLSVIFPTFGSMFSMGGKEPKNEEWDDENTIGDDDDYGHDDEDYAGDADEDDNLRSSLISRQDTGPDKAMVAPTSGSMFSMKHSSWLQGSEASGIGGGWQLAWKWSEREGLDGTKEGGFKRLYLHQEGDAGSKRGSVISLAGGEVIGDNEYVKAAALVSQPALYSRDFMDRDSIGPAMVHPSEASAKRPSWRDFLEPGVRRALVVGVGLQLLQQFAGINGVLYYTPQILEQAGVGDLLSHMGIGASSALLLISALTTLLMLPAIAVAMRLMDLSGRRTLLLTTIPVLFLSLVVLILANVIKMNTTVYAVVSTVAVVLYFCFFVMGFGPIPNILCAEIFPTKIRGVCIAICALTFWICDIIVTYTLPMMLKAVGLAGLFGFYAVVILIAWIFIFLKVPETKGMPLEVITEFFALGARQASH

SEQ ID NO: 61 - protein, 739 aa, Beta vulgaris
  BvTST2;2 (Bv9_215730_jzcj.t1)
MSGAVLVAIAAAVGNLLQGWDNATIAGAVLYIKKEFNLEGAPTMEGLIVAMSLIGATIITTCSGPVSDRFGRRPMMIISSICFFFSALIMLWSPNVYVLLLGRLLDGFGSGLAVTLVPLYISETAPTDIRGSLNTLPQFTGSGGMFVAYCMVFGMSLMEKPSWRLMLGILVVPSALYFALTVFFLPESPRWLVSKGRMNEAKKVLQRLRGREDVSAEMALLVEGLGVGGDISIEEYLIEPDVGISEEYDPMAAKDQIKLYGSDAGHSWVARPVTGQSMLGLASRQGSIQNPSVPLMDPLVTLFGSVHEKLPEQGSMRSIIFPTFGSMFSMGGKDPRNEEWDEENLHGDDDDYAHNDDDNDDYAEDDDNLHSPLISRQATGTDKAMVAPVSGSMFSMKPSGLIQGTEASGIGGGWQLAWQWSEKEGADGRKEGGFKRLYLHQEGDMVSKRGSVISLPGGDVTGETEYMKAAALVSQPALYSRELMNQHTIGPAMVHPSETAAKGSSWRDLLEPGVRRALIVGVGLQLLQQFSGINGVLYYTPQILEQAGVGDLLSNMGIGASSASLLISALTTLLMLPSIAVAMRLMDISGRRTLLLTTIPVLFLSLVVLILGNIIKMSTTVHAVISTVSVVLYFCFFVMGFGPIPNILCAEIFPTRIRGVCIAICALTFWIGDIIVTDTLPIMLNAVGLAGVFGFYAVVSVIAWIFIFLKVPETKGMPLEVITEFFALGARQPSEDKDN

SEQ ID NO: 62 - protein, 502 aa, Beta vulgaris
  BvVGT1 (Bv3_049950_gzcg.t1)
MASSTTDHQHHVLSSFGKASGEFDLDEVERPLLNGAHPTEDYSLLSCIVPFLFPALGGLLFGYDIGATSSATLSIQSPTLSGTTWYDLSSVEVGLISSGSLYGALIGSVLAFNVADFLGRRKELIAAAIFYLAGALITAIGPNFVIMMIGRFIFGIGIGLAMHAAPMYIAETAPSHIRGRLISLKEFFIVIGMVIGYAIGSFLVNVIAGWRYMYGLSSPLSVIMAIGMWWLPDSPRWLLLCAIQGKGNVPDLRENAISCMCRLRGRAVSDTASQQVDEIMAELSLAGELNNVSTTEMFRGKYLKALVIGCGLVLFQQITGQPSVLYYAASILKSAGFSAASDATRVSILLGFFKLIMTGVAVLVVDKLGRRPLLLGGVSGMVISLLFLGAYYTFLGDAPAIAVVGLLLYVGCYQLSYGPIGWLMISEIFPLRMRGRGISLAVLMNFGANALVTFAFSPLKDLIGAGAVFFMFGGIAVLSLVFIFFIIPETKGLTLEEIEAML

SEQ ID NO: 63 - protein, 502 aa, Beta vulgaris
  BvVGT2 (Bv7_173330_nupg.t1)
MMGNSSIYSLETSLLHHKVNAQKEDYPVDQTTVEEEVFAWSSVILPFLFPALGGLLFGYDIGATSGATISLQSPELSGTTWFNLSAVQQGLVVSGSLYGALFGSIMVFPIADFLGRRRELLIAATLYAIGGLTTAFAPGLEVLLFGRLIYGLGIGWAMHAAPLYIAETCPSQIRGTLISLKELFIVLGILLGFFVGSFEIEAVGGWRYMFGLSVPVAAVMGLGMFSLPPSPRWLLLRAVQGKGSLQEYKEKAVTALSKLRGRPAGDKVSEKQIDDTLVSMKSAYDRESEASFLEVFQGPNLKAFIIGGGLVLFQQITGQPSVLYYAGQILQSAGFSAASDATRVSVLIGLFKFVMTGVAVLKVDDLGRKPLLIGGVSGITVALFLLAAYYKFLGGLPFVAVAALLLYVGSYQISFGPISWLMVSEIFPLRTRGRGISLAVLTNFGSNALVTFAFSPLKELLGADNLFLLFGVIALLSLVFVLTLVPETKGLSLEEIEAKLSE

SEQ ID NO: 64 - protein, 223 aa, Beta vulgaris
  BvSWEET17 (Bv4_075980_knjf.t1)
MDKLSFIIGVIGNIISVLLFLSPLNTFIRIVRKKSTDGFESMPYVCTLLSTCLWTYYGIIRPGALLVATVNGFGALVELVYVALFITFAPPTMKAKTAKLAAILDVGFLGAVILISNLMLEGETRINMIGTIGAGLNIIMYGSPLVALKTVIKTRSVEYMPFLLSLFSFLNGGIWTVYAALVKDFFLLVPNAIGFILGTIQLVVYVCYMNPSKEQQYNEPLIY

SEQ ID NO: 65 - protein, 325 aa, Beta vulgaris
  BvFrcK1 (Bv3_066020_xjni.t1)
MKHGESLVVCFGEMLIDFVPTVAGVSLAEAPAFAKAAGGAPANVAVGISRLGGSSAFVGKVGKDEFGFMLADILKQNKVDNSGMRFDPGARTALAFVTLRADGEREFLFFRNPSADMLLHESELDKDLLEKAQVFHYGSISLIEEPCRSAHLAALTIVKKAGGFLSYDPNLRKQLWPSEEAARDGIMSIWDQADMIKVSEDEITFLTGGDDPYDDNVVMKKLFHPNLKLLIVTEGSEGCRYYTKTFKGRVSGVKVKPVDTTGAGDAFVGGILSNLASDLNILKDEKRLREALHFANACGAVTVTKRGAIPGLPTRDEVLEILQQA

SEQ ID NO: 66 - protein, 331 aa, Beta vulgaris
  BvFrcK2 (Bv3_057460_dyyp.t1)
MAELNNGGHSKGLVVSFGEMLIDFVPTSSGVSLAEAPGFLKAPGGAPANVAIAVSRLGGNAAFVGKLGDDEFGHMLAGILKKNGVSADGLSFDKGARTALAFVTLKSDGEREFMFYRNPSADMLLTPDELNLDLIRSAKVFHYGSISLIVEPCRSAHLKAMEEAKKAGALLSYDPNLRLPLWPSAEEAREQIMSIWDKAEVIKVSDNELEFLTGNSTIDDATAMSLWHPNLKLLLVTLGDQGCRYYTKNFKGSLDGFKVNAVDTTGAGDSFVGALLNKIVDDHSIIEDESRLKEVLKFANACGAITTTKKGAIPALPTVADALELIKKNAS

SEQ ID NO: 67 - protein, 313 aa, Beta vulgaris
  BvFrcK3 (Bv2_027840_oqrd.t1)
MLIDFVPTTNGVSLAEAPAFKKAAGGAPANVAVGIARLGGKSAFIGKVGEDEFGYMLANILKENNVNNEGMRFDPGARTALAFVTLRRDGEREFMFYRNPSADMLLQESELDFELIRKAKIFHYGSISLITEPCKSAHIAAAKAAKDAGVLLSYDPNLRLPLWPSAESARDGILSIWDTADIIKISEEEISFLTQGEDPYDDNVVRKLYHPNLKLLLVTEGADGCRYYTKDYSGKVGGLKVDAVDTTGAGDAFVAGLLSQLAADSNLIQVEDRLRDALQFANACGALTVTERGAIPAMPTREAVLNVMLKSVA

SEQ ID NO: 68 - protein, 311 aa, Beta vulgaris
  BvFrcK4 (Bv7_178860_gedd.t1)
MLIDFVPDEAGVSLAESRGFVKAPGGAPANVACAITKLGGTSAFIGKVGDDEFGKMLVDIIKKNGVNTEGVCFDKEARTALAFVTLKKNGEREFMFYRNPSADMLLQTSELNLDLIKQAKVFHYGSISLITEPCRSAHIAAMKAAKEAGVTLSYDPNVRLPLWSSPEAAREGIKSIWNQADIIKVSDDEVEFLTQGDATKEEVIKTLWFDGLKLLLVTDGEKGCRYFTKDFKGSVKGFSVKAIDTTGAGDAFVGSFLYSLAKDPSILQDENKLKEALTLSNACGAICTTQKGAIPALPSLSQAQDLVKQGN

SEQ ID NO: 69 - protein, 481 aa, Beta vulgaris
  BvFrcK5 (Bv8_182100_hsoh.t1)
MAIHLLSPIPSSFSLSYKPSSLFPPIFSKISTSSKIKATTLNNPQNDIQEPSKRRGRPKGSKKSTTLSPQKTAKISDGSSQNTQSTNGSTLNLDELNNFDDGMDFPYLEPPLICCFGAVQKEFLPTVRVSEQQMHPDIYSGWKMMQWNPPEFGRAPGGPASNVAIAHVRLGGRAAFMGKVGDDDFGEDLVYMMNKEKVQTRSVKFDSNVKTGCTFMKIKFSDNGKIKMELVKEAAEDSLVATELDLAVLKEARIFHFNSEVLTSPCMHLSLFKAIKISKFFGGLVFFDPNLPLPLWKSRDETREVIKEAWEEANIIEVSRQELEFLLDEDHYEKRRNYRPQYYAEDYEQSKNRRDYYHYTREEITPLWHDGLKFLFVTDGTFRIHYYTPSFDGVVVGTEDVLITPFTCDRTGSGDAIVAGIMRKLTSHPEMYEDQDVLERQLRFAIAAGIISQWTIGAVRGFPTESATQNLKEQVYVPSMW

SEQ ID NO: 70 - protein, 550 aa, Beta vulgaris
  BvFrcK6 (Bv6_136290_jzyk.t1)
MLVADNRLRNRWVLSATSKKAIVASIPEEEASTESKGTKKARSRQANARGRKKATTELLDHDFNLLASSSISEQEFSDLEASISDSEKPKRRTRKKVVSPTSTSGMEEVKTNKKSRGRKSKEEISKVEDQTSEMEVNDLEEVVYRTSQDNDDSDIDLQLGKSDGDDISFSYGWPPLVCCFGAAQHAFVPSGRPANRLIDYEIHDSLKDALWEPEKFVRAPGGSAGGVAIALASLGGRVAFMGKLGNDDYGQTMLYYLNVKNVQTRSVCVDDKRPTAVSQMKIAKRGALRTTTVKPCAEDSLSISDINIDVLKEAKMFYLNTSSLLDASMRRATLRALKISKKLGGVIFYDLNLPLSLWQSDEETKSFIEQVWSLADVIEVTKQELEFICGIKPLEEFDTKNNKRSKFEHYEPDIIAPLWHENLKVLFVTNGTSKIHYYTKEHNGAVLGVEDAPMSPFTQDMSASGDGIVAALMRMLTVQPHLITDKEYLERAVKYAINCGVIDQWIVTRQNGFPAKEGLEEEDEDEGIPDLNGIRSITERQFRTVMPVSS

SEQ ID NO: 71 - protein, 498 aa, Beta vulgaris
  BvHxK1 (Bv8_197580_aaut.t1)
MRKAAVGATVICAAAVCAAAAVVVRQRMKSSSKWARAMAILKELDEKCETPLGKLRQVADAMTVEMHAGLASEGGSKLKMLISYVDNLPTGDEHGLFYALDLGGTNFRVLRVKLGGKEKGVVQQEFDEVSIPPELMVGTSEELFDYIAAALAKFVATEGEGLHPEPNRQRELGFTFSFPVKQTSIASGTLIRWTKGFSIEDTVGEDVVAELTKAMKRKGVDMRVTALVNDTVGTLAGGRYTKGNVIAAVILGTGTNAAYVERASAIPKWHGPLPRSGEMVINMEWGNFRSSHLPLTEYDIALDEESLNPGEQIYEKMISGMYLGEIVRRVLCKMAEEASFFGDTVPPKLKTPFILRTPDMSAMHHDTSPDLKVVASKLKDVLGIPNTSLKVRKVIVDICDIIASRGACLSAAGILGIIKKLGKDALKQGENQKSVIALDGGLFEHYAKFRECMEDSLKELLGDEIADTIVVEHSNDGSGIGAALLAASHSQYLEEEES

SEQ ID NO: 72 - protein, 513 aa, Beta vulgaris
  BvHxK2 (Bv9_224680_aote.t1)
MGKVVIVATVLGAAVVCAVGGLIVSRRMKNGANWRRTMEILRDFEEKCGTPIEKLKQVADAMVMEMHAGLASDDGSSIKMLISYVDNLPTGDEDGLFYALDLGGTNFRVLRVQLGGKDGGIKHQEFAEVPIPVELMIGTSDDLFGYIASEVAKFIAQEGPEFQLPSGRERELGFTFSFPVMQTSIDSGTLITWAKGFSIDDTVGKDVVEELAKALKKQGVDMHVTALVNDTVGTLAGGQFSNKDVIAAVILGTGTNAAYVERAEAIPKWRGPLPKSGEMVINMEWGNFQTSNLPLTEYDYALDYHSPNSGEQIYEKMISGMYLGEIVRRVLCRMAEEASFFGDTIPPKLHIPFILRTPDMSAMHHDSSPDLEIVGSTMKDILEIPMLSLKKRKVIYDLCKIVATRGARLAAAGISGILKIVGRDTLSSNDEKRKSVIAMDGGLYEHYEEFRKCLEHTLKELLGDKVWERISIEHANDGSGIGAALLAASHSRYLEDNETQEDIVVVPAMLSDD

SEQ ID NO: 73 - protein, 509 aa, Beta vulgaris
  BvHxK3 (Bv4_073320_tcog.t1)
MGKVGFGLAVSIAVVTSAVAAAVVVKRVKSRRKWQRVVGVLKELEECCGTHVSRLKQVVDAMAVEMHAGLASEGGSKLKMLLTFVDKLPNGSEKGIYYALDLGGTNFRVLRVQLGGRRSGIVRHDVERKPIPEHLMTSTSEDLFDFIATSLKDFYGQENDKSSDLSPVSRRKLGFTFSFPVKQISVSSGILMKWTKGFSIRDMVGSDVSECLHQAMSRQGLDMHIAALVNDSVGTLALGHYNDEDTVAAVIIGTGTNACYFERADAIIKSQGLPTSSGGMVVNMEWGNFWSSHLPRTSYDIELDAESPNPNDQGFEKMISGMYLGEIVRRVILRMSKESDVFGPISSSLCEAFILRTPLMSTMHEDDSPDLEEVARILEEVLGICDVPLKVRKLVVNVCDVVTRRAARLAAAGIVGILKKIGRDGSGGVASSRAKGSSSSNRLKRTVVAVEGGLYSNYRMFREYLNDAVAEILGEEIAPFVILKVTEDGSGIGAALLAAAYSSPETVDT

SEQ ID NO: 74 - protein, 496 aa, Beta vulgaris
  BvHxK4 (Bv5_124820_xpum.t1)
MSIPAASTAVGSLCLPRSRIRSSALQPMMAVRSGTVSSVTQILTKLQKECATPLPVLRHVADSMGNDMRAGLAVDGASDLKMILSYVDTLPTGNEKGLFYALDLGGTNFRVLRVQLGGIDQRVIATEAQQVSIPQDLMFGTSEELFDFIASGLAKFAEKESGEFQLLQGRKRELGFTFSFPVKQTSISSGILIKWTKGFAVSGTSGKDVVACLNEAMQRQGLQMQVSALVNDAVGTLAGAKYWDNDVMVAVILGTGTNACYVERIDAIPKMPGQKSQSGTTIINTEWGAFSTGLPLTEFDREMDAESINPGEQIFEKTISGMYLGEIVRRVLLKMDEAGSLFGSSMPDKLQTPFSLRTPHICAIQQDTSNNLDEIGSILFNEAGVEAKTEARQIVLEVCDTIAKRGGRLAGAGIVGILHKMEDDMKGLIFGKRTVVAMDGGLYENYPQYRNYLQDAVTELLGPALSENIVIEHSKDGSGIGAALLAAANSKYKHHI

SEQ ID NO: 75 - protein, 466 aa, Beta vulgaris
  BvHxK5 (Bv9_224670_aurc.t1)
MGDIVNVNVGENLMEMVKKIEEEFWVPAELLKQLADDMELMMRKGLEDEHSSSIKMLVSYVDSLPSGDEEGCFYALDLGGTNLRVMQVKLQGNRTIDLKAESYMVPPKMKVGTLHELFDYIAERVSHVFETEENHDFEDVPGKRRELGFTFSFPVHQTRINSGTLLNWTKDYNAQDAIGKDMVEELTKALEKRAIDVNVTALLNDTVGTLAGGRFYDNNVVAAVILGTGMNAAYVEQSENIVKPYGIPPKSGQMVINTEWGNFNSSLLPLTDYDRALDNDTPNRHKQILEKMLSGRYLGEIVRRILQRLAEDAALFGDIVPPRLCQHYVLGTEIVSVMHSDKSTDLNVVGKCLDEVLEITNVSLDKKQLIVKICDIVATRGARLAAAAILAILKRLGKDKTNKGETVVAIDGSLFAKYTEFKSCLQKTLTEELLDEEVSKMVVLRQFKDASGIGAAVVAASHSINT

SEQ ID NO: 76 - DNA, 8183 bp, Beta vulgaris
  BvERDL4 ;2 (BvIMP2; Bv6_128840_qhip.t1)
  promoter 1..1500: /function="promoter"
  5'UTR 1501..1760: /function="5'UTR"
  misc_feature join(1761..2000,2106..2168,2372..2461,2677..2736,2828..2893,2967..3032,3138..3213,4712..4776,4864..4956,5048..5128,5224..5308,5725..5771,5863..5925,6011..6070,6589..6654,6773..6832,6982..7096,7298..7410): /gene="CDS regions"
  3'UTR 7411..7683: /note="3'UTR"
ctggcccactttcaaaaatactgccaaaagccagccacatggcaaagtgtaggatgctcatcctacacatcggtgtaggatctaatttgcgcaacatgggacccacaaaacaaaacattaaactccacgtgagctatgcaattggatatttaaaattttctcatttgttcaaccaaccatatggtgacacatggcacaaactaatacaattacaaaagttttctatacttcttgtaaccgtttaatgatctttttcttaaaatttttttaaaaagatggtaataatttattttctaacaactttaatttttctttgtttatagaataatgaacctaatattggatataaatcataaacaatctttttttttttcatatggagcaccatcaacgtcccttgtatgagcatattgcgatattgtattttaatttaaatattagcttttcatgttgtatattaattttcatttcatttctttttaatcaaactatatattaccattcaaaataatattttttaaatatataaaaaattaaattctacatacataaatatgaaaaacatataattttttgtaataatatttaatatatgtgaataatttcattcatataactttgatcataatataaaacgagtttcacttattgacatggaaagcaccaaatagtatgtaaaaagttgaatgcatacctccataaaaagtttcattattgtcggtgcttatggacataattcttaaaaattaaaatagcttacaagcagagaatagatgatagagtggagagtagggatgaaaatggatcaggttcggggtgggtggagcttcacccgtatccaccactcgcatccatccgcaccacccacatccatccatcacccgcataagccattatccacatccatccatccgtcatccatcgggcgaacgtgagttgggtggttaacgagtgatgatatatatataacaatttttacaaaaaattatgccataagatacatactattttttttttagttgcaacgattagacattttatactcacactttatgtctaatagttgcaactaaaaaaacagaggtactatttattaaaattttcaaccaaattatgtgaaattgataatatgaatgatatgagtgggtgttaatcgtgcaatgggttgagtgacagatgaaaagaaagagtacccgcatcattatccgtttcatctactacctgcttttcatacgtttatttcaggttttcacctgcttaataaaagcgagttaagcggatgattttgcatccctggtggagtggtcattgcctcataggagaacctaactagtattataatttgtacatgaagggaaaagaaaaaatcagtcacatgtgacatcaacctcatttatgaaaacttccaagaaaggatatttgttatccttcttgacctcctctctctcctctgtaaatcaaaattatataaacaaacacaacaagtaagactcaatacagggtggatcagccaaattagaaaaaccaacattaagaaaagatcaccatcatcatcatcaaatatcatcaaacaaacaggacccccattttgtcgtaagactcttcatactcacaataaaataaacaaacacaacaaacattggcgccaaacagctaattccaccatcaaataacaaagagatctaccctcatttttttctctctctctgatttactactcaattttgtttcaacaaaacccccaaaaaaaaagtgaaaaaatgagtagcagtgatgcggaggatgcgagggcggagctccgaaaaccgtttcttcatacgggtagttggtatcggatgagtacgggtggtggaaaagatccgattagtagtggtagtatgatgatgggttcaagacaatctagtattttcgggtctattgctaatatgcgtgaatccgccatttccattgttttctgtgtttttgttgttgctttgggtcccatccaatttggtttcaccgtatgttttttttttcttttttcttttttcttttttctatctcctttttcttactttatttttatttaaagtttgatttttttttatggtttatgtttttggcagtgtgggtattcatccccaactcaatccgacatcattaaggatcttgaccttaaagtttccgaggtttgaatgttttacatttgaatttcatcaagatcgcctatgattgtgtttaatttcaaactttgttatgtagtgtatatgttaattgtataaaaaccccattatatgataatttgttggtgtaagaaaaatgttgcctttagttgtatgattgatttttgaagtgattgatgaagtgatgatgatgttaatggaattgacagttctcattgtttggatcattggctaatgtgggagcaatggtgggggcaattgcgagtggacagatttctgaatacattggaagaaaaggggtatgagattttactccctttctataagtagtggatgatatagtgttttttactgtatgcctgtatggtttctaatcattggatttgtgtcgtagtcaccggttactaatgtctcgaaaagggtcctatggataagaataaggttcaattcatgtttatgtagggtgttatttcatgatttctaaaagtatgggtgtgtatgcttttaattgcagtcattaatgatcgcctcaatccctaacattataggatggcttgtcgtttcatttgcgagggtaagtgaatgagtattgttctatttgtgtatcttcctagttgcttataagcttattcgatttctgcttcttactgctgctgtttttgtaggatgtctcgtttctttacatgggacgcctgctggaaggttttggtgttggcattatttcctacacggtaagagttgttgaatttgacttctttttgttatgtttgagcagattttttttatagttttcagtgtaattaggtgcctgtttatatagccgaaatagcacctcaaaacatgaggggaatgcttggatcagtgaaccaggtgattttctggttttactttagttgatcatatttctctatatgataactcctctgtcttcaatgcttaatgtctgaagactgactagtggaatttctttttcagcttgctgttaccattggcataatgatcgtttacctgttgggaatttttgttgagtggagagcacttgcaatcattggtatgcaattattatatgtattttttgttaattactccaaatgattgaagcagcataatgtttacataactggaatagatataaacatttaaggctaatactgaggtaaagctgcagacggtcagtactgagaacatcccggtagagtaagtcttctatatagagttgtagcttgtgtgtttagcttgatggagcctgtaagagaatctatgttggcctgctgtatcttagaagcataggactcgaataatcttggatctggaaaggtattcggtcttggcattttctaatcgcataaagagcttagttttgcgggtgggacaatagaacctgcgtgaagtctttctgatgaacttttacctgctgcagagtgtagtaggctagtagctagaaaaggctaattaaatgctaatactgttctccatcggatggagaggaggattttttgtggagcccgcgccaagtagattaactaaaatgccacctctccacatttgtagtggacagttctccaaataatcgtactcagctagctttggcatagagtgtggaggtaacttctataatgcaagtccttcagatcaatgatgctatagcctacaagggatatatagtgggaggaggataaatcccatatcagatgaaaacttgtattttggcaatagtcacttcagtatagcaacgggctgtgttttccgcagtgaacaggggaccgacataagtgagtttttatccatcaaagcctcagaagtcagagctgatccaaatgtatttctgatcgattggcaacttcaaaacacaggatattactacaatatccttgccttattctctgcaactattctcatccattgttcacatgtttaactattcttgattcatgagataacacgggatctcagtctcacagaccaggtcttaggttctgtttggtttgacggggaacacaatagcaaataagttgttctttgttttgttctttgcaagaatagttagacaaaatggaaaagtgaaaaggagggagaagatggatgagagaagaggaagaagctaagtaatagggaggacaacatggtatttcttctttcataaagagaaacgtgcattccttccttcagaagggaaatgtttttcacctttagaaaaactatttctacccatggaaaaactactttccacacttacaaaccaaacaaaggaaaatagggaaactgtctttcctgaaaatgttttccatccaactaaacactcgttggaggagaaacatcaggtctggacaagcctatctccgtcttgatggaggacttgtttgtgtgataaaaaattgaccattgttctgatgtaaactcactatgaccctgtactgaatggtatatgtaagtcttgcatcttatttatgtaggaagctttttcccatgcagatatacatcattttccctttgaaggacacaaccgaatgaactctctagattctgaaatttcttctcatgctttgcaggaatcctaccttgcgctgcgttgatacctggattgtttttcataccagaatctcctcgctggctggtcaaaacctgttaacatgcatgtttattaagcctttctttattatgatatatcatattctgacttttctttccttgcctttctcaggcaaaaatggggatgatggaagaatgtgaagcgtctttgcaagttctgagaggattcgatacagatatctcgattgaaatgaatgaaatcaaagtattcagttgagctttttcatagttgataaacaatatatatttatcttgttttgctgttgcgagtccttaactaaattgatgcactgcagaaatctgtgggatcatccagcaaaagaacaacaattagcatttcacatctcaagagaaaaagatattggttcccattgatggtacaacggtttgtttgggactatgattttgtgtttccattatcaaccttcaaaacattttatttctcgtctaatgctcaattgacatgttgcagttaggaatcggattacttttgcttcagcagctctgtggtattaatggaatattgttctactcccgcaccatatttgaaatggcaggttagaatcatctagtaactgaatctggacttcaagggtgaattcctgtcaattttctaagcaaaagatacacaacacgttttctttccaaaagatttggaaattaactagccacaaatggcacaagcccctaagatagggaaagataaggacaccccgacccgaaagaaacctcatttgttaagaaggtaggtgataaattacccatgaaggaaatcaccacaataccccagcttgggatgacaagattcgaactcccaacttcatgatttggaggtgcaagttatcgatattaggcctagctgaattgaatctctgaaaaaaattcaaaagttaaagcaaatatgtccttaaagttgtgatctttgcttcaatttattagtatgaacatctttaatttaccacaaactggacaggaatatctgagggtgctgtcgccacatttggtcttggaagcattcaggtgactaaatctaatctaagttcctttttcttattttttttttgtgattagtagtaaaatcaacccttcatctttctggcaaactaaacaggtggttgctactggagttgccacttggctgatggacagggctggccgaagggttcttcttatagtatgttctgaaatataactttcatctggtgttgtggtactattcatggatggaattagagtaaacgagttttgaatctttacaggtatcctctgttggaatgactgctagcctcctcctagtttcagtcgcattttatctggaggtcggtatcattttcttcattttgcatatgcaatacatccagcaaagttaggtgctatactgctatatatcatgtttacacttactagcattaatgagccaaattcaaatctgtgggaagtggtaaacttgcaaagtctgggatcacaactcgtttctatcttgtgtcccacctcatatttcattggacatatcaccagcgtacaagcaataatctagtgttatcgccttcttagtagatgcagatgatatgggataataagataaggcgttacatgatgtgtcacaatgggatagagtaactaaactagaagaataaaggacccttcttccagggttactatttactgctagcctgctagcctgctattgacaccatcattgtgcatgatttcctcttctaatatagaattcggttgcaaggcagaagagaccgtatatgttgatgtagtggatgactataagttcctaaaattttgcttgctattttatgcctcctgctgtctacattgttgacagaccatcgtaccaaaagactcggcattgcacagcacgttgggcattctctctgtcgtaggcctcgtggtattgcttctaactctaatttcatcaccactcagaggggatcaaaaaattaaaagaacaaagaaaaatgaaattatattaagcagatttaagacttggcttcttctatctgtggcaggcaatggtggtttccttttctttgggaatgggacccattccttggcttataatgtctgaggtatgctaattcatctatatgtctaaaccatgttatatggaatctaattttgcatgaccttgggctgctcactttcgaagctatagcaagtatattatatcatgcattttgcaattaaccacttgctccttttatttccgtttaaccagatacttccagctagtataaaaggccttgctggcagtgtagcaacaatggcgaactttctaacttcctggggtgtcactatgactgcaaacttgctgctcggctggagtagcggaggtgaatctttttatggcttcttctctttaccttatttttacttggcaaaactgataattactgctttccaaggaaaaaaatgattattgctgaaactgttttattagtattagattagttcttccctattgtatttgaaagcatcttgtgtttatagcattataatctcctgattaattctgaatctccaatcctttgcaggaacctttacaatttacacattttttgctgcttttactgtgatatttgtggctgcatggcttccggagacaaaaggaaagacgctcgaggagattcaagcatacttcagataaatgcacaagtttgtggttatccctacttggcatttcatgagcattttatgcagcatacacagaagactggaaggttagaagattacatttgttttcataagtatacagaaaagctactgcttttaagaaagctgattcttgtatttgggacaacaatgctactctttcttttcatatcatttgattcatctcgcgactgttgtacaaacaatacgctttatacgcgttcatatgtattattcagattctgaaaaagaaaaatgcaaatatggaattccattcttcgtaatctaattcgcacagttatttccacaaatttagacggggaagcattgtagtccctttgtctagaactaatagtcaggttgacagtgtacgttgttcgaactggtgctgtaacgagttaacgactaactctggagtctgaacagaggcactgaatcggcttacttgtgatcagctccatcagcataaacagaagctaagaagcgcttgagacatctattgtacacacacggtctctcgaggtgaaccagatggcctgccttctttataccttcatatgtcgctttttccccgagttttctgcaaatgtcatcagggaagttggagcataagtttaagaacagaattctttgctaacactgattatcaacattatactccatccacttctttgtatcttttttaagtgaccaaggttttcaaaaactctgctttgactagtgatatcttatacaatatgtttgagccactttgaggttccctatgaa

SEQ ID NO: 77 - protein, 487 aa, Brassica rapa
  >BrA - Brassica rapa
MSFREETEEGRNDLRRPFLHTGSWYRMGSRQSSMLESSQVIRDSSISVLACVLIVALGPIQFGFTCGYSSPTQADITRDLGLTVSEYSVFGSLSNVGAMVGAIASGQIAEYIGRKGSLMIAAIPNIIGWLSISFAKDTSFLYMGRLLEGFGVGIISYTVPVYIAEIAPQNMRGALGSVNQLSVTIGIMLAYLLGLFVPWRILAVLGVLPCTLLIPGLFFIPESPRWLAKMGLTDDFETSLQVLRGFDTDITIEVNEIKRSVASSTKRSAIRFVDLKRRRYYFPLMVGIGLLVLQQLGGINGVLFYSSTIFESAGVSSSNVATFGVGAVQVVATAVATWLVDKSGRRLLLMISSIGMTISLVIVAAAFYLKEFVSPDSDMYNILSMVSVVGVVTMVITCSLGMGPIPWLIMSEILPVNIKGLAGSIATLANWFVSWLVTMTANMLLAWSSGGTFTLYALVCGFTVAFVSLWVPETKGKTLEEIQALFR

SEQ ID NO: 78 - protein, 487 aa, Brassica rapa
  >BrB - Brassica rapa
MSNRDDTEEGRSDLRRPFLHTGSWYRMGSRQSSMLESSLAIRDNSISVLACVLIVALGPIQFGFTCGYSSPTQAAITKDLGLTVSEYSVFGSLSNVGAMVGAIASGQIAEYMGRKGSLMIAAIPNIMGWLSIAFAKDTSFLYMGRLLEGFGVGIISYTVPVYIAEIAPQNMRGALGSVNQLSVTVGIMLAYLLGLFVPWRILAVLGVLPCTLLIPGLFFIPESPRWLAKMGLTDDFETSLQVLRGFDTDITIEVNEIKRSVASSGKRSAIRFVDLKRRRYYFPLMVGIGLLVLQQLGGINGVLFYSSTIFASAGVSSSNVATFGVGAVQVLATAVATWLVDKSGRRLLLMISSIGMTISLVIVAVAFYLKEFVSPDSNMYNILSMVSVVGVVAMVIACSLGMGPIPWLIMSEILPVNIKGLAGSIATLANWFVSWLVTMTANMLLAWSSGGTFTLYALVCGFTVAFVSLWVPETKGKTLEEIQALFR

SEQ ID NO: 79 - protein, 488 aa, Brassica rapa
  >BrC - Brassica rapa
MSFRDETEDARNDLRRPFIHTGSWYRMGSRQSSMMGSSQIIKDNSISVLACVLIVALGPIQFGFTCGYSSPTQAEITKDLGLTVSEYSVFGSLSNVGAMVGAIASGQIAEYIGRKGSLMIAAIPNIIGWLCISFAKDTSFLYMGRLLEGFGVGIISYTVPVYIAEIAPQNMRGGLGSVNQLSVTIGIMLAYLLGLFVPWRILAVLGTLPCIVLIPGLFFIPESPRWLAKMGMTDDFETSLQVLRGFETDITVEVNEIKRSVASSTKRSSTVRFVDLKRRRYYFPLMVGIGLLVLQQLGGINGVLFYSSTIFESAGVTSSNAATFGVGAIQVVATAISTWLVDKAGRRLLLTISSVGMTISLVIVAAAFYLKGFVSPDSDMYSMLSILSVVGVVAMVVSFSLGMGPIPWLIMSEILPVNIKGLAGSIATLANWFFSWLITMTANLLLAWSSGATFTIYGVVCAFTVVFVTLWVPETKGKTLEELQALFR

SEQ ID NO: 80 - protein, 488 aa, Brassica rapa
  >BrD - Brassica rapa
MSSRDETEEARNELRRPFMHTGSWYRMGSRQSSMMGSSQVIKDNSISVLACVLIIALGPIQFGFTCGYSSPTQAAIIKDLGLTVSEYSVFGSLSNVGAMVGAIASGQIAEYIGRKGSLMIAAIPNIIGWLCISFAEDTSFLYMGRLLEGFGVGIISYTVPVYIAEISPQNMRGGLGSVNQLSVTIGIMLAYLLGLFVPWRILAVLGTLPCIVLIPGLFFIPESPRWLAKMGMTDDFETSLQVLRGFETDITVEVNEIKRSVGTSTKRSSTVRFVDLKRRRYYFPLMVGIGLLVLQQLGGINGVLFYSSTIFESAGVTSSNAATFGVGAIQVVATAISTWLVDKAGRRLLLTISSVGMTISLVIVAAAFYLKEFVSHDSDMYSMLSILSVVGVVAMVVSFSLGMGPIPWLIMSEILPVNIKGLAGSIATLANWFISWLITMTANLLLAWSSGGTFTLYGLVCAFTVVFVTLWVPETKGKTLEELQALFR

SEQ ID NO: 81 - protein, 486 aa, Brassica rapa
  >BrE - Brassica rapa
MSDTEEARNNDLRRPFIHTGSWYRMGSRQSSMMGSSQVIRDSSISVLACVLIVALGPIQFGFTCGYSSPTQAAITKDLGLTVSEYSVFGSLSNVGAMVGAIASGQIAEYIGRKGSLMFAAIPNIIGWLCISFAKDTSFLYMGRLLEGFGVGIISYTVPVYIAEIAPQNMRGGLGSVNQLSVTIGIMLAYLLGLFVPWRILAVLGTLPCIVLIPGLFFIPESPRWLAKMGMTDDFETSLQVLRGFETDITVEVNEIKRSVASSTKRSSTVRFVDLKRRRYYFPLMVGIGLLVLQQLGGINGVLFYSSTIFESAGVTSSNAATFGVGAIQVVATAISTWLVDKAGRRLLLTISSVGMTISLVIVAAAFYLKGFVSHDSDMYSMLSILSVVGVVAMVVSFSLGMGPIPWLIMSEILPVNIKGLAGSIATLANWFFSWLITMTANLLLAWSSGGTFTLYAVVCAFTVVFVTLWVPETKGKTLEELQALFR

SEQ ID NO: 82 - protein, 468 aa, Brassica rapa
  >BrF - Brassica rapa
MKMSNASDGNREVREPLVDKDMAESKPEQPWMVYLSTFVAVCGSFAFGSCAGYSSPAQAAIRNDLSLTIAEFSLFGSLLTFGAMIGAITSGPIADLIGRKGAMRVSSAFCVVGWLAIFFAKGVVALDLGRLATGYGMGAFSYVVPIFIAEIAPKTFRGALTTLNQILICTGVSVSFIIGTMVTWRVLALIGLIPCAVSILGLFCIPESPRWLAKMGRDTEFEAALRKLRGKKANISEEAAEIQDYIETLERLPKAKALDLFQRRYIRSVFIAFGLMVFQQFGGINGICFYTSSIFEQAGFPPRLGMIIYAVLQVVITALNAPIVDKAGRKPLLLVSATGLVIGCLITAVSFYLKAHDMAHKAVPVLAVVGIMVYIASFSAGMGAMPWVVMSEIFPINIKGVAGGMATLVNWFGAWAVSYTFNFLMSWSSYGTFIIYAVINALAIFFVIAVVPETKGKTLEQIQAVVNP

SEQ ID NO: 83 - protein, 487 aa, Brassica napus
  >BnA - Brassica napus
MSFREETEEGRNDLRRPFLHTGSWYRMGSRQSSMLESSQVIRDSSISVLACVLIVALGPIQFGFTCGYSSPTQAAITRDLGLTVSEYSVFGSLSNVGAMVGAIASGQIAEYIGRKGSLMIAAIPNIIGWLSISFAKDTSFLYMGRLLEGFGVGIISYTVPVYIAEIAPQNMRGALGSVNQLSVTIGIMLAYLLGLFVPWRILAVLGVLPCTLLIPGLFFIPESPRWLAKMGLTDDFETSLQVLRGFDTDITIEVNEIKRSVASSTKRSAIRFVDLKRRRYYFPLMVGIGLLVLQQLGGINGVLFYSSTIFESAGVSSSNVATFGVGAVQVVATAVATWLVDKSGRRLLLMISSIGMTISLVIVAAAFYLKEFVSPDSDMYNILSMVSVVGVVTMVIACSLGMGPIPWLIMSEILPVNIKGLAGSIATLANWFVSWLVTMTANVLLAWSSGGTFTLYALVCGFTVAFVSLWVPETKGKTLEEIQALFR

SEQ ID NO: 84 - protein, 487 aa, Brassica napus; identical to SEQ ID NO: 77
  >BnB - Brassica napus

SEQ ID NO: 85 - protein, 487 aa, Brassica napus
  >BnC - Brassica napus
MSNRDDTEEGRSDLRRPFLHTGSWYRMGSRQSSMLESSLVIRDSSISVLACVLIVALGPIQFGFTCGYSSPTQAAITKDLGLTVSEYSVFGSLSNVGAMVGAIASGQIAEYMGRKGSLMIAAIPNIMGWLSISFAKDTSFLYMGRLLEGFGVGIISYTVPVYIAEIAPQNMRGALGSVNQLSVTVGIMLAYLLGLFVPWRILAVLGVLPCTLLIPGLFFIPESPRWLAKMGLTDDFETSLQVLRGFDTDITIEVNEIKRSVASSGKRSAIRFVDLKRRRYYFPLMVGIGLLVLQQLGGINGVLFYSSTIFASAGVSSSNVATFGVGAVQVMATAVATWLVDKSGRRLLLMISSIGMTISLVIVAVAFYLKEFVSPDSNMYNILSMVSVVGVVAMVIACSLGMGPIPWLIMSEILPVNIKGLAGSIATLANWFVSWLVTMTANMLLAWSSGGTFTLYALVCGFTVAFVSLWVPETKGKTLEEIQALFR

SEQ ID NO: 86 - protein, 487 aa, Brassica napus
  >BnD - Brassica napus
MSNRDDTEEGRSDLRRPFLHTGSWYRMGSRQSSMLESSLAIRDSSISVLACVLIVALGPIQFGFTCGYSSPTQAAITKDLGLTVSEYSVFGSLSNVGAMVGAIASGQIAEYMGRKGSLMIAAIPNIMGWLSIAFAKDTSFLYMGRLLEGFGVGIISYTVPVYIAEIAPQNMRGALGSVNQLSVTVGIMLAYLLGLFVPWRILAVLGVLPCTLLIPGLFFIPESPRWLAKMGLTDDFETSLQVLRGFDTDISIEVNEIKRSVASSGKRSAIRFVDLKRRRYYFPLMVGIGLLVLQQLGGINGVLFYSSTIFASAGVSSSNVATFGVGAVQVLATAVATWLVDKSGRRLLLMISSIGMTISLVIVAVAFYLKEFVSPDSNMYNILSMVSVVGVVAMVIACSLGMGPIPWLIMSEILPVNIKGLAGSIATLANWFVSWLVTMTANMLLAWSSGGTFTLYALVCGFTVAFVCLWVPETKGKTLEEIQALFR

SEQ ID NO: 87 - protein, 488 aa, Brassica napus
  >BnE - Brassica napus
MSSRDETEEARNELRRPFMHTGSWYRMGSRQSSMMGSSQVIKDSSISVLACVLIIALGPIQFGFTCGYSSPTQAAIIKDLGLTVSEYSVFGSLSNVGAMVGAIASGQIAEYIGRKGSLMIAAIPNIIGWLCISFAEDTSFLYMGRLLEGFGVGIISYTVPVYIAEIAPQNMRGGLGSVNQLSVTIGIMLAYLLGLFVPWRILAVLGTLPCIVLIPGLFFIPESPRWLAKMGMTDDFETSLQVLRGFETDITVEVNEIKRSVGTSTKRSSTVRFVDLKRRRYYFPLMVGIGLLVLQQLGGINGVLFYSSTIFESAGVTSSNAATFGVGAIQVVATAISTWLVDKAGRRLLLTISSVGMTISLVIVAAAFYLKEFVSHDSDMYSMLSILSVVGVVAMVVSFSLGMGPIPWLIMSEILPVNIKGLAGSIATLANWFISWLITMTANLLLAWSSGGTFTLYGLVCAFTVVFVTLWVPETKGKTLEELQALFR

SEQ ID NO: 88 - protein, 488 aa, Brassica napus
  >BnF - Brassica napus
MSFRDETEDARNDLRRPFIHTGSWYRMGSRQSSMMGSSQIIKDNSISVLACVLIVALGPIQFGFTCGYSSPTQAEITKDLGLTVSEYSVFGSLSNVGAMVGAIASGQIAEYIGRKGSLMIAAIPNIIGWLCISFAKDTSFLYMGRLLEGFGVGIISYTVPVYIAEIAPQNMRGGLGSVNQLSVTIGIMLAYLLGLFVPWRILAVLGTLPCIVLIPGLFFIPESPRWLAKMGMTDDFETSLQVLRGFETDITVEVNEIKRSVASSTKRSSTVRFVDLKRRRYYFPLMVGIGLLVRQQLGGINGVLFYSSTIFESAGVTSSNAATFGVGAIQVVATAISTWLVDKAGRRLLLTISSVGMTISLVIVAAAFYLKGFVSPDSDMYSMLSILSVVGVVAMVVSFSLGMGPIPWLIMSEILPVNIKGLAGSIATLANWFFSWLITMTANLLLAWSSGATFTIYGVVCAFTVVFVTLWVPETKGKTLEELQALFR

SEQ ID NO: 89 - protein, 488 aa, Brassica napus
  >BnG - Brassica napus
MSSRDETEEARNELRRPFMHTGSWYRMGSRQSSMMGSSQVIKDNSISVLACVLIIALGPIQFGFTCGYSSPTQAAIIKDLGLTVSEYSVFGSLSNVGAMVGAIASGQIAEYIGRKGSLMIAAIPNIIGWLCISFAEDTSFLYMGRLLEGFGVGIISYTVPVYIAEIAPQNMRGGLGSVNQLSVTIGIMLAYLLGLFVPWRILAVLGTLPCIVLIPGLFFIPESPRWLAKMGMTDDFETSLQVLRGFETDITVEVNEIKRSVGTSTKRSSTVRFVDLKRRRYYFPLMVGIGLLVLQQLGGINGVLFYSSTIFESAGVTSSNAATFGVGAIQVVATAISTWLVDKAGRRLLLTISSVGMTISLVIVAAAFYLKEFVSHDSDMYSMLSILSVVGVVAMVVSFSLGMGPIPWLIMSEILPVNIKGLAGSIATLANWFISWLITMTANLLLAWSSGGTFTLYGLVCAFTVVFVTLWVPETKGKTLEELQALFR

SEQ ID NO: 90 - protein, 486 aa, Brassica napus
  >BnH - Brassica napus
MSDTEEARNNDLRRPFIHTGSWYRMGSRQSSMMGSSQVIRDSSISVLACVLIVALGPIQFGFTCGYSSPTQAAITKDLGLTVSEYSVFGSLSNVGAMVGAIASGQIAEYIGRKGSLMIAAIPNIIGWLCISFAKDTSFLYMGRLLEGFGVGIISYTVPVYIAEIAPQNMRGGLGSVNQLSVTIGIMLAYLLGLFVPWRILAVLGTLPCIVLIPGLFFIPESPRWLAKMGMTDDFETSLQVLRGFETDITVEVNEIKRSVASSTKRSSTVRFVDLKRRRYYFPLMVGIGLLVLQQLGGINGVLFYSSTIFESAGVTSSNAATFGVGAIQVVATAISTWLVDKAGRRLLLTISSVGMTISLVIVAAAFYLKGFVSHDSDMYSMLSILSVVGVVAMVVSFSLGMGPIPWLIMSEILPVNIKGLAGSIATLANWFFSWLITMTANLLLAWSSGGTFTLYAVVCAFTVVFVTLWVPETKGKTLEELQALFR

SEQ ID NO: 91 - protein, 417 aa, Brassica napus
  >BnI - Brassica napus
MSSRDETEEARNELRRPFMHTGSWYRMGSRQSSMMGSSQVIKDNSISVLACVLIIALGPIQFGFTCGYSSPTQAAIIKDLGLTVSEYSVFGSLSNVGAMVGAIASGQIAEYIGRKGSLMIAAIPNIIGWLCISFAEDTSFLYMGRLLEGFGVGIISYTVPVYIAEIAPQNMRGGLGSVNQLSVTIGIMLAYLLGLFVPWRILAVLGTLPCIVLIPGLFFIPESPRWLAKMGMTDDFETSLQVLRGFETDITVEVNEIKRSVGTSTKRSSTVRFVDLKRRRYYFPLMVGIGLLVLQQLGGINGVLFYSSTIFESAGVTSSNAATFGVGAIQVVATAISTWLVDKAGRRLLLTISSVGMTISLVIVAAAFYLKEFVSHDSDMYSMLSILSVVGVVAMVVSFSLGMGPIPWLIMSEVIRC

SEQ ID NO: 92 - protein, 468 aa, Brassica napus
  >BnJ - Brassica napus
  VARIANT 236: X = any natural amino acid
MKMSSASDGSREVREPLVDKDMAESKPEQTWMVYLSTFVAVCGSFAFGSCAGYSSPAQAAIRNDLSLTIAEFSLFGSLLTFGAMIGAITSGPIADLVGRKGAMRVSSAFCVVGWLAIFFAKGVVALDLGRLATGYGMGAFSYVVPIFIAEIAPKTFRGALTTLNQILICTGVSVSFIVGTMVTWRVLALIGLIPCAVSILGLFCIPESPRWLAKMGRDTEFEAALRKLRGKKANIXEEAAEIQDYIETLERLPKAKVLDLFQRRYIRSVFIAFGLMVFQQFGGINGICFYTSSIFEQAGFPTRLGMIIYAVLQVVITALNAPIVDKAGRKPLLLVSATGLVIGCLITAVSFYLKVHDMAHKAVPILAVVGIMVYIASFSAGMGAMPWVVMSEIFPINIKGVAGGMATLVNWFGAWAVSYTFNFLMSWSSYGTFVIYAVINALAIVFVIAVVPETKGKTLEQIQAVVNP

SEQ ID NO: 93 - protein, 489 aa, Helianthus annuus
  >HaA - Heliantus annuus
MSFRDENEDGRSDSHLKKPFLHTGSWYRMGSRQSSMMSSSQMIRDRSVSVLACVLIVALGPIQFGFTGGYSSPTQAAITRDLKLTVSEFSVFGSLSNVGAMVGAIASGQIAEYIGRKGSLMIAAIPNIIGWLCISFANETSFLYMGRLLEGFGVGIISYTVPVYIAEIAPQNMRGGLGSVTQLSVSIGIMLAYLLGLFASWRILAILGTLPCLILIPALFFIPESPRWLAKMGMTDDFEASLQVLRGFDTDITVEVNDIKRAVASSNRRAAIRFADLKQRRYWFPLMIGIGLLVLQQISGINGVLFYASNIFRSAGISNSDAATLALGAIQVIATGVATWLVDKTGRRILLTVSSAGMTLSLVVVAVSFFVKDFAEESSSLYTAMGILSVVGVVGMVIGFSLGMGPIPWVIMSEILPVNIKGLAGSIATLGNWFTSWVITMTAPLLLAWSGGGTFTLYMLLCVATLAFVSIWVPETKGKTLEEIQFSLR

SEQ ID NO: 94 - protein, 486 aa, Helianthus annuus
  >HaB - Heliantus annuus
MSFRHENEEGRDLRKPFLHTGSWYRMGSRQSSIMTSSQMIRDGSVSVLACVLIVSLGPVQFGFTGGYSSPTQSEISRDLKLTVSEFSVFGSLSNVGAMVGAIASGQIAEYIGRKGSLMIAAIPNIIGWLAISFAKDSSFLYMGRLLEGFGVGIISYTVPVYIAEIAPQNMRGSLGSVNQLSVTIGIMLSYLLGLFVHWRALAILGTFPCLILIPGLFFIPESPRWLAKMGMTDDFEASLQVLRGFETDITQEVNEIKRSVASSNRRATVRFSDLKQRRYWFPLTIGIGLLVLQQSTGTNGVLFYSSTIFQSAGISNSNVATFGLGAIQAIATAVSTWLVDRTGRRILLIVSSSGMTASLAIVASSFFIKGFVEESSTMYNVMGILSVIGVVGMIIGFSLGMGPIPWIIMSEILPVNIKGLAGSIATLANWFICWIVTLTAPLLLSWNDGGTFTLYMLMSAITVVFAGLLVPETKGKTLEEIQFSFR

SEQ ID NO: 95 - protein, 540 aa, Helianthus annuus
  >HaC - Heliantus annuus
MVGDSVFRRIISFPVSYAFRRTHRPHSHIPIFSSHLFFAKFPTVIFPMATRDPEIEEGGGGSSLKKPLLHTGSWYRMAGMSSRQSSMLASSAQMLRESVSIFLCVSIVALGPIQFGFTCGYSNPTQADIIMDLKLKISEFSMFGSLANVGAMVGAIASGQIAENIGRKGSLMIAAIPNILGWLAISFARDYSFLCMGRLLEGFGVGVISYTVPVYIAEISPQNLRGSLGSVNQLSVTIGILLAYLLGLFLPWRVLAVIGTLPCIILIPGLFFIPESPRWLAKMGFMEDCETSLQVLRGFDTDISTEFNEIKRSVATSGKRATIRISELKRRRFWYPLMVGIGLLLLQQLSGINGVLFYSSNIFKSAGISSSKAATFGLGAIQVVATAITTSLVDKSGRRALLLLSSFLMVASSLLASMSFFLKHLVSKDSSLYGFLGTLALIGLVIMVSGFSLGLGPIPWVIMSEILPVNIKSLAGSVATLFNWLAASIVTMTAPLLLDWSSGGTFLIYAAVSTFTLFFVKVWVPETKGKTLEEIQWSFR

SEQ ID NO: 96 - protein, 464 aa, Helianthus annuus
  >HaD - Heliantus annuus
MEQTETTVDEIGAPLIAQDGKSKEDNFMVYLSTFVAVCGSFAFGSCAGYSSPTQSAIREDLNLSLAEYSLFGSILTFGAMIGAVASGPMADFFGRKGALRISTAFCTVGWLAIYFAQGPLPLDVGRLATGFGMGVFSYVVPVFIAEIAPKSLRGALTAANQLMICTGVSVAFIIGTVLTWRILALTGLIPCAVLLVGLFFVPESPRWLAKIGKHKEFEAALRKLRGKDADISEEAYEIQDYIETLQKLPKAKLFDLFQRRYLRSVTIGVGLMVCQQFGGINGICFYTSSIFESAGFPADIGTIIYAVLQVIITALNALFVDKAGRKPLLLVSGAGLVIGCLLTAISFYLKTYKIGLEAAPALAVTGILLYIASFSAGMGAVPWIIMSEIFPINIKGAAGSLATLTNWFGAWLISFTFNFLLSWSSYGTFLVYAAINLAGILFIIVMVPETKGRTLEQIQAAINA

SEQ ID NO: 97 - protein, 490 aa, Solanum tuberosum
  >StA - Solanum tuberosum
MSFREENSEDGRGGDLRKPFLHTGSWYRMGSAQTSSMLGSSQVIRDSSISVLACVMIVALGPIQFGFTSGYSSPTQTAIVNDLKLTVSEFSLFGSLSNVGAMVGAISSGQIAEYIGRKGSLMIAAIPNIIGWLSISFAKDLSFLYMGRLLEGFGVGIISYTVPVYIAEIAPQNLRGALGSVNQLSVTIGIMLAYLLGLFVNWRVLAVLGTLPCLALIPGLFFIPESPRWLAKMGLTEDFETSLQVLRGFDADISVEVNEIKRAVASTSRKSTIRFADLKQRRYWLPLMIGIGLLVLQQLSGTNGVIFYSSNIFLSAGISSSDAATLGFGAIQVVATAVSTWLVDKTGRRLLLIVSSVGMAVSLLVVAIAFFMKGFVDEDSTFYGVLGMISVVGVLLMIVSFSLGMGPIPWLIMSEILPVKIKGLAGSVATLSNWFFSWVITATAPLLLAWSSGGTFTLYTLMCVFTVAFVTIWVPETKGKTLEEIQFSFR

SEQ ID NO: 98 - protein, 486 aa, Solanum tuberosum
  >StB - Solanum tuberosum
MSFREENNEGDLKKPFLHTGSWYRMGSRQSSMMGSSQAIRDSSISVLACVLIVALGPIQFGFTCGFTSPTQIAITEDLKLTVSEFSLFGSLSNVGAMVGAISSGQISEYIGRKGSLMIAAIPNIIGWLAISFAKDPSFLYMGRLLEGFGVGIISYVVPVYIAEIAPQNMRGGLGSVNQLSVTIGIMLSYLLGLFVNWRLLAVLGALPCLALIPGLFFIPESPRWLAKMGLTEDFETSLQVLRGFEADITNEVNEIKRSVASSTNRRTAMRFADLKHRRYWFPLMVGIGLLILQQLGGINGVIFYSSNIFLSAGISSSNAATFGVGAIQVVATAVSTWLVDRTGRRILLIVSSAGMTVSLLIVSVAFYLKGYVSEDSTLYGVLGIISVVGVVFMIISFSLGMGPIPWLIMSEILPIKIKGLAGSTATLANWLFSWVITVTAPLLMAWSSGGTFTIYMVMCAFTVAFVAIWVPETKGRTLEEIQFSFR

SEQ ID NO: 99 - protein, 484 aa, Solanum tuberosum
  >StC - Solanum tuberosum
MSFRDDTTADDGLRKPLLHTGSWYRMSSRQSSMMGSSAQILHESISIYLCVLIVALGPIQFGFTCGYSNPTQSEITSDLGLTISEFSIFGSLANVGAMVGAIASGQISEYIGRKGTLMIASIPNIIGWLAVSFATDVSFLYMGRLLEGFGVGIISYVVPVYIAEISPKNMRGVLGSINQLSVTVGIMLVYLLGLFVSWRVLAVIGMLPCMVLIPGLFFIPESPRWLAKNGLNEDFETSLQVLRGFDTDISSEVNEIKKSVRSSTKKVTIRFSELKIRRYYYPLLVGIGLLALQQLSGINGVLFYSSNIFKSAGISSSKAATFGIGAIQVIVTGISASLVDKAGRRLLLIVSSSVMTASSLLVAMSFFLKEFTPENWHSFFAVLSLVGLVALVMAFGVGLGSIPWIIMSEILPVSIKSLGGSVATLANWFSAWIVTMTANLLLTWSKGGTFAIYALVSAFTVVFVRLWVPETKGKTLEEIQQSFR

SEQ ID NO: 100 - protein, 464 aa, Solanum tuberosum
  >StD - Solanum tuberosum
MSFRDDTTADDGLRKPLLHTGSWYRMSSRQSSMMGSSAQILHESISIYLCVLIVALGPIQFGFTCGYSNPTQSEITSDLGLTISEFSIFGSLANVGAMVGAIASGQISEYIGRKGTLMIASIPNIIGWLAVSFATDVSFLYMGRLLEGFGVGIISYVVPVYIAEISPKNMRGVLGSINQLSVTVGIMLVYLLGLFVSWRVLAVIGMLPCMVLIPGLFFIPESPRWLAKNGLNEDFETSLQVLRGFDTDISSEVNEIKKSVRSSTKKVTIRFSELKIRRYYYPLLVGIGLLALQQLSGINGVLFYSSNIFKSAGISSSKAATFGIGAIQVIVTGISASLVDKAGRRLLLIVSSSVMTASSLLVAMSFFLKALVMAFGVGLGSIPWIIMSEILPVSIKSLGGSVATLANWFSAWIVTMTANLLLTWSKGGTFAIYALVSAFTVVFVRLWVPETKGKTLEEIQQSFR

SEQ ID NO: 101 - protein, 470 aa, Solanum tuberosum
  >StE - Solanum tuberosum
MSFREDYASNSDENSIRKPLLLPTKGKDVTRTSFRDDSAICEDGLRKPSLHTGSWYRMSSRQSSMMESSAQILRESVSIYLCVLIVALGSFQFGFTLGYTNPTQSDIMNDLILSISEFSIFGSLANVGAMVGAIASGQISEYIGRKGTLMIAALPNISGWFAISIARVSVGIMVAYLLGLFASWRVLAVIGMLPCMVLIPGLFFIPESPRWLAKMGNFEDFETSLQVLRGFDTDISLEMNEIKKSVGSSSKKATIHFSELKRRRYYYPLLIGIGLLSLQQLSGINGILMYSSNIFKSAGVSSSKAATFGLGAIQVVVTAIAASLVDKAGRRVLLIMSSSLMTVSSFLVATAFYLKDFAPKSWHPALGILSLVGLVVLVMAFALGLGSIPWIIMSEILPVDIKSLGGSVATLANWLTSWVVTMTANLLLSWSEGGTFIIYTMVSASTVVFVRIWVPETKGKTLEEIQRFFR

SEQ ID NO: 102 - protein, 465 aa, Solanum tuberosum
  >StF - Solanum tuberosum
MERPERTEVGFTTTDPLLSTGGDTPASATLAVVFSTLVAVSGSFVFGSAVGFSSPAQNGIIKDLDLSVAEYSVFGSIWTIGAMIGAVMSGKLADLFARRGAMGFSELFCLLGWLAIIFGKNALWLDIGRLLMGYGVGIISYVVPVYIAEITPKNLRGAFTTVNQLMICCGVSLMYVVGVIINWRLLAVIGAIPCIIQLLGLFFIPESPRWLAKAGQWKECEASLQRLRGKDANISEEAAEIKEYTETLQKLSEAKLIDLFHKKYAHSLIVGVGLMVLQQFGGVNAIAYYASSIFESAGFSGRIGSIAMVVVQIPMQVLGVLLMDKSGRRPLLMVSAAGTCLGCFLLGSSFLLQDLQLWKSSPFLALVGILVFTGSFSLGMGGIPWVIMSEIFPINVKGLAGSLVTVINWFGSWIVSYSFNFLMLWSSEGTFFIFSAVCGVTVMFVAKLVPETKGRTLEEIQSSFT

SEQ ID NO: 103 - protein, 506 aa, Zea mays
  >ZmA - Zea mays
MSFRDQESGGEDGGRTSSASDLRKPLINTGSWYRMPPAGGVMGSRQSSLMERLGSSAFSLRDVAISATLCTLIVALGPIQFGFTCGYSSPTQDAIIADLGLSLSEFSLFGSLSNVGAMVGAISSGQLAEYIGRKGSLMIAAIPNIIGWLAISFAKDSSFLFMGRLLEGFGVGVISYTVPVYIAEIAPQDQRGALGSVNQLSVTIGILLAYLFGMFVPWRILAVLGILPCSILIPGLFFVPESPRWLAKMGKMEDFEYSLQVLRGFQTDITAEVNEIKRSLASSRRRTTIRFADIKQKRYSVPLVIGIGLLVLQQLSGVNGILFYAASIFKAAGITNSNLATFGLGAVQVIATGVTTWLTDKAGRRLLLIISTTGMVITLVIVSVSFFVKDNIAAGSHLYSVMSMLSLAGLVAFVIAFSLGLGAIPWIIMSEILPVNIKSLAGSVATLANWLTAWAITMTASLMLNWSSGGTFAIYAVVSTMALIFVCLWVPETKGRTLEEIAFSFR

SEQ ID NO: 104 - protein, 500 aa, Zea mays
  >ZmB - Zea mays
MGGGSNRGGAGAGEESGSDHDGVLRRPLLNTGSWYRMSSRQSSFAPGTSSMAVLRESHVSAFLCTLIVALGPIQFGFTSGFSSPTQDAMVRDLNLSISEFSAFGSLSNVGGMVGAIASGQMAEYIGRKGSLMIAAIPNIIGWLAISFAKDASFLYMGRLLEGFGVGIISYTVPVYIAEISPQNMRGALGSVNQLSVTFGIFLAYLLGMFIPWRLLAVIGALPCTMLIPGLFFIPESPRWLAKMNLTEDCETSLQVLRGFETDITTEVNDIKRAVASSSKRTTISFQELNQKKYRTPLLLGIGLLVLQNLSGINGVLFYASSIFKAAGVTNSDLATCSLGAIQVLATGVTTWLLDRAGRRILLIISTSGMTLCLLAVSVVFFLKDNISQDSNSYYILTMISLVGIVSFVITFSFGMGAIPWLMMSEILPVSIKSLGGSIATLANWLTSFAITMTTNLMLTWSVGGTFLSYMVVSAFTIVFVVLWVPETKGRTLEEIQFSFR

SEQ ID NO: 105 - protein, 496 aa, Zea mays
  >ZmC - Zea mays
MASDGDHGGALQKPLLPKAPRSGGWFRKGTSTARLGAAAAGTSSKAAALRPPHHVPALLCTLVVALGTVQFGFTSGYSSPAQDGVTRDLDLSISEFSVFGSLSNVGAMVGAIASGQMAKYVGRRGSLMIAAVPNVMGWLAISLARDTSFLYVGRLLEGFGVGVISYVVPVYVAEISPQNMRGALGAVNPLSATFGVVFADVLGLFFPWRLLALIGTLPCLLLIPGLFFIPESPRWLARMNMMDECEASLQVLRGVDADITVEANDIKIAVASANKSGAMSFQELNQKKYRTPLILGMGLLVLQQLSGINGIIFYAGSIFKAAGLKNSNLDTCILGVIAVLATAVTTKILDRAGRRILLIISSFGMTLSLLVVAVVFYIKDNISHDSDLGNTLSMVSLVGVLAYVTAYSFGMGAIPWIIMAEILPVSIKSVAGSFATLANWLTSFGITMTANLLLSWSAAGTFAFYMMVSAFTLVFVILWVPETKGRTLEEIQWSFQ

SEQ ID NO: 106 - protein, 499 aa, Zea mays
  >ZmD - Zea mays
MASDGDHGGALQKPLLPKAARGGGWFRKGTSTAHPSGLSAAAAGTSSKAAALRPTHHVPALLCTLVVALGPIQFGFTTGYSSPAQDGVTRDLNLSISEFSAFGSLSNVGAMVGAIASGQMAKYVGRRGSLMIAAVPNIMGWLAISLARDTSFLYMGRLLEGFGVGVISYVVPVYIAEISPQNMRGALGVVNPLSITFGAMLAYVLGLFFPWRLLALIGTLPCLLLIPGLFFIPESPRWLARMNMMDECETSLQVLRGIDADTTAEVNDIKVVVTSTNKSGTIRFLELNQKKYRTPIILATGLLVLQQLSGMNGIIFYSGSIFKAAGLKNSNLDTCVLGAIGVLASVVTTKILDRAGRRILLIISSSGMTLSLLTVAVVFYIKGNISHDSDLGNTLSMVSLIGVLACVTAYSFGMGAIPWIIMAEILPVSINSVAGSFATLANWLTSFGITMTANLLLSWSAAGTFALYMMVSAFTVVFVILWVPETKGKTLEEIQWFFQ

SEQ ID NO: 107 - protein, 594 aa, Zea mays
  >ZmE - Zea mays
MGPRRDLPPITSFTTATRLAHSMEVVGLPRFVSCHSSSSSPVSLSIHPIPPGEKRDKSNLAASWALSAGAMASNSAPGAGYECGSDNDGGLHKPLLPNSGSCQRTGSRQPSLNAAGTSSRAVLRESHVSAFLCTLIVALGPIQCGFTSGYSSPTQDGIIRDLNLSISEFSAFGSLSNVGAMVGAIASGQMAKYIGRRGHLTSLVTVSQSLIIAAVPNIMGWLAISFAKHTSFLYMGRLLEGFGVGVISYVVCIIKLHAWLCLEKISPQNMRGALGAVNPLSATFGVMFVYVLGLFFPWRLLALIGTLPCLFLIPGLFFIPESPRWLARMNRMDDCETSLQVLRGFNADITAEANDIKASMQIAVTSANKSGTISFQELNQKKNRTPLILGIGLLVLQQLSGINCIVFYSGSIFKAAVLQGSRTATWTHVYLELSRQVLATGVTITFLDRAGRRILLIISSCGMTLSLLAVAVVFYIKDNISHDSDMHNILSMVSLVGVVAYVIAFCFGMGAIPWIIMSEILPVSIKSVAGSFATLANWLTSFGITMTANLLLSWSAAGTFASYMVVSAFTLMFVILWVPETKGRTLEEIQWSFQ

SEQ ID NO: 108 - protein, 483 aa, Zea mays
  >ZmF - Zea mays
MAGPMEREGRDAAEKPLLVRVGGSGGSQGGSASSSSVAVVVGCTAIAVAGSFEFGMSIGYSSPTQLGIMRDLRLSLAEYSVFGSILTIGAMLGAIVSGSVADRAGRRGAMAISDVLCALGYLLIGFSQSYWWLDIGRVLIGCGIGILSYVVPVYISEITPKDLRGGFATVNQFMICCGGSLAFVLGTFIAWRTLAIVGVVPCLVQLVGLLLIPESPRWLARFGHPGAFTGALQTLRGHGTDISEEASEIKVFTEKLQRLPKSKMLDLFQKEYIRAVIAGVGLMALQQLGGVNGVLFYASEVFVSAGFSSGNTGTVAMAVVQVPMVGLGVLLMDKAGRRPLLMISAAGTCVGCLLVGLSFLSKEQHWERDLNVLALAGLLVFIGSFSLGMGGIPWVIMSEIFPINMKGSAGSLVTLVSWLGSWIVSYAFNFLLIWSSYGTFFIFAAICGLTVVFVHRLVPETKGRTLEEIQASMNSSLTPFHKY

SEQ ID NO: 109 - protein, 476 aa, Oryza sativa
  >OsA - Oryza sativa
MNGGGSRRGGASCADESGSDQDGGSGGGLRKPLLNTGSWYRMGSRSSLAASSMAAIRESHVSAFLCTLIVALGPIQFGFTSGFSSPTQDAIIRDLKLSISEFSAFGSLSNVGAMVGAIASGQMAEYIGRKGSLIIAAVPNIIGWLAISFAKDASFLYMGRLLEGFGVGVISYTVPVYIAEISHQNTRGALGSVNQLSVTIGILLAYLLGMFVPWRLLAVIGSIPCTLLIPGLFFIPESPRWLAKMKMMDDFEASLQVLRGFETDITAERAVASANKRTTVRFKELNQKKYRTPLLIGTGLLVLQNLSGINGILFYASRIFRDAGFTNSDLATCALGAIQISTAGMTLSLLAVSVVFFLEGNISHDSHSFYILSMISLVALVAYIITFSFGMGAIPWVMMSEILPVSIKSLGGSFATLANMLTSWAITMTANLLLSWSAGGTFLSYMIVSAFTLVFVIFWVPETKGRTLEEIQFSFC

SEQ ID NO: 110 - protein, 447 aa, Oryza sativa
  >OsB - Oryza sativa
MNRGGGVGVGDESGSDYESGGGMRKPLLMHTGSWYRMGSRQGSLTGAGTSSMAILRESHVSAFLCTLIVALGPIQFGFTGGFSSPTQDAIIRDLDLTLSEFSVFGSLSNVGAMVGAIASGQMAEYIGRKGSLMIAAIPNIIGWLAISFAKDSSFLYMGRLLEGFGVGVISYTVPVYIAEISPQNMRGALGSVNQLSVTVGILLAYLLGMFVPWRLLAVIGILPCTVLIPGLFFIPESPRWLAKMNMMDDFETSLQVLRGFETDISAEVNDIKVASSKQQSYFSRFGFVTRKISSGLTNSDLATCALGAIQISSAGMTLSLLAVAVVFFLKDSISQDSHMYYTLSMISLVALVAFVIAFSFGMGAIPWIIMSEILPVSIKSLAGSFATLANWLTSFGITMTANLMLSWSAGGTFVSYMVVSAFTLVFVILWVPETKGRTLEEIQWSFR

SEQ ID NO: 111 - protein, 411 aa, Oryza sativa
  >OsC - Oryza sativa
MSFRGEESGGEDGGRTASASDLRKPFLHTGSWYKMSSAGGGGGMGSRLGSSAYSLRDSSVSAVLCTLIVALGPIQFGFTCGFSSPTQDAIISDLGLTLSEFSLFGSLSNVGAMVGAIASGQIAEYIGRKGSLMIAAIPNIIGWLAISFAKVPVYIAEIAPQTMRGALGSVNQLSVTIGILLAYLLGMFVPWRILSVLGILPCSILIPGLFFIPESPRWLAKMGKMEDFESSLQVLRGFETDIAVEVNEIKIGIGLLVLQQLSGVNGILFYAASIFKAAGLTNSNLATFGLGVVQISTTGMTITLVVVSVSFFVKDNITNGSHLYSVMSMLSLVGLVILPVNIKSLAGSVATLANWLTAWLITMTASLMLSWSNGGTFAIYAAVCAGTLVFVCLWVPETKGRTLEEIAFSFR

SEQ ID NO: 112 - protein, 524 aa, Oryza sativa
  >OsD - Oryza sativa
MGIVRAAEDVEGAVVAGAAGGGGGGGGGEVTAPLLLRQHKQGRGDEEKIQNDAGGDGGGRRGGGGGGSMSMLMLSTAVAVCGSFEFGTCVGYSAPTQSGIVDEVGLSISQFALFGSVLTIGAMIGAVTSGRLADFLGRKMVCHIFRLSQTMRISATICIFGWLSLHLAKGVIMLYFGRILLGFSTGILSYVVPVFIAEIAPKNLRGGLATSNQLLICSGSSATYIIGALVAWRNLVLVGIVPCVLLLTGLLFIPESPRWLANVGREKEFHASLQMLRGEDADVSEEAVEIKEYIESLHRFPKARVQDLFLRKNIYAVTVGVGLMIFQQLGGINGVGFYASSIFTSAGFSGKLGTILIGIIQIPITLFGAILMDKSGRRVLLMVSASGTFLGCFLTGISFYLKAQGLFSEWVPELALTGILVYIGAYSIGMGPVPWVVMSEIFSIDMKAIGGSLVTLVSWLGSFAISYSFSFLMDWSSAGTFFMFSAASLITILFVVMVVPETKGRTLEEIQDSLIDSRSRLRDP

SEQ ID NO: 113 - protein, 402 aa, Oryza sativa
  >OsE - Oryza sativa
MGVSSGASESLLPRAGGDGSLAMVIASTGVAVLGSFVFGVSIGYSAPTQSKIREDLQLSLSEYSVFGSIITIGAMIGAVASGHLADISGRKGVPVFIAEIAPKALRGGLTTLNQLLVCTGLSVTYIVGTMVTWRMLVIAGLVPSIILIVGLSFIPESPRWLAKVGRQKEFEIALQRLRGKDADVSIEAAEIKEFIETIENLPKAGVQDLFNRAYIRPVIVGVGLMVFQQFVGINGILFYASETFVSAGFASGDLGTILMGCIQAPITAVGALLMDRSGRRPLLLISTSGLLIGSLMSAVSFYLKVYIASYSIGMGAVPWVIMSEIFPINIKGIGGSFVTLVNWSGSWAVSFAFNFFMSWSSSGTFFLFALVCAVAILFIVKIVPETKGKTLEEIQASMNSST

SEQ ID NO: 114 - protein, 544 aa, Oryza sativa
  >OsF - Oryza sativa
MMAAAFPLSTAAPPSPPLVLRRSAAAAYSPSSPFELYRNHRRPARRVHCAASASAAARRRDACCALRPPAAARGGAAAAQGQAGAAPHGGAGEGSLWMVFLATAVAVCGSFEFGTCVGYSAPAQAGIVNDFGLSNSEYGVFGSVLTIGAMIGALTSGRLADSLGRKTTMGLAAIIGIVGWFTIYFANVPVFISEIAPKDLRGGLASSNQLFICSGCSAAYIIGALLSWRSLVLVGLVPCAFLLVGLLFIPESPRWLANTGRVKEFNASLQKLRGENADISEEAAGIREYIESLRSLPEARVQDLFQRKNLFAVIVGVGLMVFQQLGGINALGFYTSYIFSSAGFSGKLGTTLIGIFQVGFMSFLSMKIPLTLFGALLMDRSGRRALLLVSASGTFLGCFLTGLSFYFKAQGVYAQLVPTLALYGISVYYAAYSVGMGPVPWVIMSEVGKRNTVKLILYSYYAPVFLEIFSIEIKAIAGSLVTLVSWIGSFAISYSFNFLMDWNSAGTFFLFSAASLVTVLFVARTIMAREHNNMTIASRHDLER

SEQ ID NO: 115 - protein, 503 aa, Hordeum vulgare
  >HvA - Hordeum vulgare
MNGGSSGRAGGGGGGGYESGSDHDTRKQPLLVNTGSWYRMGSRQSSLTAGTSSMAIMRESHVSAFLCTMIVALGPIQFGFTGGFSSPTQDAIIRDLNLSISEFSVFGSLSNVGAMVGAIASGQMAEHIGRKGSLMIAAIPNIIGWLAISFAKDTSFLYMGRLLEGFGVGVISYTVPVYIAEISPQNMRGALGSVNQLSVTIGIVLAYILGMFVPWRMLAVIGILPCTILIPGLFFIPESPRWLAKMNKMEDFETSLQVLRGFETDITSEVNDIKRAVTSANKRAAIRFQELNQKKFRMPLILGIGLLVLQQLSGINAILFYASSIFKAAGITNSDLATCGLGGIQVLATLVTTWLLDRAGRRILLIISSAGMTLSLLAVAVVFFIKDTVSQDSHMYYILSMVSLLAIVAYVIAFSFGMGAIPWVIMSEILPVSIKSLAGSFATLANWLTSFGITMTANLLLSWSAGGTFVSYMLVSAFTLVFVVLWVPETKGRTLEEIQWSFR

SEQ ID NO: 116 - protein, 503 aa, Hordeum vulgare
  >HvB - Hordeum vulgare
MNGGSSGRAGGGGGGGYESGSDHDTRKQPLLVNTGSWYRMGSRQSSLTAGTSSMAIMRESHVSAFLCTMIVALGPIQFGFTGGFSSPTQDAIIRDLNLSISEFSVFGSLSNVGAMVGAIASGQMAEHIGRKGSLMIAAIPNIIGWPAISFAKDTSFLYMGRLLEGFGVGVISYTVPVYIAEISPQNMRGALGSVNQLSVTIGIVLAYILGMFVPWRMLAVIGILPCTILIPGLFFIPESPRWLAKMNKMEDFETSLQVLRGFETDITSEVNDIKRAVTSANKRAAIRFQELNQKKFRMPLILGIGLLVLQQLSGINAILFYASSIFKAAGITNSDLATCGLGGIQVLATLVTTWLLDRAGRRILLIISSAGMTLSLLAVAVVFFIKDTVSQDSHMYYILSMVSLLAIVAYVIAFSFGMGAIPWVIMSEILPVSIKSLAGSFATLANWLTSFGITMTANLLLSWSAGGTFVSYMLVSAFTLVFVVLWVPETKGRTLEEIQWSFR

SEQ ID NO: 117 - protein, 499 aa, Hordeum vulgare
  >HvC - Hordeum vulgare
MNGGGGGDDSGSDHEGGGAGARKPLLLKNTGSWYRMAGSSSRQSVGASSMAVLRESHVSALLCTLIVALGPVQFGFTCGFSSPTQDAMIRDLGLSISQFSAFGSLSNVGAMVGAIASGQMAEHIGRKGSLMIAAIPNIIGWLAISFANDSSFLYMGRLLEGFGVGVISYTVPVYIAEISPQSTRGALGSVNQLSITLGIFLAYVLGMFVPWRLLAVLGTLPCTLLIPGLFFIPESPRWLAKMNLMDDFETSLQVLRGFETDITAEVNDIKRAVASANKKATVRFQELNQKKYRTPLLIGTGLLVLQNLCGINGILFYASRIFRAAGFTNGDLATCALGAIQVLATGVTTSLLDKAGRRMLLIISTAGTTLSLLAVSVAFFLKDNLPHDSHSDYILSMVSLVALVAYIITFSFGMGAIPWLIMSEILPVGIKSFAGSFATLANMLTSFGVTMTANLLLSWSAGGTFASYMVVSAFTLVFVILWVPETKGRTLEEIQWSFR

SEQ ID NO: 118 - protein, 477 aa, Hordeum vulgare
  >HvD - Hordeum vulgare
MSTEWERVEAKKPLLVSGNIRASSIWVVVASTAVAVAGSFVFGISVGYSSPSQEGIMRDLHLSLAEYSVFGSILTIGAMLGAILSGTIADRVGRRCAMAISDVFCILGYLFIVFSKNSVWLDLGRLSIGCGIGLLSYVVPVYISEITPKNLRGRFAAVNQLMICCGASLAYALGTCITWRTLAIVGVTPCLLQLVGLLVIPESPRWLANIGRPGALEEALQKLRGKETDVTEEAADIKDFTEKLHHLPQSKILDLFQKDYIHAVTVGVGLMVLQQFGGVNAICFYASEIFVSAGFSSGNTGMLAMVAVQIPMTALGVLLMDKAGRRPLLMVSAAGTCLGCLLVGLSFLSKEHHWAKNLNVVLALAGILVFTGSFSLGMGGIPWVIMSEIFPIHMKGSAGSLVTLVSWLGSWIVSYAFNFLLLWSSYGTFFMFASICGLTIVFVDQLVPETKGRTLEEIQASMNTSLAPVSSGINQVA

SEQ ID NO: 119 - protein, 499 aa, Secale cereale
  >ScA - Secale cereale
MSFRDESGGEDGSGGRSSSASDLRKPFLHTGSWYRMSAAGGGAMDRLGSSAYGLRDSSISALLCTLIVALGPIQFGFTCGYSSPTQDAIMADLGLTLSEFSLFGSLSNVGAMVGAIASGQIAEYIGRKGSLMIAAIPNIIGWLAISFANDSSFLFMGRLLEGFGVGVISYTVPVYIAEIAPQNMRGALGSVNQLSVTIGILLAYTLGMFVPWRILSVLGILPCSILIPGLFFIPESPRWLAKMGKMEDFESSLQVLRGFETDISAEVNEIKRSVASSRRRTTIRFAEIKHKRYSVPLMIGIGLLILQQLSGVNGIFFYAASIFKAAGLKNSNLATCGLGAVQVVATGITTWLTDKAGRRLLLIISAVGMTVSLLVVSVSFFVKDNIDEASHLHSVMSILSLAALVAFVFAFSLGMGAIPWIIMSEILPVNIKSLAGSTATLNWMTSWLITMTASLMLNWSNGGTFAIYAAVSMGTLLFVCLCVPETKGRTLEEIAFSFR

SEQ ID NO: 120 - protein, 504 aa, Secale cereale
  >ScB - Secale cereale
MNGGSSGRAGGGGGGGGGYESGSDHDTRKQPLLVNTGSWYRMGSRQSSLTAGTSSMAIMRESHVSAFLCTMIVALGPIQFGFTGGFSSPTQAAIIQDLGLSISEFSVFGSLSNVGAMVGAIASGQMAEHIGRKGSLMIAAIPNIIGWLAISFAKDTSFLYMGRLLEGFGVGIISYTVPVYIAEISPRNMRGALGCVNPLSVTLGMVLAYVLGMLVPWRMLAVIGTLPCTILIPGLFFIPESPRWLAKMNKMDDFETSLQVLRGFETDITSEVNDIKRAVTSANKRAAIRFQELNQKKFRMPLILGIGLLVLQQLSGINAILFYASSIFKAAGITNSDLATCGLGGIQVLATLVTTWLLDRAGRRILLIISSAGMTISLLAVAVIFFIKDTVSQDSHMYYILSMVSLLAIVAYVIAFSFGMGAIPWVIMSEILPVSIKSLAGSFATLANWLTSFGITMTANLLLSWSAGGTFVSYMLVAFTLVFVILWVPETKGRTLEEIQWSFR

SEQ ID NO: 121 - protein, 495 aa, Secale cereale
  >ScC - Secale cereale
MNGKGGDGGGGRESGHDDDMRKPLLAASTGSWYRMGSSLTAGASSMAITRESHVSVLLCTLIVALGPIQFGFTGGFSSPTQDGITRDLSLSISEFSVFGSLSNIGAMVGAIASGQMVEHVGHKAALMIAAVPNILGWLAISLAKDTTFLYTGRLLEGFGVGIISYTVPVYIAEISPQNMRGALGSVNQLSVTIGIVLAYILGMFVPWRMLAVIGILPCTILIPGLFFIPESPRWLAKMNKMDDFETSLQVLRGFETDITSEVNDIKTAVASANKMTAIRFQELNQKKFRMPLILGIGLLVLQQLSGINAILFYAGSIFKAAGLTNSNLAACGLGAIALLATGATTWLLDRAGRRILLIISSAGMTLSLLAIAVIFFLKDNVSQDSDMYYILSMVSLFAIVAYVITFSFGMGAIPWVIMSEILPVSIKSLAGSFATLANWLTSFGITMTANLLLSWSAGGTFVCYTLVSAFTLVFVILWVPETKGRTLEEIQWSFR

SEQ ID NO: 122 - protein, 498 aa, Secale cereale
  >ScD - Secale cereale
MNGGGDESGSDHEGGGGGGTRKPLLLKNTGSWYRMAGSSSRQSVGASSMAVLRESHVSALLCTLIVALGPIQFGFTCGFSSPTQDAMIRDLGLSISQFSAFGSLSNVGAMVGAIASGQMAEHIGRKGSLMIAAIPNIIGWLAISFANDSSFLYMGRLLEGFGVGVISYTVPVYIAEISPQSTRGALGSVNQLSITLGIFLAYVLGMFVPWRLLAVLGTLPCILLIPGLFFIPESPRWLAKMNLMDDFETSLQVLRGFETDITAEVNDIKRAVASANKKATVRFQELNQKKYRTPLLIGTGLLVLQNLCGINGILFYASRIFRAAGFTNSDLATCALGAIQVLATGVTTSLLDKAGRRMLLIISTAGTTLSLLAVSVAFFLKDNLPHDSHSDYILSMVSLVALVAYIITFSFGMGAIPWLIMSEILPVGIKSFAGSFATLANMLTSFGVTMTANLLLSWSAGGTFASYMVVSAFALVFVILWVPETKGRTLEEIQWSFR

SEQ ID NO: 123 - protein, 471 aa, Secale cereale
  >ScE - Secale cereale
MAMAMGGDAAAEASEHLLGLPPARGGDGSSLGMVVASTGVAVLGSFAFGVAIGYSAPAEAGISRDLQLTLSEYSVFGSVITIGAMIGAVASGQIADVAGRKGAMRASALVSIVGWLAIFSAQSASSLDFGRFCTGIGVGLFSYVVPVFIAEIAPKALRGGLTALNPLMIGTGLSVTYIVGTVVSWRMLAMVGLAPCIILIAGLFFIPESPRWLAKVGRQKEFEIALQRIRGRDADVSLEAAEIKDFVETIDTLPKAGIQDLFSRPYIRPVVIGAGLMVFQQFAGINGILFYAGETFVSAGFDSGNLGTILIACIQLPLTTLGALLMDRSGRKPLLLISTGLLVGTLMSAVSFYLKIHGIFPKQVPIVALTSILVYIASYSLGMGSVPWVIMSEIFPINMKGIGGSFVTLVNWLASLAVSFAFNFLMSWSASGTFFFFAFVCAMAILFIVKVVPETKGKTLEEIQASINCST

SEQ ID NO: 124 - protein, 507 aa, Sorghum bicolor
  >SbA - Sorghum bicolor
MSFRDQESGGEDAGRTSSASDLRKPLLNTGSWYRMPPPGGMMGSRQSSLMERLGSSAFSLRDVAISATLCTLIVALGPIQFGFTCGYSSPTQDAIIADLGLSLSEFSLFGSLSNVGAMVGAISSGQLAEYIGRKGSLMIAAIPNIIGWLAISFAKDSSFLFMGRLLEGFGVGVISYTVPVYIAEIAPQDQRGALGSVNQLSVTVGILLAYLFGMFVPWRILAVLGILPCSILIPGLFFVPESPRWLAKMGKMEDFEYSLQVLRGFQTDITAEVNEIKRSVASSRRRTTAIRFADIKQKRYSVPLAIGIGLLVLQQLSGVNGILFYAGSIFKAAGITNSNLATFGLGAVQVIATGVTTWLTDKAGRRLLLIISTTGMVITLVIVSVSFFVKDNITAGSHLYSAMSMLSLAGLVAFVIAFSLGLGAIPWVIMSEILPVNIKSLAGSVATLANWLTAWAITMTASLMLNWSNGGTFAIYAAVSAMALIFVCLWVPETKGRTLEEIAFSFR

SEQ ID NO: 125 - protein, 499 aa, Sorghum bicolor
  >SbB - Sorghum bicolor
MGGGGSNRGGAGEESGSDHDGGLRKPLLHTGSWYRMSSRQSSVAPGASSMAVLRESHVSAFLCTLIVALGPIQFGFTSGFSSPTQDTMVRDLNLSISEFSAFGSLSNVGAMVGAIASGQMAEHIGRKGLLMIAAIPNIIGWLAISFAKDASFLYMGRLLEGFGVGIISYTVPVYIAEISPQNMRGALGSVNQLSVTFGIFLAYLLGMFVPWRLLAVIGALPCTVLIPGLFFIPESPRWLAKMNLMEDCETSLQVLRGFETDITTEVNDIKRAVTSSSKRTTISFQELNQKKYRTPLLLGIGLLVLQNLSGINGVLFYASNIFKAAGVTNSNLATCSLGAIQVLATGVTTWLLDRAGRRMLLIISTSGMTLCLLAVSVVFFVKDKTSQDSNSYYILTMISLVSIVAFVITFSFGMGAIPWLMMSEILPVSIKSLGGSIATLANWLTSFAITMTTNLMLTWSVGGTFLSYMVVSAFTLVFVVLWVPETKGRTLEEIQFSFR

SEQ ID NO: 126 - protein, 501 aa, Sorghum bicolor
  >SbC - Sorghum bicolor
MASNRASGSEYESGSDHDGALQKPLLPNSGSWYRMGMGSRQSSLNAAGTSSMAVLRESHVSAFLCTLIVALGPIQFGFTGGYSSPTQASIIRDLNLSISEFSVFGSLSNVGAMVGAIASGQMAEYMGRKGSLMIAAIPNVIGWLAISFAKDSSFLYMGRLLEGFGVGIISYVVPVYIAEISPQNMRGALGSVNQLSVTLGIMFAYLLGLFVPWRLLAVIGTLPCIVLIPGLFFIPESPRWLAKMNMMDDCETSLQVLRGFDADITAEVNDIKRAVTSANRRTTIHFQELNQKKYRTPLIIGIGLLVLQQLSGINGILFYASSIFKAAGLKDSDLDTFALGAIQVLATVVTTMFLDRAGRRILLIISSAGMTISLLVVAIVFYIKDNLSHDSDLYNILSMVSLVGVVAYVIAFSFGMGAIPWIIMSEILPVSIKSLAGSFATLANWLTSFGITMTANLLISWSAGGTFASYMIVSAFTLVFVIIWVPETKGRTLEEIQWSFR

SEQ ID NO: 127 - protein, 515 aa, Sorghum bicolor
  >SbD - Sorghum bicolor
MANNRASGDGGGGGAGYESGSDHDDALQKPLLRNSGCGYRIGMGSRQSCLNGAGTSIAVLRESHVPALLCTFIVALGPLQLGFTNGYSSPTQDGVVRDLNLSISEFSVFGSLPNVGAGRSRIVVGITLDAAVGGRRGCLVTISQSLMIAAIPNIMGWLAISLAKDTSFLYMGRLLEGFGVGVMSYVVPVYVAEISPQNMRGALGAVTTLSVTFGVMLAYVLGLFFPWRLLALIGTLPCLLLIPGLFFIPESPRWLARMNRMDECETSLQVLRGFDADITAEVNDIKIAAASANKSGTIHFQELNQKKYRTPLILGIGLLALQQLSGINGIIFYSGSIFKAAGLKNSNLDTCVLGAIGVVATGVTITFLDRAGRRILLIISSSGMTLSLLAVAVVFYIQDNISNDSDLYNILSMVSLVGVVACAIAYCFGMAAIPWIIMSEILPVSIKSVAGSFATLANWLTSFGVTMTANLLLSWSAAGTFASYMIVSAFTVMFVILCVPETKGRTLEEIQWSFQ

SEQ ID NO: 128 - protein, 491 aa, Sorghum bicolor
  >SbE - Sorghum bicolor
MACMAGPMEREGQEAAEKKPLLVRVVGSGSGDGQGGSASSSSSSVAVVVGCTAIAVAGSFEFGISVGYSSPTQLGIMRDLHLSLAEYSVFGSILTIGAMLGAVVSGSIADRAGRRGAMAISDILCALGYLLIGFSQNYWWLDIGRVLIGCGIGILSYVVPVYISEITPKNLRGGFATVNQFMICCGGSLAFVLGTFIAWRTLAIAGVAPCLLQLVGLLLIPESPRWLARFGHPGAFVVALQTLRGHGTDISEEASEIKVFTEKLQRLPKSKMLDLFQKDYIRAVTAGVGLMALQQLGGVNGILFYASEVFVSAGFPSGNTGTVAMAVVQVPMVGLGVLLMDKAGRRPLLMISAAGTCLGCLLVGLSFLSKEQHWERDLNVLALAGLVVFIGSFSLGMGGIPWVIMSEIFPINMKGSAGSLVTLVSWLGSWVVSYAFNFLLIWSSYGTFFIFATICGFTVVFVHRLVPETKGRTLEEIQASMNSSLTPFHKY

SEQ ID NO: 129 - DNA, 1464 bp, Brassica rapa
  >BrA - Brassica rapa
atgagtttcagggaggagacggaggagggaagaaatgatcttcggcgaccattcttacacacgggaagttggtaccggatgggttccagacagtctagcatgttggaatcatctcaagtcattcgagacagctccatctctgtcttagcttgtgttttgatcgttgcacttggtcctattcaattcggtttcacttgtggttattcttctccaactcaagctgatattactagggatcttggcttaactgtatcagagtactctgtgtttgggtctctatccaatgtgggtgctatggttggtgcaattgcgagtggtcagattgctgaatacatcggaagaaaagggtctctgatgattgctgcaattcccaatattattggctggctttcaatatcgtttgccaaagatacctcttttctgtacatgggaagattgttagaaggtttcggcgtggggatcatatcttatacggtgcctgtatatatagccgagatcgcaccacagaacatgagaggagccttaggttctgtaaaccagctttctgtaacaattgggataatgttggcatatctactcggtctctttgttccatggagaattcttgcagttttgggagtattgccgtgtacattattgatacctggtctgtttttcatccctgaatctcctcggtggctggcaaagatgggtttaacagatgattttgaaacttcgttgcaagttcttcgtggttttgatactgatatcaccattgaggttaatgagatcaagagatctgtggcatcatctacgaaacgctctgcaattcggtttgtagacctcaagcgtaggagatactatttcccactaatggttggtataggacttcttgtacttcaacaacttggaggaattaacggcgtcttgttctactcgagtacaatctttgaatctgcaggggtctcatcaagtaatgtagcaacatttggagttggtgctgttcaggtagtggcgactgcagtagcgacatggttggtggataaatcaggtcgccgacttctgctcatgatctcttctatagggatgacgattagcctggtgattgtagcagccgcattttaccttaaggaattcgtatcacctgactcggatatgtacaacattctaagcatggtctctgttgttggagttgtgactatggttattacttgctctctagggatgggaccaattccatggctgataatgtctgagattcttccagtgaatatcaaaggcttagccggaagtatagcaactttggctaactggtttgtctcgtggttagtcacaatgactgcaaatatgctcttagcttggagcagtggtggaacgtttactctctatgctttggtttgtggattcactgtggcttttgtgagtctttgggttcctgagaccaaaggcaaaacgcttgaagagattcaagctttgttcagatga

SEQ ID NO: 130 - DNA, 1464 bp, Brassica rapa
  >BrB - Brassica rapa
atgagtaacagagatgatacggaagagggaaggagtgatcttcgacgtcccttcttacacacgggaagctggtaccggatgggttccagacaatctagcatgttggaatcgtctcttgctattcgagacaactccatctctgtcctagcttgtgtcttgatcgttgctcttggtcctattcaattcggtttcacttgtggctattcctctccaactcaagctgctattactaaggatcttggcttaactgtatcagagtactctgtgtttgggtctctatccaatgtgggtgctatggttggcgcaattgcaagtggtcagattgcagaatacatggggagaaaagggtctctgatgattgctgccattcccaatattatgggctggctttctatagcttttgcaaaagatacttcttttctttacatgggaagactgttagaaggttttggcgttgggatcatctcttatacggtgcctgtatatatagccgagatcgctccacagaacatgagaggagcattaggttcagtaaaccagctttctgtaacagttgggataatgttggcatacttactcggtctctttgttccatggagaattcttgcagttttgggagtattgccatgtacattattgataccgggtcttttcttcattcctgaatctcctcggtggctggcaaagatgggtttgacagatgattttgaaacttccttgcaagttcttcgtggttttgatactgacattaccatcgaggttaatgaaatcaagagatctgtggcctcatctggcaaacgttctgctattcggtttgtggacctcaagcgtaggagatactattttccattgatggttggtataggactgcttgtacttcaacaacttggaggaatcaacggtgtcttgttctattcgagtacaatttttgcatctgcaggggtctcatcgagtaatgtggcaacatttggagttggtgctgttcaggtactggccactgcagtagctacatggctggttgataaatcaggtcgcagacttttgctcatgatctcttctatagggatgacgattagcctggtgattgtagcagtcgcgttttaccttaaggaatttgtatcacctgattccaatatgtataacattctaagcatggtctctgtagttggagttgtggctatggttattgcttgctctctaggaatgggaccaatcccatggctgattatgtctgagattcttccagtgaatataaaaggtttggccggaagtatagcaactttagccaactggttcgtctcttggttagtcacaatgactgcaaatatgctcttagcatggagcagtggaggaacttttaccctctatgctttggtctgtggattcactgtggcctttgtgtctctttgggttcctgagaccaaaggcaaaacgcttgaagagattcaagcattgttcagatga

SEQ ID NO: 131 - DNA, 1464 bp, Brassica napus
  >BnA - Brassica napus
atgagtttcagggaggagacggaggagggaaggaatgatcttcggcgaccattcttacacacgggaagttggtaccggatgggttccagacagtctagcatgttggaatcatcccaagtcattcgagacagctccatctctgtcttagcttgtgttttgatcgttgctcttggtcctattcaattcggtttcacttgtggttattcttctccaactcaagctgctattactagggatcttggcttaactgtatcagagtactctgtgtttgggtccctatccaatgtgggtgctatggttggtgcaattgcaagtggtcagattgctgaatacattggaagaaaagggtctctgatgattgctgcaattcccaatattattggctggctttcaatatcgtttgccaaagatacttcttttctgtacatgggaagattgttagaaggtttcggcgtggggatcatatcttatacggtgcctgtatatatagccgagatcgcgccacagaacatgagaggagccttaggttctgtaaaccagctttctgtaacaattgggataatgttggcatatctactcggtctctttgttccatggagaattcttgcagttttgggagtattgccgtgtacattattgatacctggtctgtttttcatccctgaatctcctcggtggctggcaaaaatgggtttaacagatgattttgaaacttcgttgcaagttcttcgtggttttgatactgatatcaccattgaggttaatgagatcaagagatctgtggcatcatctaccaaacgctctgcaattcggtttgtagacctcaagcgtaggagatactatttcccactaatggttggtataggacttcttgtacttcaacaacttggaggaattaacggcgtcttgttctactcgagtacaatctttgaatctgcaggggtctcatcaagtaatgtagcaacatttggagttggtgctgttcaggtagtggcgactgcagtagccacatggttggtggataaatcaggtcgccgacttctgctcatgatctcttctatagggatgacgattagcctggtgattgtagcagccgcattttaccttaaggaattcgtatcacctgactcggatatgtacaacattctaagcatggtctctgttgttggagttgtgactatggttattgcttgctctctagggatgggaccaattccatggctgataatgtctgagattcttccagtgaatatcaaaggcttagccggaagtatagcaactttggctaactggtttgtctcgtggttagtcacaatgactgcaaatgtgctcttagcttggagcagtggtggaacgtttactctctatgctttggtttgtggattcactgtggcttttgtgagtctttgggttcctgagaccaaaggcaaaacgcttgaagagattcaagctttgttcagatga

SEQ ID NO: 132 - DNA, 1464 bp, Brassica napus
  >BnB - Brassica napus
atgagtttcagggaggagacggaggagggaagaaatgatcttcggcgaccattcttacacacgggaagttggtaccggatgggttccaggcagtctagcatgttggaatcatctcaagtcattcgagacagctccatctctgtcttagcttgtgttttgatcgttgcacttggtcctattcaattcggtttcacttgtggttattcttctccaactcaagctgatattactagggatcttggcttaactgtatcagagtactctgtgtttgggtctctatccaatgtgggtgctatggttggtgcaattgcgagtggtcagattgctgaatacatcggaagaaaagggtctctgatgattgctgcaattcccaatattattggctggctttcaatatcgtttgccaaagatacttcttttctgtacatgggaagattgttagaaggtttcggcgtggggatcatatcttatacggtgcctgtatatatagccgagatcgcgccacagaacatgagaggagccttaggttctgtaaaccagctttctgtaacaattgggataatgttggcatatctactcggtctctttgttccatggagaattcttgcagttttgggagtattgccgtgtacattattgatacctggtctgtttttcatccctgaatctccccggtggctggcaaagatgggtttaacagatgattttgaaacttcgttgcaagttcttcgtggttttgatactgatatcaccattgaggttaatgagatcaagagatctgtggcatcatctaccaaacgctctgcaattcggtttgtagacctcaagcgtaggagatactatttcccactaatggttggtataggacttcttgtacttcaacaacttggaggaattaacggcgtcttgttctactcgagtacaatctttgaatctgcaggggtctcatcaagtaatgtagcaacatttggagttggtgctgttcaggtagtggcgactgcagtagcgacatggttggtggataaatcaggtcgccgacttctgctcatgatctcttctatagggatgacgattagcctggtgattgtagcagccgcattttaccttaaggaattcgtatcacctgactcggatatgtacaacattctaagcatggtctctgttgttggagttgtgactatggttattacttgctctctagggatgggaccaattccatggctgataatgtctgagattcttccagtgaatatcaaaggcttagccggaagtatagcaactttggctaactggtttgtctcgtggttagtcacaatgactgcaaatatgctcttagcttggagcagtggtggaacgtttactctctatgctttggtttgtggattcactgtggcttttgtgagtctttgggttcctgagaccaaaggcaaaacgcttgaagagattcaagctttgttcagatga

SEQ ID NO: 133 - DNA, 1464 bp, Brassica napus
  >BnC - Brassica napus
atgagtaacagagatgatacggaagagggaaggagtgatcttcgacgccccttcttacacacgggaagctggtaccggatgggttccagacaatctagcatgttggaatcgtctcttgttattcgagacagctccatttctgtcctagcttgtgtcttgatcgttgctcttggtcctattcaattcggtttcacttgtggttattcctctccaactcaagctgctattactaaggatcttggcttaactgtttcagagtactctgtgtttgggtctctatccaatgtgggtgctatggttggcgcaattgcaagtggtcagattgcagaatacatggggagaaaagggtctctgatgattgctgcaattcccaatattatgggctggctttctatatcttttgcaaaagatacttcttttctttacatgggaagactgttagaaggttttggcgttgggatcatctcttatacggtgcctgtatatatagccgagatcgctccacagaacatgagaggagccttaggttcagtaaaccagctttctgtaacagttgggataatgttggcatacttactcggtctctttgttccatggagaattcttgcagttttgggagtattgccatgtacattattgataccgggtcttttcttcattcctgaatctcctcggtggctggcaaagatgggtttgacagatgattttgaaacttccttgcaagttcttcgtggttttgatactgacattaccattgaggttaatgaaatcaagagatctgtggcctcatctggcaaacgttctgcaattcggtttgtggacctcaagcgtaggagatactattttccattgatggttggtataggactgcttgtacttcaacaacttggaggaatcaacggtgtcttgttctattcgagtacaatttttgcatctgcaggggtctcatcgagtaatgtggcaacatttggagttggtgctgttcaggtaatggccactgcagtagctacatggttggttgataaatcaggtcgcagacttttgctcatgatctcttctatagggatgacgattagcctagtgattgtagcagttgcgttttaccttaaggaatttgtatcacctgattccaatatgtacaacattctaagcatggtctctgtagttggagttgtggctatggttattgcttgctctctaggaatgggaccaatcccatggctgattatgtctgagattcttccagtgaatataaaaggtttagccggaagtatagcaactttggccaactggttcgtgtcgtggttagtcacaatgacagcaaatatgctcttagcatggagcagtggaggaacttttactctctatgctttggtctgtggattcaccgtggcctttgtgagtctttgggttcctgagactaaaggcaaaacacttgaagaaattcaagcattgttcagatga

SEQ ID NO: 134 - DNA, 1464 bp, Brassica napus
  >BnD - Brassica napus
atgagtaacagagatgatacggaagagggaaggagtgatcttcgacgtcccttcttacacacgggaagctggtaccggatgggttccagacaatctagcatgttggaatcgtctcttgctattcgagacagctccatctctgtcctagcttgtgtcttgatcgttgctcttggtcctattcaattcggtttcacttgtggctattcctctccaactcaagctgctattactaaggatcttggcttaactgtatcagagtactctgtgtttgggtctctatccaatgtgggtgctatggttggcgcaattgcaagtggtcagattgcagaatacatggggagaaaagggtctctgatgattgctgccattcccaatattatgggctggctttctatagcttttgcaaaagatacttcttttctttacatgggaagactgttagaaggttttggcgttgggatcatctcttatacggtgcctgtatatatagccgagatcgctccacagaacatgagaggagcattaggttcagtaaaccagctttctgtaacagttgggataatgttggcatacttactcggtctctttgttccatggagaattcttgcagttttgggagtattgccatgtacattattgataccgggtcttttcttcattcctgaatctcctcggtggctggcaaagatgggtttgacagatgattttgaaacttccttgcaagttcttcgtggttttgatactgacattagcatcgaggttaatgaaatcaagagatctgtggcctcatctggcaaacgttctgctattcggtttgtggacctcaagcgtaggagatactattttccattgatggttggtataggactgcttgtacttcaacaacttggaggaatcaacggtgtcttgttctattcgagtacaatttttgcatctgcaggggtctcatcgagtaatgtggcaacatttggagttggtgctgttcaggtactggccactgcagtagctacatggctggttgataaatcaggtcgcagacttttgctcatgatctcttctatagggatgacgattagcctggtgattgtagcagtcgcgttttaccttaaggaatttgtatcacctgattccaatatgtataacattctaagcatggtctctgtagttggagttgtggctatggttattgcttgctctctaggaatgggaccaatcccatggctgattatgtctgagattcttccagtgaatataaaaggtttggccggaagtatagcaactttagccaactggttcgtctcttggttagtcacaatgactgcaaatatgctcttagcatggagcagtggaggaacttttaccctctatgctttggtctgtggattcactgtggcctttgtgtgtctttgggttcctgagaccaaaggcaaaacgcttgaagagattcaagcattgttcagatga

SEQ ID NO: 135 - DNA, 1470 bp, Helianthus annuus
  >HaA - Heliantus annuus
atgagtttcagagacgaaaacgaagatggaagaagcgacagtcacctcaaaaaaccatttctccacacgggcagttggtaccgtatgggttctagacaatccagcatgatgtcgtcatctcagatgatccgagatcgttctgtttctgttcttgcctgtgttctcatcgttgcacttggtcctattcagtttggtttcactggtgggtattcgtcgcctacacaagctgctattactcgagatcttaaattaacggtttctgagttctctgtgtttgggtctttgtcaaatgtgggtgccatggttggggccatagctagtggtcaaattgccgagtatatcggccgaaaagggtctttgatgattgcagctattcctaatatcattggatggctttgtatatcgtttgccaacgagacgtcgtttctttatatgggaagattgttggaaggttttggtgttggaattatatcatacacggttcctgtctatatagcggaaatagcacctcaaaacatgagaggggggctaggttctgtcactcagctatctgtttcgatcgggataatgcttgcttatttgctgggactttttgctagttggagaatacttgcaatattgggaactttaccatgcttgattttgatccccgccctcttttttatccccgaatctcctcggtggctggcgaagatgggtatgactgatgattttgaagcttctttacaagttcttcgtgggtttgataccgatatcaccgttgaagtaaacgacataaagagggccgtagcatcatcaaacagaagagctgcgattcgctttgcagaccttaaacaaagaagatattggttccctttgatgataggaattggattacttgttcttcaacagataagcgggatcaatggcgttctcttctacgccagcaacatctttcgatccgcaggaatttctaatagtgatgctgctacattagcacttggggctatccaagttatcgcgacgggggttgccacgtggttggttgacaaaacgggccgtcggattctgctaaccgtttcctctgctggaatgactctcagtcttgtagtcgttgcggtttccttcttcgtcaaggatttcgcagaagagagttcttcgttgtatactgcaatgggtatcttatcagtggtcggagtcgtgggtatggtaattggattttcacttggaatggggcccattccatgggttataatgtctgagattcttcctgtgaatataaaaggacttgcagggagtatagcaacattaggcaattggtttacttcttgggtgattacgatgaccgcacctttgcttctagcatggagtggtggaggaaccttcactttgtacatgctactgtgtgtggctacgctcgcgtttgtgtccatttgggtgccagaaacaaagggaaagacattggaggagatacagttttccttgagataa

SEQ ID NO: 136 - DNA, 1461 bp, Helianthus annuus
  >HaB - Heliantus annuus
atgagtttcaggcatgaaaatgaggaggggagagacctcagaaaaccctttcttcatacaggcagttggtatcgtatgggttccagacaatctagcatcatgacttcatctcagatgatcagagatggctcagtttctgtgttggcatgtgtcctcatcgtttccttgggcccggttcagttcggtttcactggtggctattcttcacctacacaatcggaaatcagtcgagatcttaaacttacagtctctgagttctcggtgtttggttctttatcgaatgtgggtgccatggttggtgcgatagctagcggtcagattgcagagtatattggtcgaaaagggtctttgatgattgccgctatccctaatataatcggctggcttgccatatcatttgccaaagattcgtcatttctttacatgggaaggttactagaaggattcggtgttgggatcatatcttacacggttcctgtttatatagctgagatagcacctcaaaacatgagagggagtttaggttctgttaaccagttatcagttactattgggattatgctttcttatttgctgggactttttgttcattggagagcacttgcaattttggggacatttccttgtttaattctaatacctggactctttttcatcccagaatctcctaggtggttggcaaaaatgggaatgacagatgattttgaagcttctttgcaagttcttcgcggttttgaaactgatattacccaagaagtaaacgaaattaagaggtctgtggcatcatcaaacagaagagctacagttcgtttttcggatcttaaacaaagaagatattggttccctctgacgataggaattgggttacttgtacttcaacagtcaactggaaccaatggtgttctcttttattccagtaccattttccaatctgcaggaatttctaatagcaatgttgctacatttggacttggtgccatccaagccattgcaactgcagtttcaacatggttggttgacagaacgggccgaaggattctacttatagtctcttcttctggaatgactgctagtcttgcgatcgttgcatcatccttcttcattaagggctttgtggaggaaagttccaccatgtataatgtaatgggcatcttatcagtcattggagttgtgggaatgatcattggtttttctcttggaatgggaccaattccatggattataatgtctgagattcttccggtcaatataaaaggactcgctggaagtatagctacattagccaactggtttatctgttggatcgttacattaacagcccccttgcttttatcatggaacgacggaggaacattcactctatacatgcttatgagtgctataacggttgttttcgcgggccttttggtgccagagactaaaggaaaaacactcgaagagattcagttttcattccgatga

SEQ ID NO: 137 - DNA, 1473 bp, Solanum tuberosum
  >StA - Solanum tuberosum
atgagtttcagagaagaaaatagtgaagatggaagaggaggggatctgaggaagccatttttacatactggaagttggtatcgaatgggttcagcacaaacttctagcatgttgggttcttctcaagttatccgtgatagctcaatttcagttcttgcttgcgttatgattgttgctttgggtccaattcagtttgggttcacttctggttactcatcgcctacgcaaactgccatagtcaatgatctgaagctcacagtatctgagttctctttattcggttccttatctaatgtgggtgctatggttggggcaatatctagtggtcaaattgccgagtacattggacgaaaagggtctttaatgatagctgctatacctaacatcattggttggctttccatctcgtttgccaaagatctgtccttcttatacatgggaagattattggaaggttttggagttggcataatctcttacacggttcctgtatatattgccgagatagcacctcagaacctgagaggggccctggggtcagttaatcagctctctgttacaattgggatcatgttggcttatttgctaggactttttgttaattggagagtgctcgctgttcttggaacattgccctgccttgcactgatacctggactatttttcatcccagaatctcctcggtggttggccaaaatgggtctgacagaagattttgaaacctctttgcaagttctccgagggttcgatgctgacatttctgttgaagtaaatgaaattaagagggctgtagcatccacaagccgaaagtcaacgatacgttttgcagatctcaaacaaagaagatattggctgcctctcatgataggcattggactgcttgtcctacaacaactcagtggaaccaatggtgtgatcttctattccagtaacattttcctatcggccgggatttcttcaagtgatgctgcaactttaggttttggtgctatccaggtggttgccactgctgtttctacatggctggtggataaaactggccgtaggcttttactgatagtctcgtcggttggaatggctgttagtctccttgttgttgccattgcattctttatgaagggtttcgtagatgaggattctaccttctatggcgttctaggcatgatatcagtggttggtgttttgttgatgattgtttcattttcgcttggaatggggcctattccgtggcttataatgtctgagattcttccggttaagatcaaaggccttgctggaagtgtagcgacgttatccaattggttcttttcctgggtaattacagcaactgcaccgctgctattggcttggagcagtggaggaaccttcactctttatacgcttatgtgtgtgttcaccgtggcgtttgtgacaatttgggtacctgagacaaaaggaaaaacgctagaggaaatacagttttcgtttagatga

SEQ ID NO: 138 - DNA, 1461 bp, Solanum tuberosum
  >StB - Solanum tuberosum
atgagtttcagagaagagaacaatgaaggggatctgaaaaagccatttttacatactggaagttggtatcgtatggggtcaagacagtctagtatgatgggttcttctcaagctattcgtgatagttctatttctgttcttgcttgtgttctcatagttgctttgggcccaatccagtttggtttcacttgtggcttcacttcgcctacgcaaattgcaattaccgaagatctgaagctcactgtttctgagttctctttgttcggttctttatccaatgtgggtgctatggttggtgcaatatctagtggtcaaatttcagagtacattgggcgaaaagggtctttaatgatagctgctatacctaatatcattggttggcttgccatctcatttgccaaagatccttcatttctatacatgggaagattgttggaaggctttggtgtgggaataatctcttatgtggttcctgtatatattgctgagattgcacctcaaaatatgagagggggtctagggtctgttaaccagctctctgttacaattgggatcatgttgtcctatttactgggactttttgttaattggaggctgcttgctgttcttggagcattaccttgcctagcactgatacctggactatttttcatccccgaatctcctcggtggttggccaaaatgggtttaacagaagatttcgaaacttcattgcaagttcttcgagggtttgaggctgacattaccaatgaagtaaatgaaattaagaggtctgtagcatcatcaacaaaccgaagaacagcaatgcgtttcgcggatctcaaacataggagatattggtttcctctcatggtaggaattgggctacttatcctgcaacagttaggaggaatcaacggtgttatattctattccagcaacattttcctatctgccggtatttcttcaagtaatgctgcaacttttggtgttggtgctatccaggttgttgcaactgcagtttctacatggctggtggatagaactggacgtagaattttattaattgtttcctcggctggaatgactgttagtcttctaattgtctccgttgccttctatctaaagggttatgtatctgaggattctaccctctatggtgtattgggaataatatcagtagtcggggtggtgttcatgattatttcattctcgctcggaatgggaccaattccatggcttataatgtctgagattcttccaatcaagatcaaaggtctcgctggaagtacggcaacattagccaactggttattctcgtgggtaataacagtgactgcaccattgcttatggcttggagcagtggaggaaccttcactatttacatggttatgtgtgctttcaccgtggcgttcgtggcaatttgggtaccggagacgaaagggagaactctagaggaaattcagttttctttcagatga

SEQ ID NO: 139 - DNA, 1521 bp, Zea mays
  >ZmA - Zea mays
atgagcttccgggaccaggagagtggcggggaggatgggggcaggacgtcctccgcctccgacctgcggaagccgctcatcaacaccgggagctggtaccgcatgccgccggcgggtggcgtgatgggctcgcggcaatctagcctcatggagcgattgggctcctctgcgttctctctccgcgacgtcgctatctcggcgacgctctgcacgctcattgtcgcgctaggtcccatccagttcggtttcacatgtggctactcctcacccacgcaggacgccatcattgctgaccttggcctctccctctctgagttctccctcttcggttcattatctaatgtaggggcgatggtaggcgccatctccagtgggcaacttgcagagtatatcggccgcaaggggtctctcatgatcgctgcgattccaaacataattgggtggctcgcgatatcatttgcaaaagattcctctttcttgtttatgggtcggctgctagaaggatttggagttggtgtaatatcgtatacagtaccggtttatattgcagaaatcgctcctcaagatcagaggggagctcttggttctgtcaatcagctctccgtcacgattggtatattgcttgcctatttgtttggcatgtttgttccctggagaattcttgctgttctaggcattttaccctgttcaatcctgattcctggactgttctttgtccctgaatccccaaggtggttggcaaaaatggggaagatggaggattttgaatattcattgcaagttctgcgaggatttcagacagatatcacagcagaagtaaatgaaataaagagatcattagcatcatcgaggaggaggacaaccataaggttcgctgatatcaaacagaagagatacagtgttccccttgtgataggaatcggtctccttgtcctgcagcagctaagtggtgtcaatggcattctattttatgctgcgagcatcttcaaagctgctggtattacaaacagtaatctagcaacatttggtttaggggctgttcaggtgattgctactggagtgacaacctggttgactgacaaagctggtcgaaggcttcttctcattatttccaccacaggaatggtcattactcttgttattgtttctgtgtcattttttgtgaaggacaacatagctgctggttcgcacttatactctgtaatgagtatgctttcactggctggacttgtggcatttgtgattgcattttctcttggcttgggagcgattccgtggatcattatgtctgagatccttcctgttaacatcaagagccttgctggaagtgttgcgaccctggcgaactggctgacagcatgggccattacaatgacggcaagcctgatgttgaactggagcagtggaggaacctttgctatctacgccgtcgtgtctaccatggccctcattttcgtgtgcttgtgggtgcctgagaccaagggaagaacgctagaggaaatcgccttctcattccgctga

SEQ ID NO: 140 - DNA, 1503 bp, Zea mays
  >ZmB - Zea mays
atgggtggcggcagcaacagaggcggcgccggcgccggcgaggagagcggcagcgaccacgacggtgtgctgcggaggccgctgctcaacacggggagctggtaccggatgagctcgcggcagtccagctttgccccggggacctcctccatggccgtcctgcgcgagtcccacgtctccgccttcctctgcacgctcatcgtcgcgctcggccccatccagttcggcttcaccagcggcttctcctccccgacccaggacgccatggttcgggacctcaacctctctatctccgagttctcggcgttcggatcgctgtccaacgtcggcggcatggtcggggcgatcgccagcgggcagatggccgagtacattggccgtaaagggtcgttgatgattgctgcaatcccaaatatcatcggttggcttgcgatctcctttgcaaaagatgcctcatttctatatatgggacgattgcttgaagggtttggtgtcggcatcatatcctacacggtaccggtatacatagcagagatatctcctcagaacatgaggggagctcttggttctgtgaaccagttgtctgtgacctttggcatattcttggcctatttgctcggcatgtttattccttggagacttcttgctgtgattggagccttgccctgcacaatgttgattcctggactattcttcattccagaatctcccagatggctggcaaagatgaatttgacggaagattgtgagacgtccctacaagtgctgagggggtttgagactgacatcacaacagaagtgaatgatataaagagggcagtggcatcatcaagtaagaggaccacaatcagttttcaagaattaaaccaaaagaaataccgcacgccactacttctagggattggcctacttgtactgcaaaatcttagtggaatcaacggtgtactgttttatgcaagtagcatcttcaaagctgcaggggttacaaacagcgacttggccacctgttcacttggtgctattcaggtccttgctactggagttacaacatggctgttagaccgagctggacgacgcatccttctcattatttctacctctggcatgactctatgccttcttgccgtttctgttgtattttttctcaaggataacatttcacaggattctaactcatactacatcttaacaatgatctcccttgttggtattgtgtcttttgtcattaccttctcgtttggtatgggtgccattccatggctcatgatgtctgagatcctcccggttagcatcaagagccttggcggaagcatcgcaacactggccaactggctgacatccttcgccataacaatgacgacgaacttgatgctcacgtggagtgttggaggcacttttctctcgtacatggttgtgagcgccttcaccatcgtttttgttgtcctttgggtgccggagacgaaggggagaactctagaggagatacaattttcgtttcgctga

SEQ ID NO: 141 - DNA, 1506 bp, Oryza sativa
  >OsA - Oryza sativa
atgagcttccgcggcgaggagagcggcggcgaggatggggggcggacggcgtcggcgtcggacctgcggaagccgttcctccacacggggagctggtacaagatgtcgtcggcgggcggcggcggcgggatggggtcgcgcctcggctcctccgcctactccctccgcgactcctccgtctccgccgtcctctgcaccctcatcgtcgccctcggccccatccagttcggcttcacctgcggcttctcctcgcccacccaggacgccatcatctccgacctcggcctcaccctctccgagttctcgctgttcgggtcgctgtcgaacgtcggggcaatggtgggcgccatcgccagcggccagatcgccgagtacatcggccgcaaggggtctctcatgatcgcggcaattcctaacattattgggtggctcgcaatatcttttgcaaaggactcatcctttttgtttatgggccgattgctggaaggatttggggtcggcgtgatatcctatgtggtgccagtttatatagcagaaattgctccacaaacaatgagaggagctcttggttcagtcaatcagctttctgttactattggcatattgcttgcctacttgttaggcatgtttgttccctggagaattctctccgttctcggtattttaccatgttcaattctgatacctggattgttctttatccctgaatcaccaaggtggctggcaaaaatgggaaagatggaggattttgaatcctcgctgcaagtattgcgaggatttgaaacagacatcgctgtagaagtaaatgaaataaagagaacagttcaatcatcacggaggaggacgacaatacgatttgcagatatcaagcagaagagatatagtgtacctctaatgataggaattggtctccttgtactgcagcagttaagtggtgtgaatggcattctattttatgctgctagtatcttcaaagccgccggtcttacgaatagtaatctagcaacatttggtctgggggttgttcaggtggttgctactggagtgacaacttggttgactgacaaagctggtcgacgactcctcctcattatctctactacagggatgaccattactcttgttgttgtttctgtgtcattttttgtgaaggacaacataactaatggttctcatttatactctgtaatgagtatgctttcgctggtcgggcttgtggcatttgtgatttcattttctcttggtttgggagccataccatggatcataatgtctgagattcttcctgtaaatatcaagagccttgctggaagcgttgcaacccttgcaaactggttgacggcttggctcattacgatgacagcaagcttgatgttaagctggagcaatggaggaacatttgctatctatgctgctgtgtgtgccgggaccctcgttttcgtatgcctgtgggtgccggagactaaaggaagaacacttgaggaaattgcattttctttccggtga

SEQ ID NO: 142 - DNA, 1506 bp, Oryza sativa
  >OsB - Oryza sativa
atgaacaggggcggcggcgtcggcgtcggcgatgagagcggaagcgactacgagagcggcggcggcatgcggaagccgctgctgatgcacacggggagctggtacaggatggggtcgcggcaggggagcctcaccggcgcggggacctcgtccatggccatcctacgcgagtcccacgtctccgccttcctctgcacgctcatcgtcgcgctcggccccatccagttcggattcacggggggcttctcctccccgacgcaggacgccatcatccgagacctcgacctcaccctctccgagttctcggtgttcggatcgctgtccaacgtcggcgccatggttggggcgattgccagtggtcagatggccgagtacattgggcgcaaagggtcattgatgattgctgcaattccaaacatcattggttggcttgccatctcctttgcaaaagactcatcgtttctttatatgggacgattgctcgaggggtttggtgttggtgtcatctcttatacggtgccagtttacatagcagaaatatcacctcaaaacatgagaggtgctcttggctcagtgaatcagttatctgtaaccgttggtatattgttggcatatttgctcggcatgtttgttccttggaggcttcttgctgtaataggaatcttgccttgcactgtgttgatacctggcctattcttcattccagaatccccaagatggttggcaaagatgaacatgatggatgattttgagacttctttacaagttctgaggggatttgagactgacatcagcgcggaagtgaatgatataaagagagcagtagcgtcagcaaacaaaaggacaacgatccgttttcaagaattaaaccagaagaaataccgcacacccctaatactaggaattggcctacttgtactgcaacagctaagtggaatcaatggaatattgttttatgcaggtagcatcttcaaagcagcaggtctcacaaacagtgacttggctacatgtgcacttggtgctatccaggttcttgctacaggagttacaacctggttattagacagagctggccgacggatcctccttatcatctcttctgctgggatgactctaagcctccttgcagttgctgttgtatttttcctcaaggatagcatttcacaagattctcacatgtactacaccttaagtatgatctccttggttgctcttgtggcttttgtaatcgccttctccttcggtatgggtgccattccatggatcataatgtcagagatcctcccggttagtatcaagagtctcgcaggaagctttgcgacgctcgccaactggcttacatcctttggaataacaatgacagcaaacttgatgcttagctggagtgctggagggacctttgtgtcctacatggtcgtgagtgctttcaccctcgtgttcgtcatcctttgggtgccagagacaaaaggaagaactctcgaagagatacaatggtccttccgctga

SEQ ID NO: 143 - DNA, 1494 bp, Oryza sativa
  >OsC - Oryza sativa
atgaacggcggcgggagcaggcggggaggtgcgtcgtgcgccgacgagagcggcagcgaccaggacggcggcagcggcggcggcttgcggaagccgctgctgaacacggggagctggtacaggatgggatcgcggtccagcctcgccgcctcctccatggccgccatccgggagtcccacgtctccgccttcctctgcacgctcatcgtcgcgctcggccccatccaattcggattcaccagcggcttctcctcacccacccaggacgccatcatccgcgacctcaagctctccatctccgagttctcggctttcggttcgctgtccaacgtcggcgccatggtcggagcgatcgccagtgggcagatggcggagtacattggccggaaagggtcgttgataattgcggcggttcctaacatcattggttggcttgccatctcctttgcaaaagacgcgtcatttttatacatgggacgcttgcttgaaggttttggtgttggtgttatatcatatacggtgccagtatacatagcagagatatctcatcagaacacaagaggagcacttggctccgtgaaccagttgtccgttaccattggtatcttgttggcctatttgctaggcatgtttgttccttggaggctgcttgcagtgataggaagcatcccatgtacattgttaatacctggtctattcttcattccggaatccccaagatggctggcaaaaatgaaaatgatggatgattttgaggcttctctacaagttttgagggggtttgagactgatattactgcagaaagagcagtagcatcggcaaacaaaagaaccacagtccgttttaaagagttgaaccaaaagaaataccgcactcccttactgataggaactggccttcttgtacttcagaatctaagtggaataaatggtattctgttttatgcaagtagaatcttcagagatgcagggtttacaaacagtgacttggccacatgtgcactaggagcaattcaggttcttgccactggagttacaacatggttactggacagagctggtcgacggatgctccttattatctctactgctgggatgactctaagccttcttgcagtatctgttgtattttttctggagggtaatatttcacatgattctcattcgttctacatcttaagtatgatctccttggttgctcttgtggcttatatcatcaccttttccttcggcatgggtgccattccatgggtcatgatgtctgagatcctcccagttagcatcaagagtcttgggggaagctttgcgacacttgccaacatgcttacatcctgggcaataacaatgacagcaaatttgttactcagctggagtgctggaggaacatttttgtcctacatgattgtgagtgctttcactctcgtgttcgtcatattttgggtgccagagacaaagggaagaactctggaggagatacagttttcgttctgctaa

SEQ ID NO: 144 - DNA, 1512 bp, Hordeum vulgare
  >HvA - Hordeum vulgare
atgaacggcggcagcagcggcagggccggcggaggcggagggggagggtacgagagcgggagcgaccatgacacgcggaagcagccgctgctggtcaacacggggagctggtaccggatggggtcgcgccagtccagcctcacggcgggcacctcctccatggccatcatgcgggagtcccacgtctccgccttcctctgcaccatgatcgtcgcgctcggccccatccagttcggcttcaccggcggcttctcctcccccacccaggacgccatcatccgcgacctcaacctctccatctccgagttctccgtgttcggctcgctgtccaacgtcggcgccatggtcggcgccatcgccagcggccagatggccgagcacattggccgcaaagggtcactgatgattgctgctattcctaacatcatcggctggctggccatctccttcgcaaaagacacctcttttctgtatatgggacgattgctcgaaggatttggtgttggtgtcatatcctacacggtgccagtatacatagcagagatttctcctcagaacatgagaggcgctctaggctctgtgaaccagttgtcggtaacgattggtatcgtgttggcctacattctcggcatgtttgttccttggaggatgcttgcagtgataggaatcttgccatgcacaatattgatacctggtctgttcttcattcccgaatctccaagatggctggcaaagatgaacaagatggaggacttcgaaacctcgcttcaagttttgaggggatttgagactgacatcacctcagaagtgaatgatataaagagagcagtaacatcagcaaacaaaagggcggccatccgtttccaggagttaaaccaaaagaagttccgcatgcccctcattctaggaattggcctgcttgtactgcaacagctgagtggaatcaatgctatactgttctatgcaagtagcatcttcaaagctgcaggtattacaaacagtgacttggccacatgtggacttggaggtattcaggttcttgccactctagttacaacctggttactggacagagctggccgacggattctactcattatctcttctgccgggatgaccctgagccttcttgcggttgccgtcgtattttttatcaaggacactgtttcacaagattctcacatgtattacatattgagcatggtctccttgcttgctattgtggcctatgtaatcgccttctccttcggaatgggtgccattccatgggtcataatgtcagagatcctccccgtgagcatcaagagtctcgcgggaagcttcgcgacgctcgccaactggctgacttccttcgggattacgatgacggcaaacttgctgctcagctggagtgctggaggtacatttgtgtcgtacatgctcgtgagcgccttcacgctcgtgttcgtcgtcctctgggtgccggaaaccaagggaagaacgctcgaggagatacaatggtcgttccgctga

SEQ ID NO: 145 - DNA, 1512 bp, Hordeum vulgare
  >HvB - Hordeum vulgare
atgaacggcggcagcagcggcagggccggcggaggcggagggggagggtacgagagcgggagcgaccatgacacgcggaagcagccgctgctggtcaacacggggagctggtaccggatggggtcgcgccagtccagcctcacggcgggcacctcctccatggccatcatgcgggagtcccacgtctccgccttcctctgcaccatgatcgtcgcgctcggccccatccagttcggcttcaccggcggcttctcctcccccacccaggacgccatcatccgcgacctcaacctctccatctccgagttctccgtgttcggctcgctgtccaacgtcggcgccatggtcggcgccatcgccagcggccagatggccgagcacattggccgcaaagggtcactgatgattgctgctattcctaacatcatcggctggccggccatctccttcgcaaaagacacctcttttctgtatatgggacgattgctcgaaggatttggtgttggtgtcatatcctacacggtgccagtatacatagcagagatttctcctcagaacatgagaggcgctctaggctctgtgaaccagttgtcggtaacgattggtatcgtgttggcctacattctcggcatgtttgttccttggaggatgcttgcagtgataggaatcttgccatgcacaatattgatacctggtctgttcttcattcccgaatctccaagatggctggcaaagatgaacaagatggaggacttcgaaacctcgcttcaagttttgaggggatttgagactgacatcacctcagaagtgaatgatataaagagagcagtaacatcagcaaacaaaagggcggccatccgtttccaggagttaaaccaaaagaagttccgcatgcccctcattctaggaattggcctgcttgtactgcaacagctgagtggaatcaatgctatactgttctatgcaagtagcatcttcaaagctgcaggtattacaaacagtgacttggccacatgtggacttggaggtattcaggttcttgccactctagttacaacctggttactggacagagctggccgacggattctactcattatctcttctgccgggatgaccctgagccttcttgcggttgccgtcgtattttttatcaaggacactgtttcacaagattctcacatgtattacatattgagcatggtctccttgcttgctattgtggcctatgtaatcgccttctccttcggaatgggtgccattccatgggtcataatgtcagagatcctccccgtgagcatcaagagtctcgcgggaagcttcgcgacgctcgccaactggctgacttccttcgggattacgatgacggcaaacttgctgctcagctggagtgctggaggtacatttgtgtcgtacatgctcgtgagcgccttcacgctcgtgttcgtcgtcctctgggtgccggaaaccaagggaagaacgctcgaggagatacaatggtcgttccgctga

SEQ ID NO: 146 - DNA, 1500 bp, Hordeum vulgare
  >HvC - Hordeum vulgare
atgaacggcggcggcgggggcgacgacagcggcagcgaccatgagggcggcggcgcgggcgcgcggaagccgctgctgctcaagaacacggggagctggtacaggatggcggggtcgtcgtcgcgccagtcggtcggcgcctcctccatggcggtgctccgcgagtcccacgtctccgcgctcctctgcacgctcatcgtcgccctcggccccgtccagttcggcttcacctgcggcttctcctcgcccacccaggacgccatgatccgcgacctcggcctctccatctcccagttctcggcgttcggctcgctgtccaacgtcggcgccatggtcggcgccatcgccagcggccagatggccgagcacattggccgcaaagggtcgttgatgatcgcggcgattcccaacatcatcggttggctcgccatctcattcgcgaatgactcgtcgtttctctacatgggccggttgcttgaaggatttggtgttggtgtcatatcctacacggtacctgtatacatagcagagatatctcctcagagcacgagaggagcgcttggctctgtgaaccagctatctatcacacttggcatcttcttggcctatgtgctaggcatgtttgttccttggaggctgctggcagtactagggaccttgccttgtacattgttgattcctggtctattcttcattccggagtctccaagatggctggcaaagatgaacttgatggatgatttcgagacttctctgcaagttttgaggggtttcgagaccgacatcactgcggaagtaaatgatataaagagagccgtagcgtcagcaaacaaaaaggccacggtccgttttcaagagctaaatcaaaagaagtatcgaactcccttactaataggaactggccttctagtacttcaaaatctatgtgggataaatggcatactgttctatgcaagtagaatattcagagctgcagggttcacaaacggtgacctggccacatgtgcacttggagctattcaggttctcgccacgggagttacaacctcgttgctagataaagctggccgacggatgctccttattatctccactgcagggacgactctaagccttcttgcagtttctgttgcatttttcctcaaggataatctaccgcatgattctcactcggactacatcttaagtatggtgtccttggtggctcttgtggcttatatcatcaccttctccttcggcatgggtgccattccatggctcataatgtctgagatccttccggtcggcatcaagagtttcgccgggagctttgcgacgctggccaacatgctcacttccttcggggtgacgatgacagcaaacctactactgagctggagcgctggcgggactttcgcgtcgtacatggtcgtgagcgcgttcaccctcgtgttcgtcatactttgggtgccggagaccaaggggaggaccctggaggagatacagtggtcgttccggtga

SEQ ID NO: 147 - DNA, 1500 bp, Secale cereale
  >ScA - Secale cereale
atgagcttccgggacgagagcggcggggaggacggcagcgggggccggtcgtcgtcggcgtccgacctgcgcaagccgttcctgcacacggggagctggtacaggatgtccgcggccggcggcggcgccatggaccggctcggctcctccgcctacggcctgcgcgacagctccatctccgcgctgctctgcaccctcatcgtcgcgctcggccccatccagttcggcttcacctgcggctactcctcgcccacccaggacgccatcatggccgacctcggcctcaccctctccgagttctctttattcggatccctgtccaacgtcggggccatggtgggcgccattgccagtggccagatcgccgagtacatcggccgtaaagggtctctgatgatcgccgcaatcccgaacatcattgggtggcttgcaatatcatttgcaaatgattcctcattcttgttcatgggccggttgctggaaggatttggggtcggtgtgatatcctacacggtaccagtttatatagcagaaattgctccacagaacatgagaggagctcttggttcagtcaatcagctctctgtcacaatcggtatattgcttgcctacacattaggcatgtttgttccttggagaattctctctgttcttggcattttaccttgctcaatcctgatacctgggctgttcttcatccctgaatcaccaaggtggctggcaaaaatgggaaagatggaagattttgaatcgtcactgcaggtcctccgtggatttgaaactgatatctcagcagaagtaaatgaaataaagagatcagttgcctcatctaggaggaggacaaccatacgatttgcagagatcaaacacaagagatatagtgttcctcttatgataggaattggtctccttatacttcagcaactaagtggtgtcaacggcattttcttctatgctgcaagtatcttcaaagctgctggtcttaaaaatagtaatctagcaacatgtggtttgggggctgttcaggtggttgctactggaataacaacctggttgactgacaaagctggtcgacggctacttctcattatctctgctgtagggatgacagtcagtcttctcgttgtttccgtgtcattttttgtgaaggacaacatagatgaagcttctcatttacactctgtgatgagtatactttcactggctgcacttgtggcatttgtgtttgcattttcccttggcatgggagccatcccatggattataatgtctgagattcttcctgttaacatcaagagccttgccggaagcacggccaccctgaactggatgacgtcgtggctcatcacgatgaccgcgagcttgatgctaaactggagcaatggaggaacctttgctatatacgcggcggtgtccatgggcaccctcctcttcgtgtgcctgtgcgtgccggagaccaaggggagaaccctcgaagagatcgcgttctcgttccgctga

SEQ ID NO: 148 - DNA, 1515 bp, Secale cereale
  >ScB - Secale cereale
atgaacggcggtagcagcggcagggccgggggcgggggagggggagggggagggtacgagagcgggagcgaccatgacacgcggaagcagccgctgctggtgaacacggggagctggtaccggatggggtcgcgccagtccagcctcacggcggggacctcctccatggccatcatgcgggagtcgcacgtctcggccttcctctgcacgatgatcgtcgcgctcggccccatccagttcggcttcaccggcggcttctcctcccccacccaggccgccatcatccaggacctcggcctctccatctccgagttctccgtgttcggctcgctgtccaacgtcggcgccatggtcggggccatcgccagcggccagatggccgagcacattggccggaaagggtcactgatgattgctgctattcccaacatcatcggctggcttgccatctccttcgcaaaagacacttcttttctgtatatggggcgattgcttgaagggtttggtgttggtatcatatcctacacggtgcccgtatacatagcagagatttctcctcggaacatgaggggcgctctaggctgtgtgaacccgttgtctgtaacacttgggatggtgttggcctatgtgctcggcatgcttgttccatggaggatgcttgcggtgataggaaccttgccatgcacaatattgatacctggcctattcttcattccagaatctccaagatggctggcaaagatgaacaagatggatgacttcgaaacctctctacaagttctgaggggatttgagactgacatcacctcagaagtgaatgacataaagagggcagtaacatcagcaaacaaaagggcggcaatccgtttccaagagttaaaccaaaagaaattccgcatgccgctgattctaggaattggcctgcttgttctacaacagctaagcggaatcaatgctatactgttctatgcaagtagcatcttcaaggctgcaggtattacaaacagtgacttggccacatgtggacttggaggtattcaggttcttgccactctagttacaacctggttactagacagggctggccggcgtatcctactcattatatcttctgctgggatgaccataagccttcttgcggttgccgtcatattttttatcaaggacactgtttcacaagattctcacatgtattacatactgagcatggtctccttgcttgctattgtggcttatgttatcgccttctccttcggcatgggggctattccatgggtcataatgtctgagatcctaccggtaagcatcaagagtctcgccgggagcttcgcgacgctcgccaactggctgacttcctttgggataacgatgacagcaaacttgctgctcagctggagtgctggaggtacatttgtgtcctacatgctcgtagccttcacgctcgtgttcgtcatcctctgggtgccggagacaaagggaagaacactcgaggagatacagtggtcgttccgctga

SEQ ID NO: 149 - DNA, 1488 bp, Secale cereale
  >ScC - Secale cereale
atgaacggcaagggcggagacggcggaggagggcgcgagagcggccacgacgacgacatgcggaagccgctgctggcggcgagcacggggagctggtacaggatggggtcgagcctcacggcgggggcgtcgtccatggccatcacccgcgagtcccacgtctccgtcttgctctgcacgctcatcgtggccctcggccccatccagttcggcttcaccggcggcttctcctcgccgacgcaggacggcatcacccgcgacctcagcctctccatctccgagttctcggtgttcggctcgctctccaacatcggcgccatggtgggcgccatcgccagcggccagatggtagagcacgttggccacaaagcggcattgatgatcgctgctgttcccaacatcctcggctggctcgccatctccttggcaaaagacactacgtttctgtatacggggcgattgcttgaagggtttggtgttggtatcatatcctacacggtgcccgtatacatagcagagatttctcctcagaacatgagaggcgccctaggctctgtgaaccagttgtccgtaacgattggcatcgtgctggcctatattctcggcatgtttgttccttggaggatgcttgcagtgataggaatcttgccatgcacaatactgataccaggcctattcttcattccagaatctccaagatggctggcaaagatgaacaagatggatgacttcgaaacctctctacaagttctgaggggatttgagactgacatcacctcagaagtgaatgatataaagacagcggtagcatcagcaaacaaaatgacggcaattcgtttccaagagttaaaccaaaagaaattccgcatgcccctgatactaggaattggcctgcttgtactacaacagctaagtgggatcaacgctatactgttttatgcaggcagcatcttcaaagctgcaggtcttacaaacagcaacttggccgcatgtggacttggagctattgcgcttcttgccactggagctacaacctggttgctagacagagctggccgacggattctactcattatctcttctgccgggatgaccctaagccttcttgcaattgccgtcatattttttctcaaggacaacgtttcacaagattctgacatgtattacatattaagcatggtctccttgtttgctattgtggcttatgtgatcaccttctcctttggtatgggcgccattccatgggtcataatgtctgagatcctgccggttagcatcaagagcctggcaggaagcttcgcgacgctcgccaactggctgacctcctttgggataacaatgacagcaaacttgctgctcagctggagtgctggaggtacctttgtgtgctacacgctcgtgagcgccttcacgctcgtgttcgtcatcctctgggtgccagagaccaagggaagaactctcgaggagatacagtggtcgttccggtga

SEQ ID NO: 150 - DNA, 1524 bp, Sorghum bicolor
  >SbA - Sorghum bicolor
atgagctttcgggaccaggagagtggcggggaggatgcgggcaggacgtcctccgcgtccgacctgcggaagccgctcctgaacaccgggagctggtaccgcatgccgccgccgggcggcatgatgggctcgcggcagtcgagcctcatggagcgcctaggctcctctgccttctccctccgagacgttgctatctcggcgacgctctgcacgctcattgtggctctaggtcctatccagttcggtttcacctgcggttactcctctcccacgcaggacgccatcattgctgacctcggcctctcactctccgagttctctctgttcggatcgttatcaaatgtaggggcgatggtaggtgccatctccagtgggcaacttgcagagtatatcggccgcaaggggtctctcatgattgctgcaattccaaacataattgggtggcttgcgatatcatttgcaaaagattcctcattcttgtttatgggccggctgctagaaggatttggagtgggtgtaatatcttatacagtaccggtttatattgcagaaatcgctcctcaggatcagaggggagctcttggttctgtcaatcagctctccgtcacagttggtatattgcttgcctacctgtttggcatgtttgttccctggagaattcttgctgttctaggcattttaccttgttcaatcctgattcctggactgttctttgtccctgaatccccaaggtggctggcaaaaatggggaagatggaggattttgaatattcactgcaagttctgcgaggatttcagacggacattacagcagaagtaaatgaaataaagagatcagtagcatcatcaaggaggaggacaaccgccataaggtttgctgatatcaagcagaagagatacagtgttccccttgcgataggaatcggtctccttgtcctgcagcagctaagtggtgtcaatggcattctattttatgctgggagcatcttcaaagctgctggtattacaaacagtaatctagcaacctttggtttgggggctgttcaggtgattgctactggagtgacaacctggttgactgacaaagctggtcgaaggcttcttctcattatttctaccacaggaatggtcattactcttgtcattgtttctgtgtcattttttgtgaaggacaacataactgccggttctcacttatactctgcaatgagtatgctttcactggctggacttgtggcatttgtgattgcattttctcttggcttgggagcaattccatgggtcattatgtctgagattcttcctgttaacattaagagccttgctggaagtgttgcaacccttgcgaactggctaacagcatgggccattacaatgactgcaagcctaatgttaaactggagcaatggaggaacctttgctatctatgccgctgtgtctgccatggccctcattttcgtgtgtttgtgggtgccggagaccaagggaagaacattagaggaaatcgcattctcattccgctga

SEQ ID NO: 151 - DNA, 1500 bp, Sorghum bicolor
  >SbB - Sorghum bicolor
atgggtggcggcggcagcaacagaggcggcgccggcgaggagagcggcagcgaccacgacggcgggctgcggaagccgctgctccacacgggcagctggtaccggatgagctcgcggcagtccagcgtcgcccccggggcctcctccatggccgtcctgcgggagtcccacgtctccgccttcctctgcacactcatcgtcgcgctcggccccattcagttcggcttcaccagcggcttctcctccccgacccaggacaccatggtccgggacctcaacctctccatctccgagttctcggcgttcggctcgctgtccaacgtcggcgccatggtcggggcgatcgccagcgggcagatggccgagcacattggccgtaaagggttgttgatgattgctgcaatcccgaatatcatcggttggcttgcgatctcctttgcaaaagatgcctcatttctttatatgggacgattgcttgaagggtttggtgtcggcatcatatcctatacggtacctgtatacatagcagagatatctcctcagaacatgagaggagctcttggttctgtgaaccagttgtctgtgacctttggcatattcttggcctatttgctcggcatgtttgttccttggagacttctagctgtgatcggagccttgccctgcacagtgttgattcctggactattcttcattccagaatctcccagatggctggcaaagatgaatttgatggaagattgtgagacgtccctacaagtgctgagggggtttgagactgacataacgacagaagtgaatgatataaagagagcagtgacatcatcaagtaagaggactacaataagttttcaagaattaaaccaaaagaaataccgcacgccactacttctaggaattggcctacttgtactacaaaatttaagtggaatcaacggtgtactgttttatgcaagtaacatcttcaaagctgctggtgttacaaacagcaacttggccacctgttcacttggagctatccaggtccttgctactggagttacgacatggttgttagacagagctggacgacgcatgcttctcattatttctacctctggcatgactctatgccttcttgctgtttctgttgtattttttgtcaaggataagacttcacaggattctaactcgtactacatattaactatgatctccttggtttctatcgtggcttttgtcattaccttctcgtttggtatgggtgccattccatggctcatgatgtctgagatcctcccagttagcatcaagagtctcggcggaagcatcgcaacactggccaactggctgacatctttcgccataacaatgacgacgaacttgatgctaacctggagtgttggaggcactttcctctcgtacatggttgtgagcgccttcacccttgtttttgtcgtgctttgggtgccggagacgaagggaagaactctagaggagatacaattttcgtttcgctga

SEQ ID NO: 152 - DNA, 1506 bp, Sorghum bicolor
  >SbC - Sorghum bicolor
atggcgagcaacagggcatccggcagcgagtacgagagcggcagcgaccacgacggcgcgctgcagaagccgctgctgcccaacagcgggagctggtaccggatggggatggggtcgcgccagtccagcctcaacgccgccggcacctcctccatggccgtcctgcgcgagtcccacgtctccgccttcctctgcacgctcatcgtcgcgctcggccccatccagttcggcttcaccggcggctactcctccccgacgcaggccagcatcatccgggacctcaacctctccatctccgagttctcggtgttcggctcgctctccaacgtgggcgccatggtcggggcgatcgccagcgggcagatggccgagtacatgggccgcaaagggtcgttgatgattgcagcgattccgaacgtcattggttggcttgcaatctcctttgcaaaagactcttcatttctgtatatgggacgcttacttgaaggatttggtgtcggtatcatttcctatgtggtaccagtatacatagcagagatatctcctcagaacatgagaggggctctaggttctgtgaaccagttgtctgtaacccttggtatcatgtttgcctatttgctcggcttatttgttccttggaggcttcttgcagtaataggaaccttgccctgcatagtgttgatacctggcctattcttcattccggaatctccaagatggctggcaaagatgaatatgatggatgattgtgagacttctctacaagttctgaggggattcgatgctgacatcactgcagaagtgaatgatataaagagagcagtaacatcagcaaacagaaggactacaatccattttcaggagttgaaccaaaagaaataccgaacacccctaattataggaattggtctacttgtgctgcaacagctaagtggaataaatggtatactgttttatgcaagtagcatcttcaaagctgcaggtctcaaggacagtgacttggacacatttgcacttggagctattcaggttcttgccactgttgttacaaccatgttcttggacagagctggtcgacgaatcctccttattatttcttctgctgggatgactataagccttcttgtagttgctattgtattttacatcaaggataatctttcacatgactctgacttgtataacatcttaagtatggtgtccttggttggtgtcgtggcctatgtcattgccttctccttcggtatgggtgccattccttggatcataatgtccgagatcctcccagttagcatcaagagtcttgcaggaagctttgcgacccttgccaactggttgacatcctttggaataacaatgacagccaacttgctgatcagctggagtgctggaggtacgtttgcctcctacatgattgtgagtgccttcactctcgtgtttgtaatcatttgggtgccagagacgaagggaagaaccctcgaggagatacaatggtcattccgctga

SEQ ID NO: 153 - DNA, 55 bp, Artificial Sequence
  ERDL4_fwd primer
ggggacaagtttgtacaaaaaagcaggcttaatgagttttagggatgataatacg

SEQ ID NO: 154 - DNA, 54 bp, Artificial Sequence
  ERDL4_rev primer
ggggaccactttgtacaagaaagctgggtatcatctgaacaaagcttggatctc